European Patent Application EP 4 159 862 A1, published April 5, 2023. Title: METHOD FOR PREPARING COMBINATORIAL LIBRARY OF MULTI-MODULE TYPE BIOSYNTHE SIS ENZYME GENE. Applicant: Spiber Inc. The sequence listing filed with the application follows.

SEQUENCE LISTING (38 sequences)

SEQ ID NO: 1 - DNA, 3427 bp, Artificial Sequence
  DNA fragment
cgtctcattggtcgagcgtctgtcggacgcgcagcgcctgggacaccccatcttggctgtagtgcgcggttcggccattaaccaggacggtgcctcgaacggtttgaccgcccccaacggtccggcccagcaacgcgtaattcggcaggcgcttgctacagcaggattgggtccaaccgatattgacgcggtagaaggtcacggcaccggtacgtcgctcggcgacccaatcgaggcgcaggctctgatggaaacctacggtcaagagcgacccgaggaacggcccttgtggctcggctcgttgaagtcaaacatcggtcatgcacaggcggcagccggtgtaggcggtgtaatcaagatggtcatggcgctcggagagggagtcctgccccgcaccttgcacgcggacgagccgtcaccacacattgactggaccgcgggcaacgtacgtcttctgacggaatccagggaatggccggtcaccggacagccccggcgcgccggtatttcgagcttcggtgccagcggcacaaacgcccatttgatcctggaacaggcgccggctcgtccggctgaggacacaccggaggaaccggcactcccattggtaccttggctcgtatcggcaaagagtgaggcggcattgagagctcaagccgagcgcttgcgctcctatgtcgctgagcgccctggtctgcgtccggctgacgtagcattcagcttggcgaccacgcggggcgcgctcgaacatcgtgctgtcgtggttggtacggacctgggcgagctggcggagggcctgggggctctgacccagaccgccaccgtcgtaccgggtcggaccgcattcttgttcaccggtcagggtgcacaacgcgtcggaatgggtcgcgaactctatgacacatttccggccttccggaaggcgctggacgaggtctgcgctgtgctggatccgttgctcccccgtccttcgcgggaagtgatgtgggatgaggatccagaggctctgtcgagaaccgagttcacccagccgacgttgttcgccatcgaggtcgctctgttccgcttgctggagtcatggggcattcatcctgacgcagtggcgggtcactcaatcggtgagatcgcggctgcgcacgtaaccggtgtgttgtcgctcgctgacgcatgtgtccttgttgccgctcgcggccgtctgatgcaggcattgccccatgacggcgtgatgatcgccgtacaagcaacggaggatgaggtgttgcccctgttggagaaagtgaccggtcaagctgacatagccgcggtaaacgctcccgaagccgtggtcgtgtctggcgccgaaacggaggtcgagcatgtggctgccaccttgggcgcccagggtcggcgtgtcaagcgcttgaccgtcagccacgctttccattccccgttgatggaccctatactgaaggacttccaaaccgtagtggagggcctcagtttcaggcaaccatccctgccgtttgtctccacggtcactggaacggttgctggcgccgaaataaccgaaccagcatactgggtccgtcacgttcgtcagacagtgcggttcgccgacggactccgcgcgctgcacgaacttggcgtcaggaagttcatcgaaattggaccggacgcgattctgacgggactggtggagcaaacgctcgacacccaagcggtccccgtccttcggcgtgaccgggatgaggtgcgcgccgctgtcgaagcggctggcggtttctttacacgcggcggtagcgtcgactggccagcacttctggcgggtggaagacgtgtagacttgccaacgtacgcgtttcaacatgaaaggtactggttggacgcccccgtgtccgtcggcgacgctaccgctctgggattgcgccgggcagaacatccactgctcggagcggcagtggagctggccggctccgatcggatggtattcgctgggcgtttgtccgctgcgtcccaaggctggctggtggatcatgccgtccatggtaccgtgcttgtgccgggtaccacattggtagagttggccctggctgccggtgaccagatgggctcgggccgcctggaagagttgaccctccaggcaccactggtcctgcctgaaaccggtgcggtgcagctccaggtgtccgtgggtgaggcagacgcagagggacgcagaaccgtcgaaatccatagccgcccagagcgggatgcagcggaggtcgcatgggcatgtaacgctttgggcgctctgaccgaagcggcagcggaacccacccccgccgcactgggcgaagtctggccaccgcaggacgcttccgccgtggaagtcggcgatttctatgacgatctggccgacaggggctacgaatatggacccgtgttccagggcctgcaccgggcttggcggcgtggtgacgaagtattcgccgaggtagcgttgccagaagaggcagcgaacaccgtcgatgccttcggcgtgcatcctgccctcctggacgctgccttgcatgccatgaactttgccagcgtcaccatgggaagcggaacccctttgccattcgcgtggacgggtgtgacgctgcacgcggtgggcgcaaccgcgcttcgggtgcgcatagcccccgacgatgcccggggtgccgtatcggttgaattgttcgaccaggccggacttcctgtcgcatctgtggaaagcttggcgctgcgtgaggtgtcgcccgagcaactggccgtcgcggatgaccccgatagcttgttcgaggtagaatgggtaagcgcagcggacggcggatccgccgaagccggtgccccgagttgggcggtactgggcgatagccctttggcggaaggcggtcccgtgttcgcggacgtggaagctctggtggccagcagtcaggatttgccgggtaccgtggtattgcagtgccccgcggtagaaggggcgccggtcccagatgccgtacgtgaccgcttgacgggagtcctggatgtgctgcaacgctgggtcgccgacgaacgtctggcctcctctaggctggtggtagttacacgtggtgcagtggctgcgagcgctaacgagccggtagacgtccgtgttgcccccgtgtggggtctggtgcgtgctgcacaagcggaacatccggatcgtttcgtcctggctgatttgcccgcgggcgcgggagcccgcgaactctcggtcggcctcgcctgtgatgaaccgcaatgggcagtgcgggatggtgccgtccgtgtgccacggctggtacgcgcacaggctgcggtatcaggagtgccggcatttggtaacggtccggtattggtgaccggagcctccggtgccctgggtggcgtggtcgcgaggcacttggtgtctgtccatggagtccgtgagctggtacttgagacg

SEQ ID NO: 2 - DNA, 3432 bp, Artificial Sequence
  DNA fragment
cgtctcatgatgaaccgagccctcatatcgattggtccgcaggccaggtacgtctgctgaccgaggaacgcgagtggccggaggcgggacacccccggcgtgcggctgtttctagtttcggtgtaagcggcaccaacgctcacgtgatattggaagccgcacccggtactggtggagcaccagaagtctctgacggcgtgttgggctcggcgccggaaaccgtgccttgggtcctctcagctgcgtcccctgacgccctgcgcgcccaggctgaacgcttgcggggtcacgttgcagaaaggcctggtctggccagcgctgatgtagcctttgcactggcgacccggcgcaccgcactggagtaccgggcggtcgcagtaggcgcagaacgggatgagctgttggataccttggatgctctgtccgccggtcgccctgctccccgcgcagtgccaggtgatgcagctgcccactcccgtcggccagtcttcgtgttccctggtcagggttcccagtgggccggaatggccgtcgaactgctcgacagctcaccggtgttcgcagacagcatgcacgcctgttcggaagctcttaacgagttcgtcgactggaacctgctcgaagtgctgcggtcaggcgatgaagagttgagcaaccgtgtcgatgtagtgcaacctgtcctttgggcggtgatggtgtcactggccgcgctgtggcaggcatgcggcgtccgcccggcagcggtcgtaggacattcgcaaggtgagattgctgcggccgtcgtggctggcgcgttgagcctgcgtgatggtgcccgagtggtagctctccgctccgctgtcatagctcgcttgctggccggaaagggagcaatggcctctgtcgcccttgcttccgatacggtccgtgaacgtcttacgccctgggagggccggctctcgttggctgcggtcaacggtcccagttccagcgtagtgtgtggtcacctggatgcactggatgagttcgtgtcggctcttgaacatgacggtgtgcgtgtacgtcggatcgcggtggactacgccagtcactcggtatttgtcgagcaggcggaggaagagctgaggaacgtactgaccgaggtgagccctttgccgggtcaggtaccgttctattcaaccgtaaccggcgcagtactggataccacgaccctggacgcaggttattggtatcgcaacctgcggcaaacggtacgcttcgaggaaaccgtgcgcgagctgacccgacgcggccacgacgctttcatcgaggtgtcggcccacccagtgctgaccgtcggcatacaagatactcttgaagcgaccggtacccgtcacgctgtatgcggtaccttgcggcgcggcgagggtggcgcccagcgtctgttgacgtcccttggagaagcctgggtcgcaggtatcgcagtggattggtcccgcttgacgccgaccacaaccgctgtccagctgcccacgtacgcgttccagcaccaaaggtactggctcgactccaccacggccaacaccggcgatcgcccggccgcggaccgcgacacggcgttctgggaggcagtgcagcataccgatttggatgccttcgcggccgaacttgacatcgctcccgacgctccactgggaaccgtgttgcctgccctcgctgactggcggcagcgcctgcggaccgccgcagcggtggatgcgtggcggtaccgcacggcattcaagcgtctgcctgatgcacccggcgctccagtcctgacgggctcctggttggctgtcgttccggtccgccatctcgacgatccatcggttacgaccagcctggacgcggtggcaaaggccggtgctgaggtagtgcagctggccatcgaagacgccgacgccgacgtcgaccggctgaccgagaggctgcgcggcctggtcgccggtttgggcgctgccccggccggtataatgtcgttcttgggcctcgatgaagagcggcatcgcgaccatcctgcgatgcctagcggcctggccacctccttggcgttggtccgggccctgggtcgagcaggtataggcgccccgctctggatggtcacccgtgaggctgtcgccgcgggtcaagatacgcatccacatgctcccctcggctcactgatttgggggctcgggcaggtcacggcgttggagcacgcagaccgctggggtggcctcatagatctccctggagtctgtgatgctcgcgtcgcgcgcatgctctgcgctggcctcagcggtcggggtgcggaggatcagctggcgctgcgtccatcgggaacctttgtgcggcgcttggcccatatccctggagaacaacgtgcagcccgccggtcctggcagccccggggaaccgtgatcgtgaccggaggcaccggcgcccttggcgctgtcctggcccgctggctggccaccgaagacgcggagcatctggtgctcacgggtaggcgtggagctgatgctccgggagccgaacgcttgcgcgacgagctggtcgcgacgggtgcccgcgtcaccctcgctgcgtgcgacgtcgccgaccggaaggccgtcgctgcgctgttggatgaactggccgcggacggagaaaccgtccgcgctgtcttgcacgccgcgggagtggccgatttgacctccctcgagaacaccggcccggaagccttcgccgcgggcgtcgctgcaaaggtcgatggtgcgttgcacttgaccgagttgctcgaccatgactcgctcgacgctttcgtcctgttttccagcatcgccggagtctggggttcgggtgaccacggtgcctatgccgctgcgaacgcattcctgaacgccctggcggaatacaaccgggcacggggtattcccactacctcaatcgcctggggtgtttggaacgcattcggcgtcgagggtgcgggtggcatatccgaagcggtcgacctggaccaactgcatcgccgtggtctgcctctgatcgaacctgaattgggcttgacggcgttgcgtcgcgccctggaccgcgacgagactgtcctgacggtagctccggtggcgtgggaacgcttctttccactgttctctgctgcacggccccggcctctgtttgaggatctgccgcaagtgagggcgttgtcggcccccgtgcctaccacggcgggcccagctgtggaaccgggtcgtaggggaagcggtctgggcgaccttcctctcacggaccgcgatagcgcccttttggcgcttgtacgcggagaatcagcgtcggtcttggggtacgaaagacctgaccggctcgaccctgatcgcgctctccgcgatgtgggattcgattcccttacggcaatggagctgaggaaccgtctggccactgcaaccggcctgaccctcccagcggcactgtgagacg

SEQ ID NO: 3 - DNA, 3420 bp, Artificial Sequence
  DNA fragment
cgtctcacatacggccgccagaggccccttcggcaataggctaccatgtcaacacccttccactgaggctgacggtggaccctggacgcggtttccgcgacctcgtaaaggaggctcgcaccgctttctttggagcgctggcgcattcagacaccccggtggacgcgatcgcacacgagacagctagagagcccgtatcgtggcgcgacaccctgtttcagcatatgttcaactacgtccctgttgagagcgccggtgctcttacgctgggcggtgccccggcccgtgcgcttcacgttgaaacgggtttcagtaagttcgacctggagctgttcgtccagtcgggcgctgaccacattggcctgcgtatcttgtactgctcggaggtcctggaccgcgccgacgcccaggccctggcacaccgttatgcagcgttgctgcacaccgtggcggctgaccccgatcgcccggtaggggagttggacgtgtggtcggcggaggacagagctctcccaggtccgggcacggcacgctccgtcccagacaccgaagtggaagcggatggtgacctggacgcgttccgcacgagccccgacggctcggtcctgggcctggcggacgcggccgcgcactgtgcagctgccggtggctatccttatgtggtccacccacttgatgcacgtcatatcgcggtagttggaagggcgggcaaccgcctgccggcgggcgttcgtggtgaggtttgcctggtgcggccggaccgcgccacgcacgtcgccacaggctggacgggctcactgggccgggacggcgcgttggagctgtacggccgcgctgagcgggtcgccctcctgcacggtcgcgccgtacacccagaacgcgtagaggccgctctcctggcacaccctgaggtgacccgcgctgcattggtcgtgaccgacggcaccgcattggccttcgtcactgccgacgagcggccgggattggcagatgacgtcgcaggtcatgctgcgcgtctgctccccagggccgcgcaaccggcaagagtgatccgcaccgacacccttccactccgtccagaccatggttgggataccgctgcactcatggcgctggcggctgcggagcccgaatcaggacaggatgacgcggacggcttggtcgccgagcttcgtggtctgtggagagatcttctgggtctggctgaacctgtgggcgcggatgcggacttcttttccttgggaggtcatagcctgcttggcgcccagcttgtgcaacgggtggatgacgtgacaggtcgccgtatcaagttggctgatctgttcgacaacccaacccctcgttcgttggcgcgtcacttgcgcgctccccgcgcgggatcgtgacaaacaccccatgtcgatactgaacgaatcgacgcacactcccttccttggtatctgaaaggggatacgcatggaggtcagcctgatgggtctggctggtatgggttggattgccaagtcactgacagcggccgcagaactcggtttggcagaccatctcgacggcaccccaatgaccgcagaagagctcgcaaagcagaccggcacccaccccgagacactggaggcacttttgcgcatcctgtcagccctgggtgtgtttcggcgcgacgatgccggtgtttaccgcaactccgcgttgtcggaccaattgcgcgatgaccatcctcaatccatgagacattacgtgatgctttcgggcggtctgtatgctgacaccttcacagcggtaacccacacacttcgcaccggtgaatccgcctttcggcatctgcacggtacgaggatctatgagtacttggaacagaggccggcggaggctgacctgtatgacaaggccatggcagacctggcccgcccggtggcggctgccctggcaggtacctatgattttggcgcggtaaggtcagtgcttgacgtgggaggcaactccggcgagctgttgaagggcctgctcacagcccatccgcatctgacgggtacttgcctggaccgcccggacgtctgcgctcgggcgaccgcagaattggcggcctcagaccgtgaggacctgaaggatcgtctggtctaccggccaggggacttccttcaagaagtgcccgccggatccgatctgtacacagtgaagaacgtcttgcataactggaaccatgaacattcagtggtaatcctgggccggatccgggaagctatggaaagaacagacgccgatcgttcagccggacgtagggctcggctgctcgtgatagagccacttatcgagacagatttggactggatgcgtgtcctgttccagatggtcgtatgcgaggacggcacccgtggtaggacagacgaagtgcaacgtgcgcagatagccgaagccggtcttgaagtgctcgacacgctgcgcctgagcacaggtcatacggcccacatttgcgcagcggcccactgacaaacaccccatgtcgatactgaacgaatcgacgcacactcccttccttggtatctgaaaggggatacgcatgacgtccgcagtcgatacaggtgtttggattcgtcgctaccgcccggcacctgatgcaggcgtacggttgctctgccttccacacgcgggcggagcggcaagctactatgtaccggttgccgcggcactggcccctgcagcggatgtacttgctgtccaataccccggccgccaggatcgtcgctccgaagagccccttggtgacctgcgggagctggctgatcgcgtcgcggacgctgtgggtgacggtgacgagcgccctcttgcggtctttggacattcgatgggagcgctgctcgggtacgaggtagcacttcgcctggaggaagccgggcgcggtccggtccgcctgttcgtgagcggccgtcgggcaccttccgctgtacggccgtcggaggacatgcacaagcgcaccgacagcgccctgcttgacggtgtgcggcgtctgtccggaacggacgctcaggttttcgaggacgaagagctggtgcggatggtattgccagccatccgcgccgattaccgggccgtcgaaacctacgaaccgcggcctggcgatcgtgttcgctgcccagtcaccgtcctgaccggtgatgacgatcctatggccaccgtcgaggaagcgcgggcctggagcgctcacaccgaaggccctacggacctgcacgtgttcccgggcggacatttctaccttaacgaccgcgcggctgacgtcctcaccgtggtccgcgctcatctgggcctttgatgacataaccccttggggcctctaaacgggtcttgaggggttttttgcgcgacttccagagaagatgactactgacttgagcgttccaaaacttagcaggtggtcttgaaaatgagacg

SEQ ID NO: 4 - DNA, 3419 bp, Artificial Sequence
  DNA fragment
cgtctcaattagcacctgcttggattaactacacaatgagaccttgaggtaaaccaaataagcacgtagtggcgctgctccttcggtcggacgtgcgtctacgggcaccttaccgcagccgtcggctgtgcgacacggacggatcgggcgaactggccgatgctgggagaagcgcgctgctgtacggcgcgcaccgggtgcggagcccctcggcgagcggtgtgaaacttctgtgaatggcctgttcggttgctttttttatacggctgccagataaggcttgcagcatctgggcggctaccgctatgatcggggcgttcctgcaattcttagtgcgagtatctgaaaggggatacgcatggcgggcccaccgcctttccctcgtcggcgtggcccctcaggccgacgtcggtgcggcggacgggctacaccgggtagcgtccgggaccgcaccggcagacgcccagcggctgtccccagccgcgccgtgtgcgcggccgacctttgtgaagagaacgacgatggctccaagaacgtgtcggaacaccgcggatcagcgggtggtagcgttctgtttcctcgtacgggcacagtcctgccatgggtgcttacgggaccgggcgcagcggcggtgcgtgcacgctccgaagcgctgcgcacccacctccgcgcctctacggaatggagccctgcaggcgtaggtcaggcgctgctggcaggaacaggggcgggcgcggacacccaccgtgccgttgttctcgccggtgatcgtgcccaaactctgaatgccctggccgcgctgtctgcaggagcggaccacccagccgtctttaccagcacccgtgccgacgccagcccagctggtccagtgtttgtgtttccaggccaggggtctcaatggactggtatggctcgcgaattgttggattctgcccccgtatttgcccgtaaattgcatgattgcgccgacgcatttgccccgtatttgggtcacagcctcctggattccgttactggggcggccggcgggccagagcctgttggcgcggatgttgtgcaaccagccttgttcgcagtgatggttgccttgacggatctctggaatgcggccggtgtggcaccaggcgccttgctcggtcattcactgggggagctcgccgccgcccacgtcgctggcgttctcagcctggacgattcggcgcgcgtggtcgcgcgctggagccaagcccaagcaactctcgcaggccgtggggacatggtttccgtgctgctgcctgcggacgaactggcggatctgttggaccgccgttggccggggcgtctggtagttgcggtggagaatggcccgggtagtgccgtagccagcggtgatctggatgccgcggcagaacttgtagcccatcttactgcggaaggcattcatgcgcgtcgtgtcgatgtcggcttggccgcgcactctccccacatcgacgctattctcccccgcatccgcgcggatattgctccgatccgcgcacatacccccagtatccctgtttacagcgcgctgcacggcggcgcactcgacggtacccctatggatgcggcgtattggtgccgtaatttgcgttcaactgtgcgttttgcggatgctacgcgcgcagctttggaagcaggccatacaacatttgtggaagtttcacctcatccggtcttgacgacggccatggaagtgagtgccacccgtgcggcccatgcggcgaccgtattgggaactcttcgtcgtggtgagggtggtccaagccgttttctggcatcactggcggaactccatgtttcaggtggtgatgccgatttgcgtacggttctgcccgcgagccaggcggctggcttgccggaaaccgtcctgacggcgggtccgcgtggcgagagcgctgacggcgatagccgtcatgaagtgctgtgtgcacgtctggcaccgctcgacccagccgaacgccgcgcccaacttctgacagttgtgcgtgaatctgcggcggcggccttggatggcgatgaccagggaagcatcgatggtcgtcgcacctttcgtgatttgggtattacttcacttgcggcggttggcattcgtgatcgcctgcactccgcgacaggtcttcgcctgtcacctaccgtggtctttgaccatcctactccagatgcattggccgcccaccttgatacagaactgtttgggaccggggcagatgccgaaccggctccggcagccggcggccgtgcagttccacatgatgaaccgatggcaattgtgggtatggcctgtcgttacccgggtggagttggcgcaccggcggatctctggcgtactgtcctggcaggggtggatgcggtcggcccattgccagccgatcgtggctggaatatcgctgatggctacgacccggaacttgccgggccgggccgttttagccaacgcgagggcgggtttctgcacgatgcggcagagtttgacgccgaattcttcggcatctcaccccgtgaagctctggccatggatccgcaacagcgcctcgcccttgaaagtgcatgggaagcgattgaagacgcgggcttggatgcgcattcgctccgtggcagtcgtaccggagttttcctcggcctgattacccaggattatggcccgcgcgcgggcgagccgactacccgtgcgggtgccgttgaaggtcatctgtttctggggtcaacggggagtgtagcgtcggggcgcctgagttacaccctcggcctggagggcccttccctgaccattgatactgcctgcagttccagcctggtagcgttgcatgaggcgtgccaagcattgcgtacgggtgactgcgatatggcactgacaggcggcgtgacggtaatgccttctacaggcatgctggtcgagttttcgcgtcagcgtggtctgtcacctgatggccgttgtaaagcctttagtgcgtcagctgatggctttgggctggcagaaggggttggtatgcttgttgtggaacgcttgagcgacgcacgtcgcctcgggcatcgtgtgcttgccgtggttcgcggttcagcggttaatcaagatggggccagtaatggtctgtcggcaccatccggcccggcacaacagcgtgttattcgtcaagcgcttgtgaatgcgggtgtccaggcctctcaagtggacgtggttgaagctcatggtaccggcactaagcttggtgatccaattgaagcgcaggcgcttcaggccacttatggtcaaggccgcccggcagaacgtcctttgtggctcggatctctgaaaagcaatattgggcatgcacaagcagcggcgggtgttggtggcgttatcaaaatggttatggcactgcgcgagggcgtacttccccctacgcttcatgctgattgagacg

SEQ ID NO: 5 - DNA, 3423 bp, Artificial Sequence
  DNA fragment
cgtctcaggtctggcggcagacggcatggatacactccgcgatgaattgacccatcagggtgcaagcgtcgaagtcttggcctgcgatgcggctgaccgcgacgcgctggcccaagtcctcgacggtcgtgagctgaccgcggtgatccatgcggctggagtcttggacgatggtgtgctggaggcgctggacgcctcgcgtctggatacggtccttcgcccaaagatggacgcagcttggaacctccatgagctgacccgtcatctggacctcaccgctttcgtgctgttctcgagcgcggccggtgtcctcggaaacgcaggccaggcgaactacgcagcggccaacgtcttcctggacgcactcgcacagacgcgccgtaccgagtcgctgccaggtttgtcgctggcgtggggtctttgggcagatgactccgccatgacggccggattgacagaagcagacgtgcgtcggctgagccgtagcggggctggcgccctgagtgccgacgaaggtctggcgctgctcgacacggcagccatggctgttcatcacggtttgctcatcccggttcgcctggacttggcagcgttgcgtaccgctaacgcggcccctgaacgcgtaccgcagattctgcgcggcctgcttcctacccctgcacgttctcgcaggcgtgctgcaggcgcggccaccggcaccgccgcagacggaggggaactggcgagcaccctggcgcccctggacgcgcctgcccgtgccgcgcacgtgctcgatcttattcggagcgcggtagcgtctgtcctgggtcatgcgtcgccagacgccgtcgagccggagaagtcgttccgggacctgggtttcgactcgctgaccgccgtcgacctgcgcaaccgtttgaccgccaccacgggccttcgtcttccagcgacgctggtattcgactaccctaccagcgcggctctggcggagcatgtgatgacccaagtcgtgggtgaagcagaccgtgtaacgacactggtgccggctgaagccggtgccgacgatccaattgtcatagtcggtatgtcgtgtcggtatcctggtgacgtgatgacccctgaagatctctgggacttggtgctttccggtggagatgcggttagcgaattccctagcgaccgcggctgggaccttgaaaacgtataccatcccgatcccgaccacccgggcaccacgtactcgcgcgagggcggtttcctgcaccgcgcagcggagtttgacgcggaattctttggtatatctccacgtgaggctttggcaatggacccccaacagcgtctgctgttggaaacctcctgggaggcgttcgaacgcgccggaattgatccagccaccctgcgcggttcccgcaccggtgtgttcgctggtgtcatgtaccacgattacgcatcccgcctgcgcgaggtccctggccacatggaaggattgctgggtacgggcaccgcagcgagcgtcgtgtccggacgcctgagttacaccttcggtctggagggccctgctgtcacggtcgataccgcttgtagctcctcgctggtggcactgcatctggccgtccaggccctgcgcgccggagaatgtgagatggctctggccggtggcgtgaccgtgatggctaccccaggagccttcatcaacttcagtcggcatcggggcctgtcgcctgacggtcgctgcaaggccttcgctgccggcgccgacggcacgggttgggcggagggtgccggtatgctcttggtcgaacggctctcagacgcggaacggttgggacatcgcgtcctggctgtcgtgcggggttcggcggtgaaccaagacggcgcatccaacgggttgaccgcgcctaacggtccgtcgcagcaacgcgtcataaggcaagcgttggctacagcgggccttacgcccacggatatcgacgcggtcgagggacatggtaccggcacctcgttgggtgacccgatcgaagtgcaggccctgcaggctacatacggacaggagcgccccgcggagcacccgctctggctgggtagcctgaagtcgaacatcggacacgcacaagccgcggccggcgttgggggagtcataaagatggtcatggcgctccgcgagggtgtcttgccacgcacgttgcacgccgatgaaccgtccccacatatcgactggaccgctggaaacgttaggctgcttaccgagcaaagcacctggccagacacccaacgcccccgtcgcgcggccgtgtccagtttcggattctccggcaccaacgcacacgttatcatagagcaagccccagacccggcccatccagctgacaccgccgacaccaacccgggcgacgagtccgtagtcccatgggtcatctcgggtgcgagcccccaggcgctgcgtgctcaggctgagcagctccggtcctatatagcagaacgtccaggcctcagacctgcagatgtcgcgttcagcttggcaacgacccgcggcgccttggaacaccgtgccgttgtcgtgggtacggacttgtccgagctggcagaaggcctcggtgcgctgacccagaccgcgaccgccgtgcctggtcgcaccgctttcttgttcaccggccagggcgcgcagcgcgtcgggatgggtcgcgagttgtacgacaccttcccagcctttcggaaggcacttgatgaggtctgtgctgtgctcgaccccctgctccctcgccccagccgggaagtaatgtgggatgaggaccccgaggcgttgtcccgcacggaattcacgcagcccacgcttttcgcaatcgaggttgcgcttttccggttgctggagagctggggtattcaccctgacgccgtggcaggccattcgattggtgagatcgcggctgcccatgtgacaggcgtgctgtcgctgaccgatgcttgtgtcctggtggcggctcgcggccggttgatgcaggcccttcctcatgacggagtcatgattgcggtgcaggcaacggaagacgaggtccttcctctgttggaaaaggtgaccggccaagcggacattgccgcggtgaacgccccagaagcagtggtcgtgtccggggctgaaaccgaggtggaacatgtcgcgggcattctcacagcccaaggacggcgtgtcaagcgcttgaccgtgtctcacgccttccattctccgctgatggatccgattctgaaggatttccaaaccgtggtcgagggcttgtcctttcggcaaccatccttgccattcgtgtccacggtcacgggaaccgtggcgggcgcagaaataaccgagcccgcatactgggtcaggcacgtacggcaaaccgtgcgcttcgctgacggtctgcgtacgttgcacggcctgggcgtgcgcaaattcatcgagatgagacg

SEQ ID NO: 6 - DNA, 3462 bp, Artificial Sequence
  DNA fragment
cgtctcaggaatgttgctggtcgaacggctgtctgacgcgcagcgtctgggtcatcccattctggcggtggtccgcggatccgcggtaaaccaagatggtgcaagcaacggcctgaccgctccgaacggccccgcacaacagcgtgtgatccgtcaagccttggccaccgccaggctcgaggctggtcaagtagatgtcgtagaggcgcacggcaccggaacctccttgggcgacccgatagaagctcaagctctcatggaaacctacggtcaagagcgcccggctgagcggccactgtggctgggctctttgaagagcaacattggtcatgctcaggccgcggccggtgtcggtggcgtgatcaagatggtgatggcgttgcgggaaggtgtgctcccgcgtacccttcacgcggatgaacctagtccccatatcgactggacggcgggtgcagtccgtttgctgaccgaacaatcagcatggcccgacacccagaggccgcgtcgggcagcggtgtcttcgttcggtttctcgggtaccaacgcacatgtaatcatagagcaggcgcctgacccagcccaccctgcagacacggcggacacgaacccgggcgacggaagcgtcgtaccttgggtaatctcgggtgcaagcccacaggcactgcgtgcacaagcagaacagctgcgctcctacatcgcagagcgccccggattgaggcctgcggatgtggctttctctctggctaccacacggtctgtattggagcatcgggcagttgtagtcggtgccgatcacgacgatctgttggacggtttgggtgagttgagcctgacgggcccggtcgtggaaggtatgagtgccttcctcttcacgggccaaggagcccagcgcgtcggtatgggtcgtgaactctacgacactttcccggcattcaggaacgcacttgacaaggtatgcgcagtcctggacccgctgttgccacgcccaagtcgtgaggtgatgtgggacgaagatccagaggccttgtcccgcaccgagttcacgcagccaaccttgttcgcaatcgaggtggcattgttccgtctgctcgagtcgtggggtatccatccggacgccgtagccgggcactcgataggagagatcgccgcggcacacgtgaccggagtgctcagcttgacggatgcctgtgtactcgtggccgcgcgtggtcgtctgatgcaagccctccctcatgacggcgtcatgattgccatccaggcgacggaggacgaagtgcttcccttgctggagaaggttacgggccaggctgacatagcagcggtgaacgctcctgaagccgtcgtgatctcgggtgctgaaaccgaggtggagcacgtggccggtatcctgacggctcagggccggcgcgtgaagcggttgacggtgtcgcatgctttccatagccctctgatggacccgatattgaaggacttccagacggtagtcgagggtctgtctttccaccaaccaagcctgcctttcgtcagcaccgtcaccggcaccgtggcgggtgcggagattaccgagcccgcgtactgggtacgtcatgtccggcagacagtacggttcgcggatggtttgaggactctccatgaattgggcgtccggaagtttattgaaattggtcccgacgcgatcctcaccggtctggtggaacaaactctggatacgcaagctgtgcccgtgttgcgccgggatcgggacgaggtgcgggctgcagtagaagcagccggcggattctttaccaggggcggtagtgtcgactggccagcccttctcgcgggcggaagacgcgtggacctgccaacctatgccttccagcacgagcgttactggttggaggcccccgtgtccgtcggcgacgtcgcagctgtcggcttgagcgctgcacgacaccctctgctcggtggcgcaatcacgctggctgatcgctcgggcgtgttgctgacggggcggctgtcgctggctacccacgcctggctcgcagatcacgccgtccattctaccgtgctgataccgggaacagcactcgtcgagctcgctctccgtgctggagaagaggttggatgtgacaccgtcgaggaactcacgctccaagctccactggtcctccctgctacaggtgcccgcgccgtccaagtgcagatcgttgtgggcgagccagatgcacgtaacctgcgcccggtcgacgtttacgctcgggtagaggacgataccggtgaggccccgtggacatgtcaggcgaccggcctcctggctccaggtacaggagccccggaagaggcgaccgatttcgcagtctggccccctcgtgacgctgagcctgtcgacattggaggcttctatgatgctatggccgacaggggttacgactacggccctgttttcaggggactccgttccgcttggcgccggggtgatgaagtgttcgccgaaatcgcgttgcccgaagaggccgctggtgccgctagggaattcggagtccatcctgccctgttggattccgccttgcacgccgcaacggcggcaaccgacgagcatggcgacgtgacccgggtgcccttctcctggcggcgagtcgcgctctatgcggcaggcgcaaccgcactgcgggtgcatctgacgtctgccggtgaaacgctgaccctgcgtgccgctgataccgaaggacagctcgttgctagcgttgaaagcctggctttgcgcgaagtctcgccggagcagttggcggtcgcggacgatccagactcactcttcgaagtagaatgggtatccgcggctgacggaggctcaaccgaggctggcacggcgtcctgggctgtcctgggagactcccccctcgctgaaggtggccccgtgttcgctgacgtggaggccttggtagcgtcatctcaagatcttccgggcaccgtcgtactggagtgtccagcagtggaaggagcgccagtgcccgacgcagtgcgggaccgtctgacgggtgtgctgagtgtgttgcaacagtgggtggctgacgagcgtttggcttccagccggctggtggtagtcacccgtggcgcagtggcagcttccgccaacgaaccagcagacgttcgcgtcgcgcctgtctggggtttggtctgtgcagctcaggcggaacaccccgggcgattcgttttggctgacttgccggtcggcgccggagcacgggagttgagcgccggtctggcctgtgatgaaccgcagtgggctatccgcgatggcgctgtgcgtgtacctcggctggtgcgggcccaacccgccgtgtcgggagttcccgcgtttggtaacggcccagtgctcgtcaccggcgctacaggtgctctgggtaagctcgtggcccgtcacctggtatccgtccacggagtccgggaacttgtcctgttgagccgtcggggtctgagacg

SEQ ID NO: 7 - DNA, 3414 bp, Artificial Sequence
  DNA fragment
cgtctcaaagcgacgcagtcgttcaaggagctgggattcgatagtctcaccgctgtggatctgcgtaaccgtctgaccgccgctacaggtctgcgcttgccggcgaccttgatctttgaccatccaacaagcgctgcactcgcagaccgggtgctgaacgacctggtggacgattcggccgaaaccccggccgactcggcacgtaccgcggtcatggcctcatccgaaccagtcgcgatcgtgggcatgggttgccgtttcccaggtggagtggtttctccggaaggcctgtgggaagtggtactctcgggcgccgacgtgatctccgaattccccaccgatcgtggatgggacgtcgaaggactttacgaccccgatccggaccgtcctggcaagacctatggcagacgcggcgggttcgtggacgcggtcgccgacttcgatgccggttttttcggcatcagcccgcgcgaagccctggcaatggacccccaacagcggctgcttttggaaaccagttgggaggctttcgagcgcgctgggattgatccagccacgctgcgtggatcccgtaccggcgtctttgccggcgtcatgtaccacgactatgcgtcgcgcctgcgtgaagtgccgggtcatctggaaggactgatgggcaccggcaacgccacctccgtgatagcgggtcgtctgtcttacaccttcggcttggagggtccatcagtctccgtggataccgcttgtagctcgagccttgtcgccctgcacctggcggtgcaagcgttgcgagctggcgaatgcgagatggccttggcgggtggcgtgacggtgatggccacccccgaagccttcatcaatttctcccgtcaacgtggccttgcgaccgacggaaggtgcaaggcttttggagcgggcgcggatggcacgggttgggcggagggtgccggtatgctccttgtggagcgcctgtcggatgcgcaacggctgggacatccgatcctggcggtggtacgaggatcggcggtaaaccaggatggagcgagcaacggtctgaccgcgcctaacggtccatcccaacagcgcgtcatccggcaggctctggcaaccgcaggtctgggtccaaccgatatcgacgctgtagaaggtcatggaaccggtacctcgttgggcgacccgatagaagttcaagccttgcaagccacctacggtcaagaacggccagcagagcgccccctgtggttgggctccctgaagtccaacataggacatgcgcaggcggcagccggagttggtggcgtgatcaagatggtaatggccctgcgcgagggagttctgccgcggacccttcatgcggacgagccttccccacacatagactggaccgcgggtgcggtacgcttgctgaccgagcagtccgcttggccggacacagaccggccgcgcagggcagctgtatctagcttcggtttctcgggcaccaacgcacatgtaattatagaacagccctcggaactggctgaccctgcggacacggatccgcgtgaccgtagtgtagtcccctgggtaatttccggcgcgtcgccccaggcactgcgtgctcaggcagagcagcttcgttcatacatcgcggaacggccgggcctgcggcctgtcgatgtggccttctccctggcaaccacgcggagtgtacttgagcatcgcgctgtggtcgtaggcgccgaccacgatgacttcctgacagcgctggacacgccgaccgaaacgaccgatacccccacgggccgcattgcgttcttgttcacgggccaaggtgctcagcgggtaggtatgggtcgggagctctatgatacctttccagccttccgcaacgctcttgataaggtgtgcgcggtgctggatccgctcctgcctcggccttcacgcgaggttatgtgggatgaagaccctgaggctctctcacggacggagttcacccagcctacactcttcgctatcgaggtggcattgttcaggttgctggagtcttggggcattcacccggatgccgtcgcaggtcactcgatcggcgagatcgccgcagcccacgtgaccggtgtcctgtcgctgaccgatgcgtgcgtgctggtggccgctcgaggacgcctgatgcaagcgttgccccacgacggtgtcatgatcgctatccaagccacggaggacgaggtgcttcctctgctcgagggcatcaccggtcaggcggacattgccgctgtgaacgcacccgaggcagtggtcatctctggcacggaaaccgaggtggaacacgtagcagggatcctgacagcccaaggacgcagggtcaagcggttgaccgtgtcgcacgctttccattctcctctgatggaccccatacttaaggacttccagaccattgtcgagggtttgagcttccggcaacccagcctcccattcgtgtccacagtcacgggcaccgtagcaggagcggaaattaccgagccggcgtattgggtccgtcacgtccggcagaccgtgcgcttcgccgacggtctgcgcgcccttcatggtctgggcgtgcgtaagttcatcgagatcggaccggatgcgatccttacaggcctggtggaacagaccctcgacacccaggcggtgccagtcttgcgccgagatcgcacggaagtgcgtgccgcggtcgaagccgtgggccgcctgcacctggcgggaatccctgtggattggccggcagtgctgccgggcgcccggagagtcgaactcccgacatatgctttccaacacgagcgttattggctcgaggaaacggcgggtgctggcgatgtgacggccgcaggcttgcagggtgcccgccatccgctgttgggtgctgcgatggagctcgccggtagcgatcgtaccgtctttagcggtcggttgtccgtggcctcacatggctggttggccgaccacacagtcggcggtgtcgtgttggtgccgggtgcggccctcgtggagctggcgttgcggaccggcgacgaggtaggctgcgaccgcctcgaggaattgacactgcaagctccgctggtcctgccggagacaggagcggtccagttgcaagtgtccgtgggagaggcagatgccgaaggccgccggacagtcgaaatacacagccgccctcatgatctggccggtgccaccacagctgagtgggcggcacacgccgacggagtcctggccgtggcagacgccgctccggacaagcacgacacgccgtggcctccggcccgcgcaacctcagtggacgtgtcggacgtctacgacacgcttgcagataagggcctggtgtatggtcccgtattccgcggtctgcgtgcggcctggcgtttgggcgacgaagtcttcgcagaagtggcttttgagacg

SEQ ID NO: 8 - DNA, 3465 bp, Artificial Sequence
  DNA fragment
cgtctcatggacgcagtctgtgcagttctggacccgttgctggaacggccgcttcgagaggtaatgttggccgcaccgggtacgacccaggcggaagccctcgacaccacaggttgcacacagcctgccgtcttcgcccttgaagtagctctcttccgtttgcttgaatcgtggggaatacggcccgatttgcttgctggccactcaataggtgagatcgccgcagctcacgtgtcgggtattcttagcctcgaggatgcctgtaccttggtcgctgcgcgcgcgggtctgatgcaaagactgcctagcggtggcaccatggtcgccgtcgaagcggatcctgacgaggtgttgccgctccttgccggtcatgagcatgaggtgggcctggccgctgtaaacgctcctggtgcggtggttctctcgggagctgacaccgcggtacgtgaaatagtagccttgctcaccgagcgtggccgtcgcacaaagagactgcgggtgtcgcacgcattccacagccctctgatggagccgatgttggacgagttccgccgtacccttgcccgcgttaccttccgggagccaggaatcccgatcgtgtccacggtaactggagcgaccgatccggaggaaatgcggacagctgattactgggttacccacgtccgggccacagtccgtttcgcggacgcagttaccgctttgcacgctcagggcgtgggtcgctgggtcgaggtcggcccgtcggcgacgctgctcccagtaatacaacagaccttggacgtaatggacggtcccgacggcagcgccggtccagcgggcgacggtggcgcggcagtcgtagcgccggtcgggtccgacgtggtcgtatctgttctgcgccgtgccgaaccagaagagaaggcattgctgaccgctgtatcgcgcctccacgctgccggaacgtcggtagactgggctgccgttctggaaggtctgggtgctcagcgggtggacctgcctacctatgccttccaaagacaacgttactggctggacgtgcctgccggtaccggagacatgagcgcagtaggactgggcgcagctcaccatcctttgctcggcgctagcgtggcgctggccgagggagatggagtcttgctcaccggccaattgtcgccagcggcacagacctggctgaccgatcatacggttggtggcgcgacattggtacctggcgcggcccttgtcgaattggccttgcgggccggtgacgaagtgggttgcggcagagtggatgaccttaccctggaagcccctctcgttctcccaccggagggcgcggtccaggtgcaagtcaccgtgggtgcgcctgatgagcgcggcgctcgcccagtccatgtgtattcacggccacagccagacccacgccatcctcggagcgcagacacgggctggacgcgccacgcgacgggcttgctgaccccaggcacccctgccctcgccccttcggacgattttacagcctggccaccccgcgctgcggaacccgtgggtatcgaaggtttctacgaagatcttgccgaccgcggttatgaatacggtcccgcgttccaaggtctgttgcgcgcgtggcggaggggtgaggaactgttcgcagaagtcgccctgcctgagcagcaagcttctggcgtgggtggcttcggcctgcatcccgctttgctggacgcagctctccatcctataggtctgacatccttggtggcagacggcgcgacccgtttgcctttcgcctggaccggcgtaaccctgcacgccgtcggagcaacagcgcttcgtgtacgcatagcccccacgggtcccgattcgttctcggtcaccgcagccgaccccacaggtgccccggtcgccgctgtcgagagcttgaacgtccgtgaagtgtcacgtgaacaggtgatcgccgcgatgggccccgcggccaccggagtaggcaccgactcgctcttcgaagtagaatgggtggcggcagctgacggtggctcggcggaagcgggtgccgcgtcgtgggcagtcttgggtgattccagcctggccgagggaggcctggtgttcgcagatgtcgaggccctggtagccagctcacaagatctgccgggtacggtcgtgttggaatgtccagctgtggagggcgcgcccgtgccagatgctgtgcgtgaccgtcttaccggcgtcctcagcgtgttgcagaggtgggtcgctgacgaacgtttggcatcgtcccgtcttgtagtggtcacgcggggtgcagttgcggcctccgcggacgaacccgtcgacgtgcgcgttgccccggtttggggtctggtcagggctgcacaagcggagcatccaggtcgtttcgtgcttgcagatctgcctgccggcgcaggcgcccgcgaactggcggcaggtctggcctgtgacgagccgcagtgggccatccgcgacggcgctgtacgcgtacctcgcttggtccgtgcgcaggcagccgtgtccggcgtgcccgccttcggtgatggccccgtacttgtaaccggcgcaagcggagctttgggtggagtcgtggctcgccatctggtgagcgtccatggcgtgcgggaactggtgctgttgtcccgtcggggcttggctgccgatggaatggacaccctgcgagatgaactcacgcatcagggcgcttctgtcgaagtactggcttgcgatgccgcagatcgcaacgcccttgcccaagcactgagcggccgccggttgaccgcagtgatccatgccgcgggcgtcctcgacgatggcgtgttggaagctctggatgcgtcccgcttggatacggtccttcggccgaagatggatgcggcctggaacctgcacgagctcaccagggaccttgatttgaccgcatttgtactgttctcctcagcgaccggcgtactgggtaacgcgggccaagccaactacgcagctgcgaacgttttcctggacgcgttggcacagacccgtcgcaccgagggtctgcctggtctgtcattggcatggggactctgggcggaggcttccgcaatgaccgccggcttggcagaaaccgatcgtcacaggattgctcgcctgggcgccgaacccctgaacgaaaccgaagcgctggcgcttctcgaccgcgcgctgggcgaagatgctcccggtctgttggtccctgtacgtctttctcggccagcgctccgggctcaagcgcaggctggtacgctccccatgctgatgcgcgcgctggttccggctaccgtgcgccggcatgcagccgctggcgccgcgggcgtagtcgccggtggcggtgccctggcggatcgccttattggtctgtcggctaccgaacgcgaagagcacgtgcaggacctggtgcggcgtgaggtggcgggcgtactgggccatgccacaccagatgcaattcaagctgagacg

SEQ ID NO: 9 - DNA, 3403 bp, Artificial Sequence
  DNA fragment
cgtctcaacatcaacgatactggttggacagcacgaccggatccggtgtcgatgtgggcgcggccggtttgggcgcggcccggcatcctctgttgggcgccgcagtagcattggccggcaacggtgggaccgtgctgaccggcaggctcagcctcgacacccacttgtggctcgctgatcacgccgttaggggtgtcgtactggtgccaggtacaggcttggtagaactggcagttcgtgccggtgacgaggtcggctgcggtttcgtggaggaattgaccctgcaagctccattggtcctgccccctgagggagctgtccaggtccaagtggtcgtaggtgcggcagacgatgccggtgtgcggtcggtcgacatctatagccgtccagaagagcccggtgtcgatggcccttggaccctccacggcacgggtaccgttacgcctggcgcctctgaaccagccgatggtcgtgccgacctcacggtatggcccccacgcgatgctcaggtactcgacacggacggtttctacgaaacgatggccggtcggggctacgaatatggtcccgcattccagggtctgcgtagagtctggcgcaggggcgatgaggtcttcgctgaggtggccttggcagaagagatagctggtgccgcgggagagttcggactgcatcccgcgcttgccgatgcgggtctgcaggcgggacttctgaccctgttcgccccagccgacgatggtgcgaccggtaaccgcttgccttttagttggcgcggcgtggccttgcatgccgtcggagcgacaacgttgcgagttcgcatggcacccgtggctggcgaccccacgaccgtgacgttggacatggccgatgccagcggcgccccagtcgcaagcgtcgacgtccttgctacacgcgaagtctccgaggctcaattggcggccgctgcccccggagccgacgatagcctctttcgcgtggaatggctggcgaccgctggaggtggctcagtggaagcggtgtcttgggccgtgcttggtgactcaccgctgggggacgggggactcgcgttcgcagatgcagacgccctcgtagcgtcgagcgctgacttgcctgataccgtcgtgttggaatgtcctgcaggcgagggagcaggggcagtaccagaagtcgttcgcgcacgtttggccgaggtcttgggcgttgttcagcgttgggtggcagatgagcgtctggcaagttctcgcctcgtggtagtgacccgtggggcggttggcctgcgcgcgggtgagactgtcgatgtgcgtgtggcgcctgtctggggcttggtgcgcgcggcgcaagcggagcacccggaccgctttgttctcgcggacctgccggcgggcgctggagcccgtgaacttgcggccggcttggcgtcccgtgaaccacaatgggcagtccgtgatggtgtcgttcgcgttccccgtcttgttcgtgcccaagcgccggcgggtgaggcaccgggttttggtgacggacccgtattggttactggcgccagcggtgttttgggcggtatcgttgcgcgtcaccttgtatcagcgcacggcgtgcgtgagctcgttctggtttcgcgccgcggaccggcagcggccggcatggatcgtttggaagccgaactggtcgcccttggggcaacggtcgaaagtattgcttgcgatgtagctgatcgtgatgccctggcacgcgttctgacaggacgtcgcctcaccggtgttgttcacgctgcgggcgtcttggatgacggggtccttgagagtttggacgaggcccgttttgacacggtgttgcgcccgaaagtggatgcggcgtcacatctgcatgagctgactcgcgatcacgagctgagtgcgtttgttctgtttagcgctggcgccggcactctgggaaatgcaggccaagcagggtacgcagctgcgaatgttttcctggatgccttggcccaagcacgtcgtgcggaaggtcttccgggcctttccctggcgtggggtctttgggctgagactagtgctatgaccggtcgcctgggcgagactgaccttaatcgcctggcgcgtctgggcgtgacggcaatggagactggccaagcactcgccctgttggatgccgcggcccgtactgatgaaccttacctcctgccggtgcgcctggatctggcggcgctgcgccgtcgtgcggccgtatctggtgtgcccgcgctcctttccgcactcgtgccacagcgtgttcgccgtcaagcgacgggaactggtgcaggggcggcgtcggccgatggtggcgatttgggcggtcgcctggcggcattgccggccgatcgccgcgaagagttcttgctggatctggtccgtggcgaggttgctgcagtgctcggtcacgccagcccggatgccgttgagcccgaacgtgcttttaaagatctgggttttgatagtctgaccgccgtcgaactgcgcaatcgcttgggcgcagcgacgggcctcaggttgccagctacactggtgttcgatcaccccaacgccacagcagtggtaagactgttgtggtcggagctgggtggcgctggcctggccggtgacgcgagcgccactcggccgtccacgcccgctgccgctgacgaaccaatggctataatcggcatgtcctgccggttcccgggcgacgtggaatcgcccgaagacctgtggcgcctggtggcagaggcccgggacgccatcgacgtcatgccaggcgatcgcggttgggacgtggacgctctttacgatccaacgcctggtgtgccaggccgcatctatagcagggagggcggtttcttgcggaacgccgcggaattcgatcctgcattctttggcatcagcccgcgggaagccttggcgatggaccctcagcaacgcctgctccttgaaacatcctgggaagccttcgagcgcgcgggcatcgacccagctaccttgcgtggctcccgaaccggcgtcttcgcgggagtcatgtaccacgactacggctcgcgactgggcgcgggtaccgtgcccgaggacgtggagggatacgtgggcaacggatccgctgggtccatcgctaccggccgcatcgcatacacccttggtctggaaggtccggctgtcacggtggacaccgcatgctcatcctcacttgtcgcgatgcatctggcaatgcaggcgattcgccagggcgaatgctcattggctctggtcggcggtgtcacggtgatgtcctctattgaaatgttcctcgagttctcccggcaacgcgcggtgagccctgatgcacgttgcaaggcctttggcgctggcgctgatggtgctggtttctccgaaggagccggaatgctgttggtgagacg

SEQ ID NO: 10 - DNA, 3435 bp, Artificial Sequence
  DNA fragment
cgtctcagagattggccctgatgctatacttaccggcctggtagaacaaaaccagaccctcgacacgcaggccgtacccgtactgcgccgtgaccgggacgaggtgcgcgctgcagtcgaggctgtcggtcgcctgcacctggcgggcatccccgtggattggccggcggtccttcctggtgcccgccgtgtcgaactgccgacctacgcgttccaacacgagcgctactggctggacccagaggaactggcggctgcagccgaggacaccgttgcaccttcaggtacggaagtccccgaccccgatacccgcttctggggcgccgtcgcagacgaggatttgggcagcttggcagcgctgcttggtatagacggagaaaagggaggtgctcaggaccgcgcggctgtggaagcggctctgcctgtgctggcttcgtggttgggccgccggcaggctgcggcacgcgtgtcccactatcgggtgggttggacgccagtcgctagacggcctgacggcacgacagcgcggttgcggggtatctggctgttgaccattcccgcacgcataggcgccgacgatgcgttggtgactcgtctggcaagtgcattgggcggtgccggagccgacgttcgtgtggttacggttggtgatccgggagcagattcgtatgacgatctggctgccgaagtttcgtcgttgaccgccgacggcggtgaactcgccggcgtcctgagtctgctgggattggcgtctgctgatggtcccggggatgcgcgtgaggccgcagtaggtacactcgccctgctgcgtgcgctctcgggttcggttgcatcagtccctgtttggtcactgacatctggtgccgtatcgaccggcggatcagagcgtgtaagcgcccctgcccaggctgtgctctggggactgggtcgcctgctggccgaagacagtgatgtgcgttgggcgggcgttgtggatgtgccggcgccgtgtggtgatcgtgtgttgcgccgcctcgccgaagtgctcgcaaatccagccgaggagactgaagtggccgtacgtgacgctggcgtgtttgcgcgtcgtcttctgcgtgcaaccggggcagcggacgggcccgcccgtcctactgctcttgctccccgcggcaccctgttggtatcaggcggttcagatacatggcgtgatcgtgttgctcgccgtctgcttgcatcgggcgcggcacatgtgttggtcgcgacagcgccagatgagccagaacctgcttctaccccggggtcggcggttaccggggtttcccgtgtcgtgtgtgacgtttctgacggtccggctctggcgcatttggccgccagcctgccggcgggccccgacggccgtccgctgacgggtgtagtgcacgcgcccccggcaacagccagcgatggacccttggataaggcactggatgaggtattgggtgctggactgccggcgctggcaggcgtatcatcgaccgctggcccgatcgccctcttcctggccgtggatgttgatgacctggttggcgccccgggagcaggcgccgtcgcggctctggccggttggtgggaagccgccgcacgcgtacgtacggccgaccgcgcacctgtacgcctgattgcggcagatcccgatgcactggatctggccgtgttggatcgtgcaatggaacgtgccgatggtctgctcgtcgtgacgggtcgtgattgggcacaatacgcgggaacccacgcggatacccgcggtcgccgcttgctggaaggagtgcctgaggcacgtgcagttcttgcagcagcagcccctgcgggtgacgcgggcaagagcgggctgttggctggtgtagacgggccggaatcgttgcgtcgcgtgttggcggcgcgcgaagcagaccacaagctcgcgaccctggtggagctggtgcgcggtcaagtcgcggtcgtcctcggacacgcgagtgccgatgcggtcagtgcggatggagactttatggatctgggatttgcttcgctgacagccgttgagtttggccaccgtttaagcgccatcacaggcctcaaattgcctacgactctggtctacgaccacctgaacccagtggaactggccgagcacctggctgacgagctggcgagggaactgaccgccgcgtgatagcataaccccttggggcctctaaacgggtcttgaggggttttttgcaaacattccgagaccatgtcgatactgaacgaatcgacgcacactcccttccttggctgctccttcggtcggacgtgcgtctacgggcaccttaccgcagccgtcggctgtgcgacacggacggatcgggcgaactggccgatgctgggagaagcgcgctgctgtacggcgcgcaccgggtgcggagcccctcggcgagcggtgtgaaacttctgtgaatggcctgttcggttgctttttttatacggctgccagataaggcttgcagcatctgggcggctaccgctatgatcggggcgttcctgcaattcttagtgcgagtatctgaaaggggatacgcatgcagtccgcagaaaaggcaaagcctgctgatggcgccgcagcggcattgctggcaaccctcacccataaacggcgtctggacgcggccaccccgaaggaaagcgcactgtggttgctggaccgcctgctccctgaagcgggtgtaaacaatgttccactggccgtccgcgtcgatggtcgtctggacgccgcggctttgcaagcagcggtcgacggtctcgtgcgccgtcacgaggtgttgcgcaccgtatacctggatcggcaggccggtctggtgcgtgaagtgctgggagaggacaccccaggaccgcgcgtggaggtccatgacacggtggccggcgtcccggagaaagccttgcgtgaattcgccgctacaccgatccggtgtgacggccggctgatgctgcgcgcagcggtgttccgcggtccggatgctgacaccctcgcggtcgttgtgcatcacctggtgttcgacgccgcttcggtacctgtactgatcgccgaacttgccgctgcctacgacgcaagagccaccggtcgtgacttgcctgatgaactgcgcaccccggtcgcggcattgcgggatcccgcaccccgtgaggaatccctggcatattggcgcaccgccctggatggtttcgacccagcgggactggacctcgattgcgcacggcccgccccagcgcgtgcgaccctcgtgggtgacaccgttcttcacgtccttgacgatgaaacccgtgacctggtccggggcctgcagcgaacgcaaagagcaccagaagctgttatcctgttcacggcattctgtctgctcttggcagctcacggtgcgggtccagatttggtcgtgggctccccggtgaacatatgagacg

SEQ ID NO: 11 - DNA, 3399 bp, Artificial Sequence
  DNA fragment
cgtctcactttgccagaggaagcggctaacgcggctgacgcattcggtctgcaccccgcgcttctggatgcagccctgcacgccatcggcttgctgcaattggctgactcggagggaatgcgtctgccattcgcttggagtggagtttcgctccaagctgtcggcgctaccacgcttcgcgtgagaatcgcccccgacggtcgcggtggagctaccgttgacctgttcgacgaagcgggcctgcccgtcgccagggtcgagagtctgacccttcgcgaagtctcgcgcgagcagatggcggccgcggcctccgcggccggcgacgagtccttgttccaggtcgaatgggtaccggtggttggcgatcccgatgaagctgtgtcctgggccgtgctcggcgactcgccgctggcagagggcggattggtcttcgctgatgtagaagccttgctggccagctcccaggacctgccaggtacagtcgtgttggaatgccctgcagttgaaggtgctccagtgcctgatgcagttcgcgaccggctcaccggcgtgttgggcgtcctgcagcgctgggtggctgatgaacgactggcctcgtcccggttggtcgtggtcacgcgtggtgccgtcgccgcgagcgccaacgaaccagcggacgtccgcgtcgcgcctgtatggggcctcgtccgggcggctcaggccgaacatccggaccggttcgtactggcagatttgcctgcaggcgccggtgcccgcgagttggccgctggtctggcttgtgacgaaccgcagtgggcgatccgcgatggtgcgatccatgtaccacgtctggttcgcgctcaagactctaccgacggagcctccggtttcggcgatggccccgtcttgatcaccggagccagcggcgcgttgggtggagtggtagcgcgccacctcgtaagcgtgcacggtgtgcgtgaactcgtcttgctttcacgtaggggcctggcggcagagggaatggatacgctgcgggatgagctgacccaccaaggcgcatcggtcgaagtgctggcatgtgatgcggctgaccgcaacgctctggcacaggcgctgtcaggccgccggctgacggcagtgatccacgccgctggagtcttggacgatggtgtcctggaagccctggacgcctcacgcttggataccgttcttcggccgaagatggacgctgcctggaacctccatgaactcactcgacaccttgacctcaccgccttcgtattgttctcgagcgctaccggtgtactcggcaatgcgggccaggccaactacgcagcggcaaacgtattcctcgatgccttggcacagacgcggcgcacagaaaacctgcccggccacagccttgcttgggggctctgggctgaggcttcagccatgaccgccggactggcggagactgatcgtcataggatcgcgcgcctgggcgctcaacctctgaacgaggctgaagctctggcccttctggacaaggccgtgaccggtgatggcgaaggtctgctcgtacccgtgcgtttgaacctcccggcactccgcgcacttgcggattccggtcgcctccctgccctgctttccggcttggtccgcacccggccccgccgtgctgcagaaaccaaggccggctcgggtgtgggtctgcgcgatcgcctggccggtatgaacgaagctgaggctgagagacatctggtccgcctggtgcgctcggaagtggctaccgtactgggtcacgcgtccccggacgcggtgggctccaagcgatccttcaccgaactgggtttcgactcgttgacggcggtcgaattgcgcaaccgtctgacagcagccaccggtctgcggctgccggctaccctcatatttgaccacccgaatagcaccctcctggccgaacgtatacggctggagatactcccggagggtgcagcgacggaattggacgatcctgaagagaacgcgttccgcgaagcagtttcagctatacctatgtcacggttccgagaagcaggcctgttggatgtggtcttgcagctcgcgggacctaagcggcagcaagaaacggcggtcgagggcgaagaaaccgagtcgatcgacgagatggatgtagataaccttattcggatggcactggacgggaaagactcctgatgacataaccccttggggcctctaaacgggtcttgaggggttttttgaggactagatgagaccgcgcagatgtacgacaatatcgcttagtcacccttgggccgctgctccttcggtcggacgtgcgtctacgggcaccttaccgcagccgtcggctgtgcgacacggacggatcgggcgaactggccgatgctgggagaagcgcgctgctgtacggcgcgcaccgggtgcggagcccctcggcgagcggtgtgaaacttctgtgaatggcctgttcggttgctttttttatacggctgccagataaggcttgcagcatctgggcggctaccgctatgatcggggcgttcctgcaattcttagtgcgagtatctgaaaggggatacgcatggcgaccccaaacgagaaagttgtggaggctctgcgcgcctccctcaaggaaaccgaactccttcgtcaacagaacaatgcgctccgcgcggccagctcggaaccagtagcaatcgttggcatgggctgccgcttccctggaggtgtggtatcccctgaaggtctctgggaagtcgtgttgtccggtgccgacgtcatctcggagttcccaaccgaccggggttgggatgtcgaaggtctgtatgatcctgacccggaccggcccggtaagacgtacggtcgccgtggtggattcgtcgacgcggtagcggacttcgatgccgggtttttcggcatctcacctcgggaagccctggcgatggatccacagcaacgtctgctcttggaaactagctgggaggcgttcgagcgcgccggtatcgaccccgcaaccctgcgcggatcgcggacgggtgtgttcgccggtgtcatgtatcatgattacgcgagcaggctgcgtgaggtacctggacaccttgaaggccttatgggcacgggcaacgccaccagcgtcatcgcgggtcgcttgtcttataccttcggactggagggcccgagtgtttcggtggacaccgcctgttcctcgagtctcgttgccctgcacctggctgtgcaagccctccgggcaggggaatgcgagatggccctcgcgggcggagtaaccgtgatggcgaccccagaggcgttcatcaacttcagtcgccagagaggtctggctgcagacggccggtgcaaggcgttcggtgcaggagcagacggcacgggttgggccgaaggagctggaatgagacg

SEQ ID NO: 12 - DNA, 3438 bp, Artificial Sequence
  DNA fragment
cgtctcatactgctttcgcggcgcggtccatccgccgatggcatggccgaagtccaacgcgagttggctgaagctggagcgtccgtagaagtactggcgtgcgatgctgcggaccgcgacgctttggcccaggtactggacggtcgagagctcacggctgtcatccatgcggccggcgtcctggacgatggagtgctggaagcgctggacgcgtcgcggttggacaccgtcttgcaaccaaagatggatgcggcatggaacctgcacgagcttacacggcacctggacttgacagcgtttgtcttgttctccagcgccaccggcgtcctgggcaacgctggccaggcgaactatgcggccgctaacgtattccttgacgcattggcacaaacccgcaggaccgaaaacctccctggtcatagcttggcatggggtctgtgggcagaagcttccgccatgacggccggcctgagcgaaaccgaccgccatagaattgcccgtctgggcgctcagccgctcaacgaaaccgaagcactggcacttttggacagggctttgggtgaagacgcacccgcactgttggtccctgtgcgtctgaaccttgcggcactgcagggtcgctctcaagcggttcctgccgttctgcgcgcgcttgtaccagtccgggcgcggcgccaggccgcggtcggcgcagccgctggttctggtggaggcctcgtagaaaggcttgcggctatgtccgagtcacgacgtgccgcgcatctgcttgatctggtccggaccgaagtcgctggtgtactgggccaccgctccgcggctaccattgaacccgagcgcgccttcaaggacctgggtttcgattcgctcaccgccgtcgagctgcggaaccggctccatgctgccaccggtctgaagccggcggccaccgtggtcttcgaccacccaacctccgccgacctggcgcgccaccttcgtacgcagatcccagatctgccagctgccggaccagaatgtcttctgggcgaactggatcggatagaacagatgctgacagatgttgaccccacagacgaaaagtcgggagacatccagcgccgcctgacggcgctgcttgctcgctttgacgaggccgcggggccagtcgaagcagctcaagtggcagataagatcgatgcagccaccgacgatgaaatttttgctttcattgacaacgagctcggttgatagcataaccccttggggcctctaaacgggtcttgaggggttttttgactacgtaatgagaccttgaggtaaaccaaataagcacgtagtggcgctgctccttcggtcggacgtgcgtctacgggcaccttaccgcagccgtcggctgtgcgacacggacggatcgggcgaactggccgatgctgggagaagcgcgctgctgtacggcgcgcaccgggtgcggagcccctcggcgagcggtgtgaaacttctgtgaatggcctgttcggttgctttttttatacggctgccagataaggcttgcagcatctgggcggctaccgctatgatcggggcgttcctgcaattcttagtgcgagtatctgaaaggggatacgcatgtcgaacgaacaaaagctccgtgattatttgaagcgcgtcaccacagatcttgcagaaacccggcgtcgtctgggtcaagccgaggcggcacggcacgaaccaatagcgattgtcggcatggcctgccgctatccagggggtgtagagtctccagaagacctgtgggaactggttgcggagggccgcgacgccatcgatgtcatgccaggcgaccggggttgggatgtcgacgcgctgtatgatcctgacccgagctcgaccggtaagacgtactctcgcgagggtggattcctgcgaaacgcagcggaattcgatcccgcgtttttcggcatctcacctcgggaagccctggcgatggatccacagcaacgtttgctcttggaaactagctgggaggcgttcgagcgcgccggtatcgaccccgcaaccctgcgcggatcgcggacgggtgtgttcgccggtgtcatgtatcatgattacgggtctcggctgggtaccggaacggtacccgaggacgtcgagggctatgtcggcaacggaagcgccggttcgatcgccacgggtcgtatcgcctacacccttggcctggaaggtccggcggtcaccgtcgataccgcgtgcagctctagtctggtcgccatgcatttggccatccaagcgatacggcaaggagagtgcagcatggcgctggccggaggtgtgaccgtcatggcaaccccggacacctttgtggaattctcgagacagcgcggtctggcccccgacggccgctgtaaggctttcggagcaggagccgatggtaccggctgggcagagggagctggtatgctgctcgtggaacgtctgtcggatgctgaacgtttgggccatcccatccttgctgtcgtacggggtagcgcggtcaaccaggacggagccagtaacggcttgaccgcgccaaacggaccctcgcagcaacgcgtgatacgccaggccctggccacagcaggtttgggtcccaccgatatcgacgcggtcgagggtcacggaaccggcacgtccctgggtgaccccattgaagtgcaagcgctgcaagcgacctacggccaggagcggccggcagagcggccgttgtggttgggtagcctcaagtctaacattgggcacgcccaggcggccgctggtgtgggcggtgtgatcaagatggtcatggcccttcgggaaggcgtgctgccgcggacccttcacgctgacgaaccttcaccgcatatcgattggacagccggtgcggtccgcctcctgaccgaacaatccgcctggccggacaccgatcgtccacggcgtgccgcggtgtcgtccttcggagtctcgggcaccaacgcgcacgttatcattgagcagccatccgaacctgtagaacctgcggacacggacccggagtcacacagcgacagcgaggcagattcggatggaaccccagtggtacaccctgcactgctcccctggcctgtctccgcccggggtgcagatgccgtcagagctcaagctgcccgtttgcatgcgcatctgttggccaggccggatctcacggcggctgatgtagctttcagccttggcaccacacggaccgcgctgcctcatcggtttattgcactgggtaccgaccgcgccgaattgatcaacaccctcgcccggttcgccgaaggctcggaatcagcggctgatggcctcaccggcactgcgaccccaggcgcaaccgcattcctcttcagcggccaaggctcacaatgggcgggcatgggtagagaactccaagctcggttcccccgctttaggcaggccttggatgagacg

SEQ ID NO: 13 - DNA, 3440 bp, Artificial Sequence
  DNA fragment
cgtctcaactggtcttcgaccaccctaccccgctggctatcgccgcatacttgaaggccgagctgtacggacctgatccgggtgacgattccagcgtcctgaccgagctcgatggcctgtcccaacggttggcggcaatcgatcccgacaccaacacccgccttgagatcaccctgcgtctgcgctcgttgctgacgcagtggtccgaaccggacggtggacgcaccactgcagagacagcaacggcaacgagtaccacggcattggaatcggcatccgcggacgaggtcctggctttcattgacaccgagttggggatttgatgacataaccccttggggcctctaaacgggtcttgaggggttttttgccgtgaactagagaccgtcagcgtcgagcacgcggcgctgctccttcggtcggacgtgcgtctacgggcaccttaccgcagccgtcggctgtgcgacacggacggatcgggcgaactggccgatgctgggagaagcgcgctgctgtacggcgcgcaccgggtgcggagcccctcggcgagcggtgtgaaacttctgtgaatggcctgttcggttgctttttttatacggctgccagataaggcttgcagcatctgggcggctaccgctatgatcggggcgttcctgcaattcttagtgcgagtatctgaaaggggatacgcatggcggaccacgacaagctcgttgattatttgaagcgcgtcaccgcagatcttcaacagacccgccagcgtctgcgggagtacgaaacccagagccatgaaccaatagcaatcgttggcatgggctgccgctaccctggatccgtggcatcccctgaagagctgtggcgcctggtccacggtggcgtggacgccgtcggcggtctcccgaccgaccgggggtgggatgtggaagccttgtacgatcctaaggcacagaacccgggcacgacctatgcccgtgaaggtggctacctgaccggagcgacagagttcgacccggaattctttggtatctccccccgtgaggccctggccatggatcctcaacagcgcttggtgctcgaggtcgcttgggaaaccctggagcatgccggcatcgactccgccacactgcgcggcagctcgaccggtgttttcgtgggatgtaactatcaggagtaccgggcaaggctgtcggaggtacaggaaggccttgaaggccatctggtgaccggctccgtaagctccgtggtgtcgggccgtgtttcttacgtcctcggccttgagggccccgctcttacggtcgacaccgcttgttccagtagcttggtcaccctgcacttggcttgcgaagcacttaggcggaacgaatgtaccatggcacttgccggcggagtggctgtcatgtcaacaccgcataccatcacgggtttctcccggcaacggggcgtggcagcggacggccggtgcaaggcatttagcgcaagcgcagacggtatgggtttcggcgaaggtgtaggtcttctgctcgtggaacgtctgtcggatgctcgacgtttgggccatcgcgtgcttgctgtcgtacggggtagcgcggtcaaccaggacggagccagtaacggcttgtccgcgccatcaggacccgctcagcaacgcgtgatacgccaggccctggtcaacgccggtgtgcaggccagccaggtcgacgtggtcgaggctcacggaaccggcacgcgcctgggtgaccccattgaagctcaagcgctgcaagcgacctacggccagggtcggccggcagagcggccgttgtggttgggtagcctcaagtctaacattgggcacgcccaggcggccgctggtgtgggcggtgtgatcaagatggtcatggcccttcgggaaggcgtgctgccgcccacccttcacgctgacgaaccttcaccgcatatcgattggacagccggtaacgtccgcctcctgaccgaatcacgggaatggccggaagcgggtcagccacggcgtgccgcggtgtcgtccttcggaatctcgggcaccaacgcgcacgttatcttggaggcggcagaagcagttgacgcatcgggggaggctgacggcggtgccggcgacgaaggcacgccagtgctttctggaaccgacgtggtagcctggcctgtcagtgcagcctcgccagacgccctgcgggcacaggccgaaagattgagggctcatgtggctgagcgtcctgggttggccagcgcggatgtagctttctcgcttgcaactagcaggtcggcccttgcacggcgcgcgctggttgtgggtggggatcgcgacgagctggtcgcaggcctggagagtctggccgcagaccggcccggcaacggccttgtcaagggtttggctgacctcgcaaccaagccggtgttcgtcttccccggccagggatcccaatgggccggaatggccgtcgaactgctcgatagctccccagtctttgcggatagtatgcaagcttgctcggaagctctgaacgagttcgtagattggaacctcctggaggtcctgcggtccgatgacgaagagttgagcaaccgcgtagatgtggtccagcctgtgctgtgggccgtaatggtgtccctcgcggcactctggcaggcgtgcggcgtccgcccggcagccgtggtaggccattctcagggcgagatagcagctgccgtggtcgctggtgccctgtcactccgtgatggggcccgcgtggtagccttgcggtcggcggtaatagcgcggctgttggccggtaagggtgcgatggcctccgttgcgctcgcatccgataccgtgcgtgaacgcctgaccccctgggagggtcgtctgtccttggcggctgtaaacggcccttcgtcatcggtggtctgcggccacttggacgcgttggatgagttcgtgtctgcattggaacatgacggcgtgagggtgcgcaggatagccgtggactacgcgtcccactctgtcttcgtagaacaagcggaggaagagttgcgcaacgtcctgaccgaagtctcgccgttgccgggcgaggtaccgttctattccaccgttaccggcgcggtgctcgacaccacgacccttgatgctggatattggtaccggaacttgcgccagacggtacgtttcgaagagactgtgcgcgaactgaccaggcgcggtcacgatgcattcattgaagtttctgcccatccggtcctgacggtcggcattcaggacaccttggaggctaccggaacacgccacgccgtctgtgggacactgcgtcgcggcgaaggaggcgcgcaacggctcctgacgtcccttggagaagcatgggtggcgggcatcgcggtcgattggtcgcgattgacgcccaccgctaccgccgtagaactgccaacgtacgcctttcaacattgagacg

SEQ ID NO: 14 - DNA, 900 bp, Artificial Sequence
  promoter
actacgagatttgaggtaaaccaaataagcacgtagtggcacaatgagaccttgaggtaaaccaaaacgccacgcgtagtgagacatacacgttcgttgggttcacgactcaacacgctagggacgtgaagtcgattccttcgatgcattgtaatagccaccaaaagagtgatgatagtcatgggtgtctgtagcacgtgcatcgctcattacaacggttattaagcacgtagtggcgtgcacgcggtcgatcttgacggctggcgagaggtgcggggaggatctgaccgacgcggtccacacgtggcaccgcgatgctgttgtgggcacaatcgtgccggttggtaggatccagcgatggcgggcccaccgcctttccctcgtcggcgtggcccctcaggccgacgtcggtgcggcggacgggctacaccgggtagcgtccgggaccgcaccggcagacgcccagcggctgtccccagccgcgccgtgtgcgcggccgacctttgtgaagagaacgacgatggctccaagaacgtgtcggaacaccgcggatcagcgggtggtagcgttctgtttcctcgtacgggcacagtcctgccatgggtgcttacgggaccgggcgcagcggcggtgcgtgcacgctccgaagcgctgcgcacccacctccgcgcctctacggaatggagccctgcaggcgtaggtcaggcgctgctggcaggaacaggggcgggcgcggacacccaccgtgccgttgttctcgccggtgatcgtgcccaaactctgaatgccctggccgcgctgtctgcaggagcggaccacccagccgtctttaccagcacccgtgccgacgccagcccagctggtccagtgtttgtgtttccaggccaggggtctcaatgg

SEQ ID NO: 15 - DNA, 571 bp, Artificial Sequence
  promoter
actacgagatttgaggtaaaccaaataagcacgtagtggcattccgagaccatgtcgatactgaacgaatcgacgccacgcgtagtgagacatacacgttcgttgggttcacgactcaacacgctagggacgtgaagtcgattccttcgatgcattgtaatagccaccaaaagagtgatgatagtcatgggtgtctgtagcacgtgcatcgctcattacaacggttatacgcacactcccttccttgtgttcacattcgaacggtgtctgctttgacaacatgctgtgcggtgttgtaaagtcgtggccaggagaatacgacagcgtgcaggactgggggagttatgcagtccgcagaaaaggcaaagcctgctgatggcgccgcagcggcattgctggcaaccctcacccataaacggcgtctggacgcggccaccccgaaggaaagcgcactgtggttgctggaccgcctgctccctgaagcgggtgtaaacaatgttccactggccgtccgcgtcgatggtcgtctggacgccgcggctttgcaagcagcggtcgacggtctcgtgcg

SEQ ID NO: 16 - DNA, 829 bp, Artificial Sequence
  promoter
actacgagatttgaggtaaaccaaataagcacgtagtggcgtaatgagaccttgaggtaaaccaacgccacgcgtagtgagacatacacgttcgttgggttcacgactcaacacgctagggacgtgaagtcgattccttcgatgcattgtaatagccaccaaaagagtgatgatagtcatgggtgtctgtagcacgtgcatcgctcattacaacggttataataagcacgtagtggctgttcacattcgaacggtgtctgctttgacaacatgctgtgcggtgttgtaaagtcgtggccaggagaatacgacagcgtgcaggactgggggagttatgtcgaacgaacaaaagctccgtgattatttgaagcgcgtcaccacagatcttgcagaaacccggcgtcgtctgggtcaagccgaggcggcacggcacgaaccaatagcgattgtcggcatggcctgccgctatccagggggtgtagagtctccagaagacctgtgggaactggttgcggagggccgcgacgccatcgatgtcatgccaggcgaccggggttgggatgtcgacgcgctgtatgatcctgacccgagctcgaccggtaagacgtactctcgcgagggtggattcctgcgaaacgcagcggaattcgatcccgcgtttttcggcatctcacctcgggaagccctggcgatggatccacagcaacgtttgctcttggaaactagctgggaggcgttcgagcgcgccggtatcgaccccgcaaccctgcgcggatcgcggacgggtgtgttcgccggtgtcatgtatcatgattacgggtctcggctg

SEQ ID NO: 17 - DNA, 594 bp, Artificial Sequence
  promoter
actacgagatttgaggtaaaccaaataagcacgtagtggcattccgagaccatgtcgatactgaacacgccacgcgtagtgagacatacacgttcgttgggttcacgactcaacacgctagggacgtgaagtcgattccttcgatgcattgtaatagccaccaaaagagtgatgatagtcatgggtgtctgtagcacgtgcatcgctcattacaacggttatgaatcgacgcacactcccttccttggtgcacgcggtcgatcttgacggctggcgagaggtgcggggaggatctgaccgacgcggtccacacgtggcaccgcgatgctgttgtgggcacaatcgtgccggttggtaggatccagcgatgcagtccgcagaaaaggcaaagcctgctgatggcgccgcagcggcattgctggcaaccctcacccataaacggcgtctggacgcggccaccccgaaggaaagcgcactgtggttgctggaccgcctgctccctgaagcgggtgtaaacaatgttccactggccgtccgcgtcgatggtcgtctggacgccgcggctttgcaagcagcggtcgacggtctcgtgcg

SEQ ID NO: 18 - DNA, 540 bp, Artificial Sequence
  promoter
actacgagatttgaggtaaaccaaataagcacgtagtggctagatgagaccgcgcagatgtacgacaatatcgcacgccacgcgtagtgagacatacacgttcgttgggttcacgactcaacacgctagggacgtgaagtcgattccttcgatgcattgtaatagccaccaaaagagtgatgatagtcatgggtgtctgtagcacgtgcatcgctcattacaacggttatttagtcacccttgggccgtgcacgcggtcgatcttgacggctggcgagaggtgcggggaggatctgaccgacgcggtccacacgtggcaccgcgatgctgttgtgggcacaatcgtgccggttggtaggatccagcgatggcgaccccaaacgagaaagttgtggaggctctgcgcgcctccctcaaggaaaccgaactccttcgtcaacagaacaatgcgctccgcgcggccagctcggaaccagtagcaatcgttggcatgggctgccgcttccctggaggtgtggtatcccctgaaggtctctggga

SEQ ID NO: 19 - DNA, 852 bp, Artificial Sequence
  promoter
actacgagatttgaggtaaaccaaataagcacgtagtggcgtaatgagaccttgaggtaaaccaaataagacgccacgcgtagtgagacatacacgttcgttgggttcacgactcaacacgctagggacgtgaagtcgattccttcgatgcattgtaatagccaccaaaagagtgatgatagtcatgggtgtctgtagcacgtgcatcgctcattacaacggttatcacgtagtggcgtgcacgcggtcgatcttgacggctggcgagaggtgcggggaggatctgaccgacgcggtccacacgtggcaccgcgatgctgttgtgggcacaatcgtgccggttggtaggatccagcgatgtcgaacgaacaaaagctccgtgattatttgaagcgcgtcaccacagatcttgcagaaacccggcgtcgtctgggtcaagccgaggcggcacggcacgaaccaatagcgattgtcggcatggcctgccgctatccagggggtgtagagtctccagaagacctgtgggaactggttgcggagggccgcgacgccatcgatgtcatgccaggcgaccggggttgggatgtcgacgcgctgtatgatcctgacccgagctcgaccggtaagacgtactctcgcgagggtggattcctgcgaaacgcagcggaattcgatcccgcgtttttcggcatctcacctcgggaagccctggcgatggatccacagcaacgtttgctcttggaaactagctgggaggcgttcgagcgcgccggtatcgaccccgcaaccctgcgcggatcgcggacgggtgtgttcgccggtgtcatgtatcatgattacgggtctcggctg

SEQ ID NO: 20 - DNA, 559 bp, Artificial Sequence
  promoter
actacgagatttgaggtaaaccaaataagcacgtagtggcaactagagaccgtcagcgtcacgccacgcgtagtgagacatacacgttcgttgggttcacgactcaacacgctagggacgtgaagtcgattccttcgatgcattgtaatagccaccaaaagagtgatgatagtcatgggtgtctgtagcacgtgcatcgctcattacaacggttatgagcacgcggcgtgcacgcggtcgatcttgacggctggcgagaggtgcggggaggatctgaccgacgcggtccacacgtggcaccgcgatgctgttgtgggcacaatcgtgccggttggtaggatccagcgatggcggaccacgacaagctcgttgattatttgaagcgcgtcaccgcagatcttcaacagacccgccagcgtctgcgggagtacgaaacccagagccatgaaccaatagcaatcgttggcatgggctgccgctaccctggatccgtggcatcccctgaagagctgtggcgcctggtccacggtggcgtggacgccgtcggcggtctcccgac

SEQ ID NO: 21 - DNA, 517 bp, Artificial Sequence
  promoter
actacgagatttgaggtaaaccaaataagcacgtagtggctagatgagaccgcgcagatgtacgacaatatcgcttagtcacccacgccacgcgtagtgagacatacacgttcgttgggttcacgactcaacacgctagggacgtgaagtcgattccttcgatgcattgtaatagccaccaaaagagtgatgatagtcatgggtgtctgtagcacgtgcatcgctcattacaacggttatttgggcctgttcacattcgaacggtgtctgctttgacaacatgctgtgcggtgttgtaaagtcgtggccaggagaatacgacagcgtgcaggactgggggagttatggcgaccccaaacgagaaagttgtggaggctctgcgcgcctccctcaaggaaaccgaactccttcgtcaacagaacaatgcgctccgcgcggccagctcggaaccagtagcaatcgttggcatgggctgccgcttccctggaggtgtggtatcccctgaaggtctctggga

SEQ ID NO: 22 - DNA, 536 bp, Artificial Sequence
  promoter
actacgagatttgaggtaaaccaaataagcacgtagtggcaactagagaccgtcagcgtcgacgccacgcgtagtgagacatacacgttcgttgggttcacgactcaacacgctagggacgtgaagtcgattccttcgatgcattgtaatagccaccaaaagagtgatgatagtcatgggtgtctgtagcacgtgcatcgctcattacaacggttatagcacgcggctgttcacattcgaacggtgtctgctttgacaacatgctgtgcggtgttgtaaagtcgtggccaggagaatacgacagcgtgcaggactgggggagttatggcggaccacgacaagctcgttgattatttgaagcgcgtcaccgcagatcttcaacagacccgccagcgtctgcgggagtacgaaacccagagccatgaaccaatagcaatcgttggcatgggctgccgctaccctggatccgtggcatcccctgaagagctgtggcgcctggtccacggtggcgtggacgccgtcggcggtctcccgac

SEQ ID NO: 23 - DNA, 877 bp, Artificial Sequence
  promoter
actacgagatttgaggtaaaccaaataagcacgtagtggcacaatgagaccttgaggtaaaccaaataagacgccacgcgtagtgagacatacacgttcgttgggttcacgactcaacacgctagggacgtgaagtcgattccttcgatgcattgtaatagccaccaaaagagtgatgatagtcatgggtgtctgtagcacgtgcatcgctcattacaacggttatcacgtagtggctgttcacattcgaacggtgtctgctttgacaacatgctgtgcggtgttgtaaagtcgtggccaggagaatacgacagcgtgcaggactgggggagttatggcgggcccaccgcctttccctcgtcggcgtggcccctcaggccgacgtcggtgcggcggacgggctacaccgggtagcgtccgggaccgcaccggcagacgcccagcggctgtccccagccgcgccgtgtgcgcggccgacctttgtgaagagaacgacgatggctccaagaacgtgtcggaacaccgcggatcagcgggtggtagcgttctgtttcctcgtacgggcacagtcctgccatgggtgcttacgggaccgggcgcagcggcggtgcgtgcacgctccgaagcgctgcgcacccacctccgcgcctctacggaatggagccctgcaggcgtaggtcaggcgctgctggcaggaacaggggcgggcgcggacacccaccgtgccgttgttctcgccggtgatcgtgcccaaactctgaatgccctggccgcgctgtctgcaggagcggaccacccagccgtctttaccagcacccgtgccgacgccagcccagctggtccagtgtttgtgtttccaggccaggggtctcaatgg

SEQ ID NO: 24 - DNA, 17749 bp, Artificial Sequence
  OGAB vector1.0
gcggccgcaagcttgaagagctcttctttcagaacgctcggttgccgccgggcgttttttatgagacgtctcggcctgtttggccattaacgtgcaggtggatccagatctaagcttctatagaagcttggtaccgacgtctcggcctgtttggcccgccgcatccataccgccagttgtttaccctcacaacgttccagtaaccgggcatgttcatcatcagtaacccgtatcgtgagcatcctctctcgtttcatcggtatcattacccccatgaacagaaatcccccttacacggaggcatcagtgaccaaacaggaaaaaaccgcccttaacatggcccgctttatcagaagccagacattaacgcttctggagaaactcaacgagctggacgcggatgaacaggcagacatctgtgaatcgcttcacgaccacgctgatgagctttaccgcagctgcctcgcgcgtttcggtgatgacggtgaaaacctctgacacatgcagctcccgaagacggtcacagcttgtctgtaagcggatgccgggagcagacaagcccgtcagggcgcgtcagcgggtgttggcgggtgtcggggcgcagccatgacccagtcacgtagcgatagcggagtgtatactggcttaactatgcggcatcagagcagattgtactgagagtgcaccatatgcggtgtgaaataccgcacagatgcgtaaggagaaaataccgcatcaggcactcttccgcttcctcgctcactgactcgctgcgctcggtcgttcggctgcggcgagcggtatcagctcactcaaaggcggtaatacggttatccacagaatcaggggataacgcaggaaagaacatgtgagcaaaaggccagcaaaaggccaggaaccgtaaaaaggccgcgttgctggcgtttttccataggctccgcccccctgacgagcatcacaaaaatcgacgctcaagtcagaggtggcgaaacccgacaggactataaagataccaggcgtttccccctggaagctccctcgtgcgctctcctgttccgaccctgccgcttaccggatacctgtccgcctttctcccttcgggaagcgtggcgctttctcatagctcacgctgtaggtatctcagttcggtgtaggtcgttcgctccaagctgggctgtgtgcacgaaccccccgttcagcccgaccgctgcgccttatccggtaactatcgtcttgagtccaacccggtaagacacgacttatcgccactggcagcagccactggtaacaggattagcagagcgaggtatgtaggcggtgctacagagttcttgaagtggtggcctaactacggctacactagaaggacagtatttggtatctgcgctctgctgaagccagttaccttcggaaaaagagttggtagctcttgatccggcaaacaaaccaccgctggtagcggtggtttttttgtttgcaagcagcagattacgcgcagaaaaaaaggatctcaagaagatcctttgatcttttctacggggtctgacgctcagtggaacgaaaactcacgttaagggattttggtcatgagattatcaaaaaggatcttcacctagatccttttaaattaaaaatgaagttttaaatcaatctaaagtatatatgagtaaacttggtctgacagttaccaatgcttaatcagtgaggcacctatctcagcgatctgtctatttcgttcatccatagttgcctgactccccgtcgtgtagataactacgatacgggagggcttaccatctggccccagtgctgcaatgataccgcgagacccacgctcaccggctccagatttatcagcaataaaccagccagccggaagggccgagcgcagaagtggtcctgcaactttatccgcctccatccagtctattaattgttgccgggaagctagagtaagtagttcgccagttaatagtttgcgcaacgttgttgccattgctgcaggcatcgtggtgtcacgctcgtcgtttggtatggcttcattcagctccggttcccaacgatcaaggcgagttacatgatcccccatgttgtgcaaaaaagcggttagctccttcggtcctccgatcgttgtcagaagtaagttggccgcagtgttatcactcatggttatggcagcactgcataattctcttactgtcatgccatccgtaagatgcttttctgtgactggtgagtactcaaccaagtcattctgagaatagtgtatgcggcgaccgagttgctcttgcccggcgtcaacacgggataataccgcgccacatagcagaactttaaaagtgctcatcattggaaaacgttcttcggggcgaaaactctcaaggatcttaccgctgttgagatccagttcgatgtaacccactcgtgcacccaactgatcttcagcatcttttactttcaccagcgtttctgggtgagcaaaaacaggaaggcaaaatgccgcaaaaaagggaataagggcgacacggaaatgttgaatactcatactcttcctttttcaatattattgaagcatttatcagggttattgtctcatgagcggatacatatttgaatgtatttagaaaaataaacaaataggggttccgcgcacatttccccgaaaagtgccacctggatccacctgcacgtaaaaggccttcttggccaccccgggccgtcgaccaattctcatgtttgacagcttatcatcgaatttctgccattcatccgcttattatcacttattcaggcgtagcaaccaggcgtttaagggcaccaataactgccttaaaaaaattacgccccgccctgccactcatcgcagtactgttgtaattcattaagcattctgccgacatggaagccatcacaaacggcatgatgaacctgaatcgccagcggcatcagcaccttgtcgccttgcgtataatatttgcccatggtgaaaacgggggcgaagaagttgtccatattggccacgtttaaatcaaaactggtgaaactcacccagggattggctgagacgaaaaacatattctcaataaaccctttagggaaataggccaggttttcaccgtaacacgccacatcttgcgaatatatgtgtagaaactgccggaaatcgtcgtggtattcactccagagcgatgaaaacgtttcagtttgctcatggaaaacggtgtaacaagggtgaacactatcccatatcaccagctcaccgtctttcattgccatacggaattccggatgagcattcatcaggcgggcaagaatgtgaataaaggccggataaaacttgtgcttatttttctttacggtctttaaaaaggccgtaatatccagctgaacggtctggttataggtacattgagcaactgactgaaatgcctcaaaatgttctttacgatgccattgggatatatcaacggtggtatatccagtgatttttttctccattttagcttccttagctcctgaaaatctcgataactcaaaaaatacgcccggtagtgatcttatttcattatggtgaaagttggaacctcttacgtgccgatcaacgtctcattttcgccaaaagttggcccagggcttcccggtatcaacagggacaccaggatttatttattctgcgaagtgatcttccgtcacaggtatttattcgcgataagctcatggagcggcgtaaccgtcgcacaggaaggacagagaaagcgcggatctgggaagtgacggacagaacggtcaggacctggattggggaggcggttgccgccgctgctgctgacggtgtgacgttctctgttccggtcacaccacatacgttccgccattcctatgcgatgcacatgctgtatgccggtataccgctgaaagttctgcaaagcctgatgggacataagtccatcagttcaacggaagtctacacgaaggtttttgcgctggatgtggctgcccggcaccgggtgcagtttgcgatgccggagtctgatgcggttgcgatgctgaaacaattatcctgagaataaatgccttggcctttatatggaaatgtggaactgagtggatatgctgtttttgtctgttaaacagagaagctggctgttatccactgagaagcgaacgaaacagtcgggaaaatctcccattatcgtagagatccgcattattaatctcaggagcctgtgtagcgtttataggaagtagtgttctgtcatgatgcctgcaagcggtaacgaaaacgatttgaatatgccttcaggaacaatagaaatcttcgtgcggtgttacgttgaagtggagcggattatgtcagcaatggacagaacaacctaatgaacacagaaccatgatgtggtctgtccttttacagccagtagtgctcgccgcagtcgagcgacagggcgaagccctcgagtgagcgaggaagcaccagggaacagcacttatatattctgcttacacacgatgcctgaaaaaacttcccttggggttatccacttatccacggggatatttttataattattttttttatagtttttagatcttcttttttagagcgccttgtaggcctttatccatgctggttctagagaaggtgttgtgacaaattgccctttcagtgtgacaaatcaccctcaaatgacagtcctgtctgtgacaaattgcccttaaccctgtgacaaattgccctcagaagaagctgttttttcacaaagttatccctgcttattgactcttttttatttagtgtgacaatctaaaaacttgtcacacttcacatggatctgtcatggcggaaacagcggttatcaatcacaagaaacgtaaaaatagcccgcgaatcgtccagtcaaacgacctcactgaggcggcatatagtctctcccgggatcaaaaacgtatgctgtatctgttcgttgaccagatcagaaaatctgatggcaccctacaggaacatgacggtatctgcgagatccatgttgctaaatatgctgaaatattcggattgacctctgcggaagccagtaaggatatacggcaggcattgaagagtttcgcggggaaggaagtggttttttatcgccctgaagaggatgccggcgatgaaaaaggctatgaatcttttccttggtttatcaaacgtgcgcacagtccatccagagggctttacagtgtacatatcaacccatatctcattcccttctttatcgggttacagaaccggtttacgcagtttcggcttagtgaaacaaaagaaatcaccaatccgtatgccatgcgtttatacgaatccctgtgtcagtatcgtaagccggatggctcaggcatcgtctctctgaaaatcgactggatcatagagcgttaccagctgcctcaaagttaccagcgtatgcctgacttccgccgccgcttcctgcaggtctgtgttaatgagatcaacagcagaactccaatgcgcctctcatacattgagaaaaagaaaggccgccagacgactcatatcgtattttccttccgcgatatcacttccatgacgacaggatagtctgagggttatctgtcacagatttgagggtggttcgtcacatttgttctgacctactgagggtaatttgtcacagttttgctgtttccttcagcctgcatggattttctcatactttttgaactgtaatttttaaggaagccaaatttgagggcagtttgtcacagttgatttccttctctttcccttcgtcatgtgacctgatacgcgtgctaccttaagagagtcaattcgcccttcccggtcgatatgaacagcttatttacataattcacgttattggtagttataaatgaaattcctaatatcggttatgaagtgaaattgaatttctacttgatctttctctctatttttgtaaaataaaattaagaatatttaaatattcaatgattcatttttgcagaaatcggaggaagaagaatatatgaaaacatttaacatttctcaacaagatccccccatattgttgtataagtgatgaaatactgaatttaaaacttagtttatatgtggtaaaatgttttaatcaagtttaggaggaattaattatgaagtgtaatgaataatgaatgtaacagggttcaattaaaagagggaagcgtatcattaaccctataaactacgtctgccctcattattggagggtgaaatgtgaatacatcctattcacaatcgaatttacgacacaaccaaattttaatttggctttgcattttatctttttttagcgtattaaatgaaatggttttgaacgtctcattacctgatattgcaaatgattttaataaaccaccagcgagtacaaactgggtgaacacagcctttatgttaaccttttccattggaacagctgtatatggaaagctatctgatcaattaggcatcaaaaggttactcctatttggaattataataaattgtttcgggtcggtaattgggtttgttggccattctttcttttccttacttattatggctcgttttattcaaggggctggtgcagctgcatttccagcactcgtaatggttgtagttgcgcgctatattccaaaggaaaataggggtaaagcatttggtcttattggatcgatagtagccatgggagaaggagtcggtccagcgattggtggaatgatagcccattatattcattggtcctatcttctactcattcctatgataacaattatcactgttccgtttcttatgaaattattaaagaaagaagtaaggataaaaggtcattttgatatcaaaggaattatactaatgtctgtaggcattgtattttttatgttgtttacaacatcatatagcatttcttttcttatcgttagcgtgctgtcattcctgatatttgtaaaacatatcaggaaagtaacagatccttttgttgatcccggattagggaaaaatataccttttatgattggagttctttgtgggggaattatatttggaacagtagcagggtttgtctctatggttccttatatgatgaaagatgttcaccagctaagtactgccgaaatcggaagtgtaattattttccctggaacaatgagtgtcattattttcggctacattggtgggatacttgttgatagaagaggtcctttatacgtgttaaacatcggagttacatttctttctgttagctttttaactgcttcctttcttttagaaacaacatcatggttcatgacaattataatcgtatttgttttaggtgggctttcgttcaccaaaacagttatatcaacaattgtttcaagtagcttgaaacagcaggaagctggtgctggaatgagtttgcttaactttaccagctttttatcagagggaacaggtattgcaattgtaggtggtttattatccatacccttacttgatcaaaggttgttacctatggaagttgatcagtcaacttatctgtatagtaatttgttattacttttttcaggaatcattgtcattagttggctggttaccttgaatgtatataaacattctcaaagggatttctaaatcgttaagggatcaactttgggagagagttcaaaattgatcctttttttataacaggaattgggcatcaaataaaacgaaaggctcagtcgaaagactgggcctttcgttttatctgttgtttgtcggtgaacgctctcctgagtaggacaaatccgccgggagcggatttgaacgttgcgaagcaacggcccggagggtggcgggcaggacgcccgccataaactgccaggcatcaaattaagcagaaggccatcctgacggatggcctttttgcgtttctacaaactcttcctgtcgtcatatctacaattctacacagcccagtccagactattcggcactgaaattatgggtgaagtggtcaagacctcactaggcaccttaaaaatagcgcaccctgaagaagatttatttgaggtagcccttgcctacctagcttccaagaaagatatcctaacagcacaagagcggaaagatgttttgttctacatccagaacaacctctgctaaaattcctgaaaaattttgcaaaaagttgttgactttatctacaaggtgtggcataatgtgtggaattgtgagcggataacaattaagctaattctatggtaaaagcattcctgaacccaatatccttatttttagtggacaaggccttgttctcatatggttgcttgagccagtgccttacaaggctcttccgctttggcaggctgttcaaaattatttattagagcaactcaaggaactaggcggagatccaaaagcaaccgatgcagcacgtgtttttcggattgctgggagcgtcaatagtaagaatggagcggaagtaagagcggaatatcggcacgattacagatatgagttaaggcagattcaatttgattaccttccagaactcaatgaggttattaatcccgctccacaaaagaaaaaacgggggcgtaaaaagaaagtagttcagttattcaatacctacaaactccattacgctcgcctattggatatagtgaaattggtggaactacgaaattatgaggtaactggatacagggaaatcatttgctttttataccgttattggttgtgctgttacacgaacgaccctgtagaggctttaaatcaaacacagacacttaatttacagttcactgagcctttacccttaaaagaggttgaaagggctacacggagcgcagaaaaggcgtgggaagcacgaaataacgaagaggctaaccggattgcaatcgaaaaaggatatcccagtgctggatacaatattagcaataaaaagttgattgaatggctagatatcacaccagaagaacagaagcatttacagacgattatagacgctaatgagaaacggagaagaaagcgggaaagggataggatttatcaagaacaaaaacgtcgtgagcggggagatatgacccgacaggagtatattaagcaacaacaggataaaacagatgataaattatttaaattgcaggagttattagaacagaatcccaaaatctcaaaaattaaattagcaaaaatacttggtgtagataaatcgcacttatacagactgctgaaacaactataactggaaaaaattagtgtctcatggttcgtcgcccttatattatgggcgttagcctgcttgctaattggataggtgttattgtcatttcaacgtcggacgttttggtagatgaacgtcggacgttatttgcttcaatagattgttgatgtattaagggttgcagtgaatcgacaagcaaaaagttatgacgttgtgaaaaaattgaatagaaaattggaaattacgtcggacgttctaacttaaaaaccctgttatatcaatgatttaaaaggaaattaacgtcataaaagacctttctgcaacaaaagtttttctggaagagttgaggttattttataggtattatggacttttgtagactttttgtgtactttttgtggactccacactcgctggtatcgtgttattttttaattgagatatgaatatggaaattaaacgttttaggcgttggtttggtgatgacaaaaaaataagagtacccgctcacaacggatactctttcgagaaatgtacgaaacgctataaataaaaaataactagatacatttacattgtatcacgtttcgtacatttctccaataacaaattgattggaggaatgcaaagtgaataatgaaccagtaaaacgtggtaagaagaacagatgggaattaaacctacctataatgacttatgtagtagctgatgattggattgataaactaggacacgaaacgtttactttatggttgaggttccatacttgggtagatagagaagatgaactccgagattatgatcgcatacctagaagttttgagaacatatataaaaagacactaggaatctcaaaaagtaagttttatagattgataaaacctttatgggaatatggattaatagacatcatagaatacgaagaatctaaccgtaattctactaaacctaaaaatataattgtttatgagtatcctttacacgaaatagaaagaaagtataaaccactagaaaaattaagagattgggataaagactataattccgtttctaaagaattaggtaaaacaggtggtagaccaaggaaaaaagatagtgaagaagaacccgaaaagaaacccgaagaagtaactaaaaagaaacgtaaatataagttaaaaagagttatccacaacggtttcaaaaatgaaacggtggagggtttcaaaaatgaaacggtggagggtttcaaaaatgaaacggtgaccgtttcaaaaataaaacccaataattattcaaatatctttaataacttatcaaatatttctactaatgtttcaaataatttattaattgatgatgatgaggaaatcgaaaatgaaccaactggtcgtacaataaataggtcattacttttttcacaagaagatattaaacaggcctatcaatttattaatagattttcagttatacagttacgtgaaaactttagctttgataaacactttgaagaacggttggtatgttatttatggaaagcagggatttctactttttacacgcacgaaatcagtaaaatgataaaaaaaatagcagactatgaaaaatctaaaaaaggtagattaaacccaatacgtgaccgagccttatatatggtaaatggtcttgtaatgaatagagcttcttcccaaagtgaacatgctacttataaactaaaccaatataaaaaacagaaggaacaggaaaaacaacaacaggagcaacaaagatcaagagtaccgttctataattggttggaggaaagagaagaacaaaccgaaggtcaactacccaccacttaaagcctaacggcttttgaagtggggcttgtaaaaagccctagttgactaccccaagtctttcgaggactacgttggaaaggtcatgacacctacaaatgctcctctagttcgtagccactgtcgttgatggttaaaagtcctgatgggtagggacggtgctgtcaacatcacaagcccttccaacatgggggaagaggaagaacactccgagaaaggagggggctgtcgtacacgccttgttcgtgtacgtgatttttaacacttttatctctaatataatctctccttgagttagcagagactaagaataaaacacattaggattttttatctacataaggaggttcaatacatgcctactatttcgtttaagggaaagtcttttgtacaaaatcatcacttgactgtaaaatatcatgaattgatcccagaaccagaaaaaagtctgaccgataaagttagtcttcatgacaatcttatcattcatggggacaatttaaaggcgttgaaagctctactacctacatatgctggtaagatagattgcatctatattgacccaccatacaatactggaactgaaaaatggatttataatgataatgtcaactccccaatgattagggaatggcttggaaaagtggtagacaaagaagacttatcccgacatgataagtggctttgtatgatgatgccgaggttaaaactgttgaaagagttgttgtcagaagacggagtgatatttgtaagcattgactacaatgaaatacaccatcttacgtgccttatgaacgaaatattcggtgaggagaattttcgtgacgctattatcattcgtagaggagtaaaaaatgttcaagcgcaatttgacacaattgattctctttcaaatggttatgagtctattttggtttacactaaacagccatctcgacgatttaataaggtttatgaagatgtagaagaaaagcctggtagttggaataatcattggagaggtacagaccgtaaaactatgagatatgaattatttggggttactccgacagaaggtcaatggagatgggggaaagaacgtagtctccaggctattgaaaactatcaaatgatgttagatgaacttagacaaaaaggcattactaatccaactcaagaggatattgataaatggtatcttgaatatgtagaaaataatggggaagatattgacttgttacgacaaaatgataatggcacgattgagcactttgttccaccgactagcaaaaagttgttaagtaatgcctggtttgacttaaaacccaacggttctagtcaattaaagaagatatttggaaggaaggttttcgataaccctaaatcaattgatttggtaaaaagactaatacaatttgcgactgaaaacaaagaagcgattgtacttgactcatttgcagggagtggcactactgctcatgcagtattatcgcttaacaaacaagatggagggaatcgtcgtttcatccttattgagatggaagaatatgcacatgagattaccgcagaacgcggatctttatcgatttgcatgcaagctaattcggtggaaacgaggtcatcatttccttccgaaaaaacggttgcatttaaatcttacatatgtaatactttcaaagactacatttgtaagatttgatgtttgagtcggctgaaagatcgtacgtaccaattattgtttcgtgattgttcaagccataacactgtagggatagtggaaagagtgcttcatctggttacgatcaatcaaatattcaaacggagggagacgattttgatgaaaccagtaacgttatacgatgtcgcagagtatgccggtgtctcttatcagaccgtttcccgcgtggtgaaccaggccagccacgtttctgcgaaaacgcgggaaaaagtggaagcggcgatggcggagctgaattacattcccaaccgcgtggcacaacaactggcgggcaaacagtcgttgctgattggcgttgccacctccagtctggccctgcacgcgccgtcgcaaattgtcgcggcgattaaatctcgcgccgatcaactgggtgccagcgtggtggtgtcgatggtagaacgaagcggcgtcgaagcctgtaaaacggcggtgcacaatcttctcgcgcaacgcgtcagtgggctgatcattaactatccgctggatgaccaggatgccattgctgtggaagctgcctgcactaatgttccggcgttatttcttgatgtctctgaccagacacccatcaacagtattattttctcccatgaagacggtacgcgactgggcgtggagcatctggtcgcattgggtcaccagcaaatcgcgctgttagcgggcccattaagttctgtctcggcgcgtctgcgtctggctggctggcataaatatctcactcgcaatcaaattcagccgatagcggaacgggaaggcgactggagtgccatgtccggttttcaacaaaccatgcaaatgctgaatgagggcatcgttcccactgcgatgctggttgccaacgatcagatggcgctgggcgcaatgcgcgccattaccgagtccgggctgcgcgttggtgcggatatctcggtagtgggatacgacgataccgaagacagctcatgttatatcccgccgttaaccaccatcaaacaggattttcgcctgctggggcaaaccagcgtggaccgcttgctgcaactctctcagggccaggcggtgaagggcaatcagctgttgcccgtctcactggtgaaaagaaaaaccaccctggcgcccaatacgcaaaccgcctctccccgcgcgttggccgattcattaatgcagctggcacgacaggtttcccgactggaaagcgggcagtgagcgcaacgcaattaatgtgagttaggatcgctaccttaagagagacgcgttatcgggggttagttcgtcatcattgatgagggttgattatcacagtttattactctgaattggctatccgcgtgtgtacctctacctggagtttttcccacggtggatatttcttcttgcgctgagcgtaagagctatctgacagaacagttcttctttgcttcctcgccagttcgctcgctatgctcggttacacggctgcggcgagcgctagtgataataagtgactgaggtatgtgctcttcttatctccttttgtagtgttgctcttattttaaacaactttgcggttttttgatgactttgcgattttgttgttgctttgcagtaaattgcaagatttaataaaaaaacgcaaagcaatgattaaaggatgttcagaatgaaactcatggaaacacttaaccagtgcataaacgctggtcatgaaatgacgaaggctatcgccattgcacagtttaatgatgacagcccggaagcgaggaaaataacccggcgctggagaataggtgaagcagcggatttagttggggtttcttctcaggctatcagagatgccgagaaagcagggcgactaccgcacccggatatggaaattcgaggacgggttgagcaacgtgttggttatacaattgaacaaattaatcatatgcgtgatgtgtttggtacgcgattgcgacgtgctgaagacgtatttccaccggtgatcggggttgctgcccataaaggtggcgtttacaaaacctcagtttctgttcatcttgctcaggatctggctctgaaggggctacgtgttttgctcgtggaaggtaacgacccccagggaacagcctcaatgtatcacggatgggtaccagatcttcatattcatgcagaagacactctcctgcctttctatcttggggaaaaggacgatgtcacttatgcaataaagcccacttgctggccggggcttgacattattccttcctgtctggctctgcaccgtattgaaactgagttaatgggcaaatttgatgaaggtaaactgcccaccgatccacacctgatgctccgactggccattgaaactgttgctcatgactatgatgtcatagttattgacagcgcgcctaacctgggtatcggcacgattaatgtcgtatgtgctgctgatgtgctgattgttcccacgcctgctgagttgtttgactacacctccgcactgcagtttttcgatatgcttcgtgatctgctcaagaacgttgatcttaaagggttcgagcctgatgtacgtattttgcttaccaaatacagcaatagtaatggctctcagtccccgtggatggaggagcaaattcgggatgcctggggaagcatggttctaaaaaatgttgtacgtgaaacggatgaagttggtaaaggtcagatccggatgagaactgtttttgaacaggccattgatcaacgctcttcaactggtgcctggagaaatgctctttctatttgggaacctgtctgcaatgaaattttcgatcgtctgattaaaccacgctgggagattagataatgaagcgtgcgcctgttattccaaaacatacgctcaatactcaaccggttgaagatacttcgttatcgacaccagctgccccgatggtggattcgttaattgcgcgcgtaggagtaatggctcgcggtaatgccattactttgcctgtatgtggtcgggatgtgaagtttactcttgaagtgctccggggtgatagtgttgagaagacctctcgggtatggtcaggtaatgaacgtgaccaggagctgcttactgaggacgcactggatgatctcatcccttcttttctactgactggtcaacagacaccggcgttcggtcgaagagtatctggtgtcatagaaattgccgatgggagtcgccgtcgtaaagctgctgcacttaccgaaagtgattatcgtgttctggttggcgagctggatgatgagcagatggctgcattatccagattgggtaacgattatcgcccaacaagtgcttatgaacgtggtcagcgttatgcaagccgattgcagaatgaatttgctggaaatatttctgcgctggctgatgcggaaaatatttcacgtaagattattacccgctgtatcaacaccgccaaattgcctaaatcagttgttgctcttttttctcaccccggtgaactatctgcccggtcaggtgatgcacttcaaaaagcctttacagataaagaggaattacttaagcagcaggcatctaaccttcatgagcagaaaaaagctggggtgatatttgaagctgaagaagttatcactcttttaacttctgtgcttaaaacgtcatctgcatcaagaactagtttaagctcacgacatcagtttgctcctggagcgacagtattgtataagggcgataaaatggtgcttaacctggacaggtctcgtgttccaactgagtgtatagagaaaattgaggccattcttaaggaacttgaaaagccagcaccctgatgcgaccacgttttagtctacgtttatctgtctttacttaatgtcctttgttacaggccagaaagcataactggcctgaatattctctctgggcccactgttccacttgtatcgtcggtctgataatcagactgggaccacggtcccactcgtatcgtcggtctgattattagtctgggaccacggtcccactcgtatcgtcggtctgattattagtctgggaccacggtcccactcgtatcgtcggtctgataatcagactgggaccacggtcccactcgtatcgtcggtctgattattagtctgggaccatggtcccactcgtatcgtcggtctgattattagtctgggaccacggtcccactcgtatcgtcggtctgattattagtctggaaccacggtcccactcgtatcgtcggtctgattattagtctgggaccacggtcccactcgtatcgtcggtctgattattagtctgggaccacgatcccactcgtgttgtcggtctgattatcggtctgggaccacggtcccacttgtattgtcgatcagactatcagcgtgagactacgattccatcaatgcctgtcaagggcaagtattgacatgtcgtcgtaacctgtagaacggagtaacctcggtgtgcggttgtatgcctgctgtggattgctgctgtgtcctgcttatccacaacattttgcgcacggttatgtggacaaaatacctggttacccaggccgtgccggcacgttaaccgggctgcatccgatgcaagtgtgtcgctgtcgacgagctcgcgagctcggacatgaggttgccccgtattcagtgtcgctgatttgtattgtctgaagttgtttttacgttaagttgatgcagatcaattaatacgatacctgcgtcataattgattatttgacgtggtttgatggcctccacgcacgttgtgatatgtagatgataatcattatcactttacgggtcctttccggtgatccgacaggttacggggcggcgacctcgcgggttttcgctatttatgaaaattttccggtttaaggcgtttccgttcttcttcgtcataacttaatgtttttatttaaaataccctctgaaaagaaaggaaacgacaggtgctgaaagcgagctttttggcctctgtcgtttcctttctctgtttttgtccgtggaatgaacaatggaagtccgagctcatcgctaataacttcgtatagcatacattatacgaagttatattcgat

SEQ ID NO: 25 - DNA, 16509 bp, Artificial Sequence
  OGAB vector2.0
gcgaccgcaagcttgaagagctcttctttcagaacgctcggttgccgccgggcgttttttatgacggtcattacaacggttatacgacgccacgcgtagtgagacatacacgttcgttggatccgggttcactttggttcatgtgcagctccatcagcaaaaggggatgataagtttatcaccaccgactatttgcaacagtgccgttgatcgtgctatgatcgactgatgtcatcagcggtggagtgcaatgtcgtgcaatacgaatggcgaaaagccgagctcatcggtcagcttctcaaccttggggttacccccggcggtgtgctgctggtccacagctccttccgtagcgtccggcccctcgaagatgggccacttggactgatcgaggccctgcgtgctgcgctgggtccgggagggacgctcgtcatgccctcgtggtcaggtctggacgacgagccgttcgatcctgccacgtcgcccgttacaccggaccttggagttgtctctgacacattctggcgcctgccaaatgtaaagcgcagcgcccatccatttgcctttgcggcagcggggccacaggcagagcagatcatctctgatccattgcccctgccacctcactcgcctgcaagcccggtcgcccgtgtccatgaactcgatgggcaggtacttctcctcggcgtgggacacgatgccaacacgacgctgcatcttgccgagttgatggcaaaggttccctatggggtgccgagacactgcaccattcttcaggatggcaagttggtacgcgtcgattatctggagaatgaccactgctgtgagcgctttgccttggcggacaggtggctcaaggagaagagccttcagaaggaaggtccagtcggtcatgcctttgctcggttgatccgctcccgcgacattgtggcgacagccctgggtcaactgggccgagatccgttgatcttcctgcatccgccagaggcgggatgcgaagaatgcgatgccgctcgccagtcgattggctgagctcatgagcggagaacgagatgacgttggaggggcaaggtcgcgctgattgctggggcaacacgtggagcggatcggggattgtctttcttcagctcgctgatgatatgccttcctggttggcttggtttcatcagccatccgcttgccctcatctgttacgccggcggtagccggccagcctcgcagagcaggattcccgttgagcaccgccaggtgcgaataagggacagtgaagaaggaacacccgctcgcgggtgggcctacttcacctatcctgcccggctgacgccgttggatacaccaaggaaagtctacacgaaccctttggcaaaatcctgtatatcgtgcgaaaaaggatggatataccgaaaaaatcgctataatgaccccgaagcagggttatgcagcggaaaagatccgtcgacctgcaggcatgcaagctctagcgattccagacgtcccgaaggcgtggcgcggcttccccgtgccggagcaatcgccctgggtgggttacacgacgcccctctatggcccgtactgacggacacaccgaagccccggcggcaaccctcagcggatgccccggggcttcacgttttcccaggtcagaagcggttttcgggagtagtgccccaactggggtaacctttgagttctctcagttgggggcgtagggtcgccgacatgacacaaggggttgtgaccggggtggacacgtacgcgggtgcttacgaccgtcagtcgcgcgagcgcgaaaattcgagcgcagcaagcccagcgacacagcgtagcgccaacgaggacaaggcggccgaccttcagcgcgaagtcgagcgcgacgggggccggttcaggttcgtcgggcatttcagcgaagcgccgggcacgtcggcgttcgggacggcggagcgcccggagttcgaacgcatcctgaacgaatgccgcgccgggcggctcaacatgatcattgtctatgacgtgtcgcgcttctcgcgcctgaaggtcatggacgcgattccgattgtctcggaattgctcgccctgggcgtgacgattgtttccactcaggaaggcgtgttccggcagggaaacgtcatggacctgattcacctgattatgcggctcgacgcgtcgcacaaagaatcttcgctgaagtcggcgaagattctcgacacgaagaaccttcagcgcgaattgggcgggtacgtcggcgggaaggcgccttacggcttcgagcttgtttcggaaacgaaggagatcacgcgcaacggccgaatggtcaatgtcgtcatcaacaagcttgcgcactcgaccactccccttaccggacccttcgagttcgagcccgacgtaatccggtggtggtggcgtgagatcaagacgcacaagcaccttcccttcaagccgggcagtcaagccgccattcacccgggcagcatcacggggctttgtaagcgcatggacgctgacgccgtgccgacccggggcgaaacgattgggaagaaaaccgcttcaagcgcctgggacccggcaaccgttatgcgaatccttcgggacccgcgtattgcgggcttcgccgctgaggtgatctacaagaagaagccggacggcacgccgaccacgaagattgagggttaccgcattcagcgcgacccgatcacgctccggccggtcgagcttgattgcggaccgatcatcgagcccgctgagtggtatgagcttcaggcgtggttggacggcagggggcgcggcaaggggctttcccgggggcaagccattctgtccgccatggacaagctgtactgcgagtgtggcgccgtcatgacttcgaagcgcggggaagaatcgatcaaggactcttaccgctgccgtcgccggaaggtggtcgacccgtccgcacctgggcagcacgaaggcacgtgcaacgtcagcatggcggcactcgacaagttcgttgcggaacgcatcttcaacaagatcaggcacgccgaaggcgacgaagaaacgttggcgcttctgtgggaagccgcccgacgcttcggcaagctcactgaggcgcctgagaagagcggcgaacgggcgaaccttgttgcggagcgcgccgacgccctgaacgcccttgaagagctgtacgaggaccgcgcggcaggcgcgtacgacggacccgttggcaggaagcacttccggaagcaacaggcagcgctgacgctccggcagcaaggggcggaagagcggcttgccgaacttgaagccgccgaagccccgaagcttccccttgaccaatggttccccgaggacgccgacgctgacccgaccggccctaagtcgtggtgggggcgcgcgtcagtagacgacaagcgcgtgttcgtcgggctcttcgtagacaagatcgttgtcacgaagtcgactacgggcagggggcagggaacgcccatcgagaagcgcgcttcgatcacgtgggcgaagccgccgaccgacgacgacgaggacgacgcccaggacggcacggaggacgtagcggcgtagcgagacacccgggaagcctgatctacgtctgtcgagaagtttcgatgacactcgttcgttcacacgttgcagcatggatccctcgaggagttactggccctgatttctccgcttctaataccgcacatgcggccgcaagctgtctcgacggcgcgcctagaaacaaggcagttccgggctgaaagtagcgccgggactagtcttaattaacggcctgtttggccattatgagacgccctgatgacttgacgctcgagaaggttcacgattagcatgccggttacggacctttgaggagggctcaatgctttccaagggcgaggaggacaacatggccatcatcaaggagttcatgcgcttcaaggtccacatggagggctccgtcaacgggcacgagttcgagatcgagggcgagggggagggccggccgtacgagggcacccagaccgccaagctgaaggtgaccaagggcggccccctcccgttcgcctgggacatcctctccccccagttcatgtacggctcgaaggcctacgtcaagcacccggccgacatcccggactacctgaagctctcgttcccggaggggttcaagtgggagcgggtcatgaacttcgaggacggcggcgtcgtcaccgtcacccaggacagctccctgcaggacggcgagttcatctacaaggtcaagctgcggggcacgaacttcccgagcgacggccccgtgatgcagaagaaaacgatgggctgggaagcgtcctcggagcgcatgtacccggaggacggcgccctcaagggcgagatcaagcagcgcctgaagctgaaggacggcggccactacgacgccgaagtcaagacgacgtacaaggccaagaagccggtgcagctcccggacgcctacaacgtgaacatcaagctcgacatcacctcgcacaacgaggactacacgatcgtggagcagtacgagcgcgccgagggccggcactcgaccggcggcatggacgagctgtacaagtgatgacgtctctaaaatccccggataactgccttaaaaaaagaataaatgccttggcctttatatggaaatgtggaactgagtggatatgctgtttttgtctgttaaacagagaagctggctgttatccactgagaagcgaacgaaacagtcgggaaaatctcccattatcgtagagatccgcattattaatctcaggagcctgtgtagcgtttataggaagtagtgttctgtcatgatgcctgcaagcggtaacacgatttgaatatgccttcaggaacaatagaaatcttcgtgcggtgttacgttgaagtggagcggattatgtcagcaatggacagaacaacctaatgaacacagaaccatgatgtggtctgtccttttacagccagtagtgctcgccgcagtcgagcgacagttcgaagccatcgagtgagcgaggaagcaccagggaacagcacttatatattctgcttacacacgatgcctgaaaaaacttcccttggggttatccacttatccacggggatatttttataattattttttttatagtttttagatcttcttttttagagcgccttgtaggcctttatccatgctggttctagagaaggtgttgtgacaaattgccctttcagtgtgacaaatcaccctcaaatgacagtcctgtctgtgacaaattgcccttaaccctgtgacaaattgccctcagaagaagctgttttttcacaaagttatccctgcttattgactcttttttatttagtgtgacaatctaaaaacttgtcacacttcacatggatctgtcatggcggaaacagcggttatcaatcacaagaaacgtaaaaatagcccgcgaatcgtccagtcaaacgacctcactgaggcggcatatagtctctcccgggatcaaaaacgtatgctgtatctgttcgttgaccagatcagaaaatctgatggcaccctacaggaacatgacggtatctgcgagatccatgttgctaaatatgctgaaatattcggattgacctctgcggaagccagtaaggatatacggcaggcattgaagagtttcgcggggaaggaagtggttttttatcgccctgaagaggatgccggcgatgaaaaaggctatgaatcttttccttggtttatcaaacgtgcgcacagtccatccagagggctttacagtgtacatatcaacccatatctcattcccttctttatcgggttacagaaccggtttacgcagtttcggcttagtgaaacaaaagaaatcaccaatccgtatgccatgcgtttatacgaatccctgtgtcagtatcgtaagccggatggctcaggcatcgtgtctctgaaaatcgactggatcatagagcgttaccagctgcctcaaagttaccagcgtatgcctgacttccgccgccgcttcctgcaggtctgtgttaatgagatcaacagcagaactccaatgcgcctctcatacattgagaaaaagaaaggccgccagacgactcatatcgtattttccttccgcgatatcacttccatgacgacaggatagtctgagggttatctgtcacagatttgagggtggttcgtcacatttgttctgacctactgagggtaatttgtcacagttttgctgtttccttcagcctgcatggattttctcatactttttgaactgtaatttttaaggaagccaaatttgagggcagtttgtcacagttgatttccttctctttcccttcgtcatgtgacctgatacgcgtgctaccttaagagagtcaattcgcccttcccggtcgatatgaacagcttatttacataattcacgttattggtagttataaatgaaattcctaatatcggttatgaagtgaaattgaatttctacttgatctttctctctatttttgtaaaataaaattaagaatatttaaatattcaatgattcatttttgcagaaatcggaggaagaagaatatatgaaaacatttaacatttctcaacaagatccccccatattgttgtataagtgatgaaatactgaattcaaaacttagtttatatgtggtaaaatgttttaatcaagtttaggaggaattaattatgaagtgtaatgaataatgaatgtaacagggttcaattaaaagagggaagcgtatcattaaccctataaactacgtctgccctcattattggagggtgaaatgtgaatacatcctattcacaatcgaatttacgacacaaccaaattttaatttggctttgcattttatctttttttagcgtattaaatgaaatggttttgaacgtgtcattacctgatattgcaaatgattttaataaaccaccagcgagtacaaactgggtgaacacagcctttatgttgaccttttccattggaacagctgtatatggaaagctatctgatcaattaggcatcaaaaggttactcctatttggaattataataaattgtttcgggtcggtaattgggtttgttggccattctttcttttccttacttattatggctcgttttattcaaggggctggtgcagctgcatttccagcactcgtaatggttgtagttgcgcgctatattccaaaggaaaataggggtaaagcatttggtcttattggatcgatagtagccatgggagaaggagtcggtccagcgattggtggaatgatagcccattatattcattggtcctatcttctactcattcctatgataacaattatcactgttccgtttcttatgaaattattaaagaaagaagtaaggataaaaggtcattttgatatcaaaggaattatactaatgtctgtaggcattgtattttttatgttgtttacaacatcatatagcatttcttttcttatcgttagcgtgctgtcattcctgatatttgtaaaacatatcaggaaagtaacagatccttttgttgatcccggattagggaaaaatataccttttatgattggagttctttgtgggggaattatatttggaacagtagcagggtttgtctctatggttccttatatgatgaaagatgttcaccagctaagtactgccgaaatcggaagtgtaattattttccctggaacaatgagtgtcattattttcggctacattggtgggatacttgttgatagaagaggtcctttatacgtgttaaacatcggagttacatttctttctgttagctttttaactgcttcctttcttttagaaacaacatcatggttcatgacaattataatcgtatttgttttaggtgggctttcgttcaccaaaacagttatatcaacaattgtttcaagtagcttgaaacagcaggaagctggtgctggaatgagtttgcttaactttaccagctttttatcagagggaacaggtattgcaattgtaggtggtttattatccatacccttacttgatcaaaggttgttacctatggaagttgatcagtcaacttatctgtatagtaatttgttattacttttttcaggaatcattgtcattagttggctggttaccttgaatgtatataaacattctcaaagggatttctaaatcgttaagggatcaactttgggagagagttcaaaattgatcctttttttataacaggaattcggcatcaaataaaacgaaaggctcagtcgaaagactgggcctttcgttttatctgttgtttgtcggtgaacgctctcctgagtaggacaaatccgccgggagcggatttgaacgttgcgaagcaacggcccggagggtggcgggcaggacgcccgccataaactgccaggcatcaaattaagcagaaggccatcctgacggatggcctttttgcgtttctacaaactcttcctgtcgtcatatctacaattctacacagcccagtccagactattcggcactgaaattatgggtgaagtggtcaagacctcactaggcaccttaaaaatagcgcaccctgaagaagatttatttgaggtagcccttgcctacctagcttccaagaaagatatcctaacagcacaagagcggaaagatgttttgttctacatccagaacaacctctgctaaaattcctgaaaaattttgcaaaaagttgttgactttatctacaaggtgtggcataatgtgtggaattgtgagcggataacaattaagctaattctatggtaaaagcattcctgaacccaatatccttatttttagtggacaaggccttgttctcatatggttgcttgagccagtgccttacaaggctcttccgctttggcaggctgttcaaaattatttattagagcaactcaaggaactaggcggagatccaaaagcaaccgatgcagcacgtgtttttcggattgctgggagcgtcaatagtaagaatggagcggaagtaagagcggaatatcggcacgattacagatatgagttaaggcagattcaatttgattaccttccagaactcaatgaggttattaatcccgctccacaaaagaaaaaacgggggcgtaaaaagaaagtagttcagttattcaatacctacaaactccattacgctcgcctattggatatagtgaaattggtggaactacgaaattatgaggtaactggatacagggaaatcatttgctttttataccgttattggttgtgctgttacacgaacgaccctgtagaggctttaaatcaaacacagacacttaatttacagttcactgagcctttacccttaaaagaggttgaaagggctacacggagcgcagaaaaggcgtgggaagcacgaaataacgaagaggctaaccggattgcaatcgaaaaaggatatcccagtgctggatacaatattagcaataaaaagttgattgaatggctagatatcacaccagaagaacagaagcatttacagacgattatagacgctaatgagaaacggagaagaaagcgggaaagggataggatttatcaagaacaaaaacgtcgtgagcggggagatatgacccgacaggagtatattaagcaacaacaggataaaacagatgataaattatttaaattgcaggagttattagaacagaatcccaaaatctcaaaaattaaattagcaaaaatacttggtgtagataaatcgcacttatacagactgctgaaacaactataactggaaaaaattagtgtctcatggttcgtcgcccttatattatgggcgttagcctgcttgctaattggataggtgttattgtcatttcaacgtcggacgttttggtagatgaacgtcggacgttatttgcttcaatagattgttgatgtattaagggttgcagtgaatcgacaagcaaaaagttatgacgttgtgaaaaaattgaatagaaaattggaaattacgtcggacgttctaacttaaaaaccctgttatatcaatgatttaaaaggaaattaacgtcataaaagacctttctgcaacaaaagtttttctggaagagttgaggttattttataggtattatggacttttgtagactttttgtgtactttttgtggactccacactcgctggtatcgtgttattttttaattgagatatgaatatggaaattaaacgttttaggcgttggtttggtgatgacaaaaaaataagagtacccgctcacaacggatactctttcgagaaatgtacgaaacgctataaataaaaaataactagatacatttacattgtatcacgtttcgtacatttctccaataacaaattgattggaggaatgcaaagtgaataatgaaccagtaaaacgtggtaagaagaacagatgggaattaaacctacctataatgacttatgtagtagctgatgattggattgataaactaggacacgaaacgtttactttatggttgaggttccatacttgggtagatagagaagatgaactccgagattatgatcgcatacctagaagttttgagaacatatataaaaagacactaggaatctcaaaaagtaagttttatagattgataaaacctttatgggaatatggattaatagacatcatagaatacgaagaatctaaccgtaattctactaaacctaaaaatataattgtttatgagtatcctttacacgaaatagaaagaaagtataaaccactagaaaaattaagagattgggataaagactataattccgtttctaaagaattaggtaaaacaggtggtagaccaaggaaaaaagatagtgaagaagaacccgaaaagaaacccgaagaagtaactaaaaagaaacgtaaatataagttaaaaagagttatccacaacggtttcaaaaatgaaacggtggagggtttcaaaaatgaaacggtggagggtttcaaaaatgaaacggtgaccgtttcaaaaataaaacccaataattattcaaatatctttaataacttatcaaatatttctactaatgtttcaaataatttattaattgatgatgatgaggaaatcgaaaatgaaccaactggtcgtacaataaataggtcattacttttttcacaagaagatattaaacaggcctatcaatttattaatagattttcagttatacagttacgtgaaaactttagctttgataaacactttgaagaacggttggtatgttatttatggaaagcagggatttctactttttacacgcacgaaatcagtaaaatgataaaaaaaatagcagactatgaaaaatctaaaaaaggtagattaaacccaatacgtgaccgagccttatatatggtaaatggtcttgtaatgaatagagcttcttcccaaagtgaacatgctacttataaactaaaccaatataaaaaacagaaggaacaggaaaaacaacaacaggagcaacaaagatcaagagtaccgttctataattggttggaggaaagagaagaacaaaccgaaggtcaactacccaccacttaaagcctaacggcttttgaagtggggcttgtaaaaagccctagttgactaccccaagtctttcgaggactacgttggaaaggtcatgacacctacaaatgctcctctagttcgtagccactgtcgttgatggttaaaagtcctgatgggtagggacggtgctgtcaacatcacaagcccttccaacatgggggaagaggaagaacactccgagaaaggagggggctgtcgtacacgccttgttcgtgtacgtgatttttaacacttttatctctaatataatctctccttgagttagcagagactaagaataaaacacattaggattttttatctacatgtttgagtcggctgaaagatcgtacgtaccaattattgtttcgtgattgttcaagccataacactgtagggatagtggaaagagtgcttcatctggttacgatcaatcaaatattcaaacggagggacacgattttgatgaaaccagtaacgttatacgatgtcgcagagtatgccggtgtctcttatcagaccgtttcccgcgtggtgaaccaggccagccacgtttctgcgaaaacgcgggaaaaagtggaagcggcgatggcggagctgaattacattcccaaccgcgtggcacaacaactggcgggcaaacagtcgttgctgattggcgttgccacctccagtctggccctgcacgcgccgtcgcaaattgtcgcggcgattaaatctcgcgccgatcaactgggtgccagcgtggtggtgtcgatggtagaacgaagcggcgtcgaagcctgtaaaacggcggtgcacaatcttctcgcgcaacgcgtcagtgggctgatcattaactatccgctggatgaccaggatgccattgctgtggaagctgcctgcactaatgttccggcgttatttcttgatgtctctgaccagacacccatcaacagtattattttctcccatgaagatggtacgcgactgggcgtggagcatctggtcgcattgggtcaccagcaaatcgcgctgttagcgggcccattaagttctgtctcggcgcgtctgcgtctggctggctggcataaatatctcactcgcaatcaaattcagccgatagcggaacgggaaggcgactggagtgccatgtccggttttcaacaaaccatgcaaatgctgaatgagggcatcgttcccactgcgatgctggttgccaacgatcagatggcgctgggcgcaatgcgcgccattaccgagtccgggctgcgcgttggtgcggatatctcggtagtgggatacgacgataccgaagatagctcatgttatatcccgccgcttaccaccatcaaacaggattttcgcctgctggggcaaaccagcgtggaccgcttgctgcaactctctcagggccaggcggtgaagggcaatcagctgttgcccgtgtcactggtgaaaagaaaaaccaccctggcgcccaatacgcaaaccgcctctccccgcgcgttggccgattcattaatgcagctggcacgacaggtttcccgactggaaagcgggcagtgagcgcaacgcaattaatgtgagttaggatcgctaccttaagagacacgcgttatcgggggttagttcgtcatcattgatgagggttgattatcacagtttattactctgaattggctatccgcgtgtgtacctctacctggagtttttcccacggtggatatttcttcttgcgctgagcgtaagagctatctgacagaaacagttcttctttgcttcctcgccagttcgctcgctatgctcggttacacggctgcggcgagcgctagtggataataagtgactgaggtatgtgctcttcttatctccttttgtagtgttgctcttattttaaacaactttgcggttttttgatgactttgcgattttgttgttgctttgcagtaaattgcaagatttaataaaaaaacgcaaagcaatgattaaaggatgttcagaatgaaactcatggaaacacttaaccagtgcataaacgctggtcatgaaatgacgaaggctatcgccattgcacagtttaatgatgacagcccggaagcgaggaaaataacccggcgctggagaataggtgaagcagcggatttagttggggtttcttctcaggctatcagagatgccgagaaagcagggcgactaccgcacccggatatggaaattcgaggacgggttgagcaacgtgttggttatacaattgaacaaattaatcatatgcgtgatgtgtttggtacgcgattgcgacgtgctgaggacgtatttccaccggtgatcggggttgctgcccataaaggtggcgtttacaaaacctcagtttctgttcatcttgctcaggatctggctctgaaggggctacgtgttttgctcgtggaaggtaacgacccccagggaacagcctcaatgtatcacggatgggtaccagatcttcatattcatgcagaggacactctcctgcctttctatcttggggaaaaggacgatgtcacttatgcaataaagcccacttgctggccggggcttgacattattccttcctgtctggctctgcaccgtattgaaactgagttaatgggcaaatttgatgaaggtaaactgcccaccgatccacacctgatgctccgactggccattgaaactgttgctcatgactatgatgtcatagttattgacagcgcgcctaacctgggtatcggcacgattaatgtcgtatgtgctgctgatgtgctgattgttcccacgcctgctgagttgtttgactacacctccgcactgcagtttttcgatatgcttcgtgatctgctcaagaacgttgatcttaaagggttcgagcctgatgtacgtattttgcttaccaaatacagcaatagtaatggctctcagtccccgtggatggaggagcaaattcgggatgcctggggaagcatggttctaaaaaatgttgtacgtgaaacggatgaagttggtaaaggtcagatccggatgagaactgtttttgaacaggccattgatcaacgctcttcaactggtgcctggagaaatgctctttctatttgggaacctgtctgcaatgaaattttcgatcgtctgattaaaccacgctgggagattagataatgaagcgtgcgcctgttattccaaaacatacgctcaatactcaaccggttgaagatacttcgttatcgacaccagctgccccgatggtggattcgttaattgcgcgcgtaggagtaatggctcgcggtaatgccattactttgcctgtatgtggtcgggatgtgaagtttactcttgaagtgctccggggtgatagtgttgaaaagacctctcgggtatggtcaggtaatgaacgtgaccaggagctgcttactgaggacgcactggatgatctcatcccttcttttctactgactggtcaacagacaccggcgttcggtcgaagagtatctggtgtcatagaaattgccgatgggagtcgccgtcgtaaagctgctgcacttaccgaaagtgattatcgtgttctggttggcgagctggatgatgagcagatggctgcattatccagattgggtaacgattatcgcccaacaagtgcttatgaacgtggtcagcgttatgcaagccgattgcagaatgaatttgctggaaatatttctgcgctggctgatgcggaaaatatttcacgtaagattattacccgctgtatcaacaccgccaaattgcctaaatcagttgttgctcttttttctcaccccggtgaactatctgcccggtcaggtgatgcacttcaaaaagcctttacagataaagaggaattacttaagcagcaggcatctaaccttcatgagcagaaaaaagctggggtgatatttgaagctgaagaagttatcactcttttaacttctgtgcttaaaacgtcatctgcatcaagaactagcttaagctcacgacatcagtttgctcctggagcgacagtattgtataagggcgataaaatggtgcttaacctggacaggtcccgtgttccaactgagtgtatagagaaaattgaggccattcttaaggaacttgaaaagccagcaccctgatgcgaccacgttttagtctacgtttatctgtctttacttaatgtcctttgttacaggccagaaagcataactggcctgaatattctctctgggcccactgttccacttgtatcgtcggtctgataatcagactgggaccacggtcccactcgtatcgtcggtctgattattagtctgggaccacggtcccactcgtatcgtcggtctgattattagtctgggaccacggtcccactcgtatcgtcggtctgataatcagactgggaccacggtcccactcgtatcgtcggtctgattattagtctgggaccatggtcccactcgtatcgtcggtctgattattagtctgggaccacggtcccactcgtatcgtcggtctgattattagtctggaaccacggtcccactcgtatcgtcggtctgattattagtctgggaccacggtcccactcgtatcgtcggtctgattattagtctgggaccacgatcccactcgtgttgtcggtctgattatcggtctgggaccacggtcccacttgtattgtcgatcagactatcagcgtgagactacgattccatcaatgcctgtcaagggcaagtattgacatgtcgtcgtaacctgtagaacggagtaacctcggtgtgcggttgtatgcctgctgtggattgctgctgtgtcctgcttatccacaacattttgcgcacggttatgtggacaaaatacctggttacccaggccgtgccggcacgttaaccgggctgcatccgatgcaagtgtgtcgctgtcgacgagctcgcgagctcgattcgat

SEQ ID NO: 26 - DNA, 16499 bp, Artificial Sequence
  OGAB vector2.1
gcgaccgcaagcttgaagagctcttctttcagaacgctcggttgccgccgggcgttttttatgacggtcattacaacggttatacgacgccacgcgtagtgagacatacacgttcgttggatccgggttcactttggttcatgtgcagctccatcagcaaaaggggatgataagtttatcaccaccgactatttgcaacagtgccgttgatcgtgctatgatcgactgatgtcatcagcggtggagtgcaatgtcgtgcaatacgaatggcgaaaagccgagctcatcggtcagcttctcaaccttggggttacccccggcggtgtgctgctggtccacagctccttccgtagcgtccggcccctcgaagatgggccacttggactgatcgaggccctgcgtgctgcgctgggtccgggagggacgctcgtcatgccctcgtggtcaggtctggacgacgagccgttcgatcctgccacgtcgcccgttacaccggaccttggagttgtctctgacacattctggcgcctgccaaatgtaaagcgcagcgcccatccatttgcctttgcggcagcggggccacaggcagagcagatcatctctgatccattgcccctgccacctcactcgcctgcaagcccggtcgcccgtgtccatgaactcgatgggcaggtacttctcctcggcgtgggacacgatgccaacacgacgctgcatcttgccgagttgatggcaaaggttccctatggggtgccgagacactgcaccattcttcaggatggcaagttggtacgcgtcgattatctggagaatgaccactgctgtgagcgctttgccttggcggacaggtggctcaaggagaagagccttcagaaggaaggtccagtcggtcatgcctttgctcggttgatccgctcccgcgacattgtggcgacagccctgggtcaactgggccgagatccgttgatcttcctgcatccgccagaggcgggatgcgaagaatgcgatgccgctcgccagtcgattggctgagctcatgagcggagaacgagatgacgttggaggggcaaggtcgcgctgattgctggggcaacacgtggagcggatcggggattgtctttcttcagctcgctgatgatatgccttcctggttggcttggtttcatcagccatccgcttgccctcatctgttacgccggcggtagccggccagcctcgcagagcaggattcccgttgagcaccgccaggtgcgaataagggacagtgaagaaggaacacccgctcgcgggtgggcctacttcacctatcctgcccggctgacgccgttggatacaccaaggaaagtctacacgaaccctttggcaaaatcctgtatatcgtgcgaaaaaggatggatataccgaaaaaatcgctataatgaccccgaagcagggttatgcagcggaaaagatccgtcgacctgcaggcatgcaagctctagcgattccagacgtcccgaaggcgtggcgcggcttccccgtgccggagcaatcgccctgggtgggttacacgacgcccctctatggcccgtactgacggacacaccgaagccccggcggcaaccctcagcggatgccccggggcttcacgttttcccaggtcagaagcggttttgtttcgggtgctgggttgttgtctctggacagtgatccatgggaaactactcagcaccaccaatgttcccaaaagaaagcgcaggtcagcgcccatgagccaagatctaggcatgtcgcccttcatcgctcccgacgtccctgagcaccttctagacactgttcgcgtcttcctgtacgcgcgtcagtctaagggccggtccgacggctcagacgtgtcgaccgaagcacagctagcggccggtcgtgcgttggtcgcctctcgcaacgcccaggggggtgcgcgctgggtcgtggcaggtgagttcgtggacgtcgggcgctccggctgggacccgaacgtgacccgtgccgacttcgagcgcatgatgggcgaagtccgcgccggcgaaggtgacgttgtcgttgtgaatgagctttcccggctcactcgcaagggcgcccatgacgcgctcgaaatcgacaacgaattgaagaagcacggcgtgcgcttcatgtcggttcttgagccgttccttgacacgtctacccctatcggcgtcgccattttcgcgctgatcgctgcccttgcgaaacaggacagtgacctgaaggcggagcgcctgaagggtgcgaaagacgagattgccgcgctgggtggcgttcactcgtcttccgccccgttcggaatgcgcgccgtgcgcaagaaggtcgataatctcgtgatctccgttcttgagccggacgaagacaacccggatcacgtcgagctagttgagcgcatggcgaaaatgtcgttcgaaggcgtgtccgacaacgccattgcaacgaccttcgagaaggaaaagatcccgtcgcccggaatggctgagcggcgcgccacggaaaagcgtcttgcgtccatcaaggcacgtcgcctgaacggcgctgaaaagccgatcatgtggcgcgctcaaacggtccgatggattctcaaccatcccgcaatcggcggtttcgcattcgagcgtgtgaagcacggtaaggcgcacatcaacgtcatacggcgcgaccccggcggcaagccgctaacgccccacacgggcattctcagcggctcgaagtggcttgagcttcaagagaagcgttccgggaagaatctcagcgaccggaagcctggggccgaagtcgaaccgacgcttctgagcgggtggcgtttcctggggtgccgaatctgcggcggctcaatgggtcagtcccagggtggccgtaagcgcaacggcgaccttgccgaaggcaattacatgtgcgccaacccgaaggggcacggcggcttgtcggtcaagcgcagcgaactggacgaattcgttgcttcgaaggtgtgggcacggctccgcacagccgacatggaagatgaacacgatcaggcatggattgccgccgctgcggagcgcttcgcccttcagcacgacctagcgggggtggccgatgagcggcgcgaacaacaggcgcacctagacaacgtgcggcgctccatcaaggaccttcaggcggaccgtaaggccggtctgtacgtcgggcgtgaagagctggaaacgtggcgctcaacggtgctgcaataccggtcctacgaagcggagtgcacgacccgactcgctgagcttgacgagaagatgaacggcagcacccgcgttccgtctgagtggttcagcggcgaagacccgacggccgaagggggcatctgggcaagctgggacgtgtacgagcgtcgggagttcctgagcttcttccttgactccgtcatggtcgaccgggggcgccaccctgaaaccaagaaatacatccccctgaaggaccgtgtgacgctcaagtgggcggagctgctgaaggaggaagacgaagcgagcgaagccactgagcgggagcttgcggcgctgtagcgagacacccgggaagcctgatctacgtctgtcgagaagtttcgatgacactcgttcgttcacacgttgcagcatggatccctcgaggagttactggccctgatttctccgcttctaataccgcacatgcggccgcaagctgtctcgacggcgcgcctagaaacaaggcagttccgggctgaaagtagcgccgggactagtcttaattaacggcctgtttggccattatgagacgccctgatgacttgacgctcgagaaggttcacgattagcatgccggttacggacctttgaggagggctcaatgctttccaagggcgaggaggacaacatggccatcatcaaggagttcatgcgcttcaaggtccacatggagggctccgtcaacgggcacgagttcgagatcgagggcgagggggagggccggccgtacgagggcacccagaccgccaagctgaaggtgaccaagggcggccccctcccgttcgcctgggacatcctctccccccagttcatgtacggctcgaaggcctacgtcaagcacccggccgacatcccggactacctgaagctctcgttcccggaggggttcaagtgggagcgggtcatgaacttcgaggacggcggcgtcgtcaccgtcacccaggacagctccctgcaggacggcgagttcatctacaaggtcaagctgcggggcacgaacttcccgagcgacggccccgtgatgcagaagaaaacgatgggctgggaagcgtcctcggagcgcatgtacccggaggacggcgccctcaagggcgagatcaagcagcgcctgaagctgaaggacggcggccactacgacgccgaagtcaagacgacgtacaaggccaagaagccggtgcagctcccggacgcctacaacgtgaacatcaagctcgacatcacctcgcacaacgaggactacacgatcgtggagcagtacgagcgcgccgagggccggcactcgaccggcggcatggacgagctgtacaagtgatgacgtctctaaaatccccggataactgccttaaaaaaagaataaatgccttggcctttatatggaaatgtggaactgagtggatatgctgtttttgtctgttaaacagagaagctggctgttatccactgagaagcgaacgaaacagtcgggaaaatctcccattatcgtagagatccgcattattaatctcaggagcctgtgtagcgtttataggaagtagtgttctgtcatgatgcctgcaagcggtaacacgatttgaatatgccttcaggaacaatagaaatcttcgtgcggtgttacgttgaagtggagcggattatgtcagcaatggacagaacaacctaatgaacacagaaccatgatgtggtctgtccttttacagccagtagtgctcgccgcagtcgagcgacagttcgaagccatcgagtgagcgaggaagcaccagggaacagcacttatatattctgcttacacacgatgcctgaaaaaacttcccttggggttatccacttatccacggggatatttttataattattttttttatagtttttagatcttcttttttagagcgccttgtaggcctttatccatgctggttctagagaaggtgttgtgacaaattgccctttcagtgtgacaaatcaccctcaaatgacagtcctgtctgtgacaaattgcccttaaccctgtgacaaattgccctcagaagaagctgttttttcacaaagttatccctgcttattgactcttttttatttagtgtgacaatctaaaaacttgtcacacttcacatggatctgtcatggcggaaacagcggttatcaatcacaagaaacgtaaaaatagcccgcgaatcgtccagtcaaacgacctcactgaggcggcatatagtctctcccgggatcaaaaacgtatgctgtatctgttcgttgaccagatcagaaaatctgatggcaccctacaggaacatgacggtatctgcgagatccatgttgctaaatatgctgaaatattcggattgacctctgcggaagccagtaaggatatacggcaggcattgaagagtttcgcggggaaggaagtggttttttatcgccctgaagaggatgccggcgatgaaaaaggctatgaatcttttccttggtttatcaaacgtgcgcacagtccatccagagggctttacagtgtacatatcaacccatatctcattcccttctttatcgggttacagaaccggtttacgcagtttcggcttagtgaaacaaaagaaatcaccaatccgtatgccatgcgtttatacgaatccctgtgtcagtatcgtaagccggatggctcaggcatcgtgtctctgaaaatcgactggatcatagagcgttaccagctgcctcaaagttaccagcgtatgcctgacttccgccgccgcttcctgcaggtctgtgttaatgagatcaacagcagaactccaatgcgcctctcatacattgagaaaaagaaaggccgccagacgactcatatcgtattttccttccgcgatatcacttccatgacgacaggatagtctgagggttatctgtcacagatttgagggtggttcgtcacatttgttctgacctactgagggtaatttgtcacagttttgctgtttccttcagcctgcatggattttctcatactttttgaactgtaatttttaaggaagccaaatttgagggcagtttgtcacagttgatttccttctctttcccttcgtcatgtgacctgatacgcgtgctaccttaagagagtcaattcgcccttcccggtcgatatgaacagcttatttacataattcacgttattggtagttataaatgaaattcctaatatcggttatgaagtgaaattgaatttctacttgatctttctctctatttttgtaaaataaaattaagaatatttaaatattcaatgattcatttttgcagaaatcggaggaagaagaatatatgaaaacatttaacatttctcaacaagatccccccatattgttgtataagtgatgaaatactgaattcaaaacttagtttatatgtggtaaaatgttttaatcaagtttaggaggaattaattatgaagtgtaatgaataatgaatgtaacagggttcaattaaaagagggaagcgtatcattaaccctataaactacgtctgccctcattattggagggtgaaatgtgaatacatcctattcacaatcgaatttacgacacaaccaaattttaatttggctttgcattttatctttttttagcgtattaaatgaaatggttttgaacgtgtcattacctgatattgcaaatgattttaataaaccaccagcgagtacaaactgggtgaacacagcctttatgttgaccttttccattggaacagctgtatatggaaagctatctgatcaattaggcatcaaaaggttactcctatttggaattataataaattgtttcgggtcggtaattgggtttgttggccattctttcttttccttacttattatggctcgttttattcaaggggctggtgcagctgcatttccagcactcgtaatggttgtagttgcgcgctatattccaaaggaaaataggggtaaagcatttggtcttattggatcgatagtagccatgggagaaggagtcggtccagcgattggtggaatgatagcccattatattcattggtcctatcttctactcattcctatgataacaattatcactgttccgtttcttatgaaattattaaagaaagaagtaaggataaaaggtcattttgatatcaaaggaattatactaatgtctgtaggcattgtattttttatgttgtttacaacatcatatagcatttcttttcttatcgttagcgtgctgtcattcctgatatttgtaaaacatatcaggaaagtaacagatccttttgttgatcccggattagggaaaaatataccttttatgattggagttctttgtgggggaattatatttggaacagtagcagggtttgtctctatggttccttatatgatgaaagatgttcaccagctaagtactgccgaaatcggaagtgtaattattttccctggaacaatgagtgtcattattttcggctacattggtgggatacttgttgatagaagaggtcctttatacgtgttaaacatcggagttacatttctttctgttagctttttaactgcttcctttcttttagaaacaacatcatggttcatgacaattataatcgtatttgttttaggtgggctttcgttcaccaaaacagttatatcaacaattgtttcaagtagcttgaaacagcaggaagctggtgctggaatgagtttgcttaactttaccagctttttatcagagggaacaggtattgcaattgtaggtggtttattatccatacccttacttgatcaaaggttgttacctatggaagttgatcagtcaacttatctgtatagtaatttgttattacttttttcaggaatcattgtcattagttggctggttaccttgaatgtatataaacattctcaaagggatttctaaatcgttaagggatcaactttgggagagagttcaaaattgatcctttttttataacaggaattcggcatcaaataaaacgaaaggctcagtcgaaagactgggcctttcgttttatctgttgtttgtcggtgaacgctctcctgagtaggacaaatccgccgggagcggatttgaacgttgcgaagcaacggcccggagggtggcgggcaggacgcccgccataaactgccaggcatcaaattaagcagaaggccatcctgacggatggcctttttgcgtttctacaaactcttcctgtcgtcatatctacaattctacacagcccagtccagactattcggcactgaaattatgggtgaagtggtcaagacctcactaggcaccttaaaaatagcgcaccctgaagaagatttatttgaggtagcccttgcctacctagcttccaagaaagatatcctaacagcacaagagcggaaagatgttttgttctacatccagaacaacctctgctaaaattcctgaaaaattttgcaaaaagttgttgactttatctacaaggtgtggcataatgtgtggaattgtgagcggataacaattaagctaattctatggtaaaagcattcctgaacccaatatccttatttttagtggacaaggccttgttctcatatggttgcttgagccagtgccttacaaggctcttccgctttggcaggctgttcaaaattatttattagagcaactcaaggaactaggcggagatccaaaagcaaccgatgcagcacgtgtttttcggattgctgggagcgtcaatagtaagaatggagcggaagtaagagcggaatatcggcacgattacagatatgagttaaggcagattcaatttgattaccttccagaactcaatgaggttattaatcccgctccacaaaagaaaaaacgggggcgtaaaaagaaagtagttcagttattcaatacctacaaactccattacgctcgcctattggatatagtgaaattggtggaactacgaaattatgaggtaactggatacagggaaatcatttgctttttataccgttattggttgtgctgttacacgaacgaccctgtagaggctttaaatcaaacacagacacttaatttacagttcactgagcctttacccttaaaagaggttgaaagggctacacggagcgcagaaaaggcgtgggaagcacgaaataacgaagaggctaaccggattgcaatcgaaaaaggatatcccagtgctggatacaatattagcaataaaaagttgattgaatggctagatatcacaccagaagaacagaagcatttacagacgattatagacgctaatgagaaacggagaagaaagcgggaaagggataggatttatcaagaacaaaaacgtcgtgagcggggagatatgacccgacaggagtatattaagcaacaacaggataaaacagatgataaattatttaaattgcaggagttattagaacagaatcccaaaatctcaaaaattaaattagcaaaaatacttggtgtagataaatcgcacttatacagactgctgaaacaactataactggaaaaaattagtgtctcatggttcgtcgcccttatattatgggcgttagcctgcttgctaattggataggtgttattgtcatttcaacgtcggacgttttggtagatgaacgtcggacgttatttgcttcaatagattgttgatgtattaagggttgcagtgaatcgacaagcaaaaagttatgacgttgtgaaaaaattgaatagaaaattggaaattacgtcggacgttctaacttaaaaaccctgttatatcaatgatttaaaaggaaattaacgtcataaaagacctttctgcaacaaaagtttttctggaagagttgaggttattttataggtattatggacttttgtagactttttgtgtactttttgtggactccacactcgctggtatcgtgttattttttaattgagatatgaatatggaaattaaacgttttaggcgttggtttggtgatgacaaaaaaataagagtacccgctcacaacggatactctttcgagaaatgtacgaaacgctataaataaaaaataactagatacatttacattgtatcacgtttcgtacatttctccaataacaaattgattggaggaatgcaaagtgaataatgaaccagtaaaacgtggtaagaagaacagatgggaattaaacctacctataatgacttatgtagtagctgatgattggattgataaactaggacacgaaacgtttactttatggttgaggttccatacttgggtagatagagaagatgaactccgagattatgatcgcatacctagaagttttgagaacatatataaaaagacactaggaatctcaaaaagtaagttttatagattgataaaacctttatgggaatatggattaatagacatcatagaatacgaagaatctaaccgtaattctactaaacctaaaaatataattgtttatgagtatcctttacacgaaatagaaagaaagtataaaccactagaaaaattaagagattgggataaagactataattccgtttctaaagaattaggtaaaacaggtggtagaccaaggaaaaaagatagtgaagaagaacccgaaaagaaacccgaagaagtaactaaaaagaaacgtaaatataagttaaaaagagttatccacaacggtttcaaaaatgaaacggtggagggtttcaaaaatgaaacggtggagggtttcaaaaatgaaacggtgaccgtttcaaaaataaaacccaataattattcaaatatctttaataacttatcaaatatttctactaatgtttcaaataatttattaattgatgatgatgaggaaatcgaaaatgaaccaactggtcgtacaataaataggtcattacttttttcacaagaagatattaaacaggcctatcaatttattaatagattttcagttatacagttacgtgaaaactttagctttgataaacactttgaagaacggttggtatgttatttatggaaagcagggatttctactttttacacgcacgaaatcagtaaaatgataaaaaaaatagcagactatgaaaaatctaaaaaaggtagattaaacccaatacgtgaccgagccttatatatggtaaatggtcttgtaatgaatagagcttcttcccaaagtgaacatgctacttataaactaaaccaatataaaaaacagaaggaacaggaaaaacaacaacaggagcaacaaagatcaagagtaccgttctataattggttggaggaaagagaagaacaaaccgaaggtcaactacccaccacttaaagcctaacggcttttgaagtggggcttgtaaaaagccctagttgactaccccaagtctttcgaggactacgttggaaaggtcatgacacctacaaatgctcctctagttcgtagccactgtcgttgatggttaaaagtcctgatgggtagggacggtgctgtcaacatcacaagcccttccaacatgggggaagaggaagaacactccgagaaaggagggggctgtcgtacacgccttgttcgtgtacgtgatttttaacacttttatctctaatataatctctccttgagttagcagagactaagaataaaacacattaggattttttatctacatgtttgagtcggctgaaagatcgtacgtaccaattattgtttcgtgattgttcaagccataacactgtagggatagtggaaagagtgcttcatctggttacgatcaatcaaatattcaaacggagggacacgattttgatgaaaccagtaacgttatacgatgtcgcagagtatgccggtgtctcttatcagaccgtttcccgcgtggtgaaccaggccagccacgtttctgcgaaaacgcgggaaaaagtggaagcggcgatggcggagctgaattacattcccaaccgcgtggcacaacaactggcgggcaaacagtcgttgctgattggcgttgccacctccagtctggccctgcacgcgccgtcgcaaattgtcgcggcgattaaatctcgcgccgatcaactgggtgccagcgtggtggtgtcgatggtagaacgaagcggcgtcgaagcctgtaaaacggcggtgcacaatcttctcgcgcaacgcgtcagtgggctgatcattaactatccgctggatgaccaggatgccattgctgtggaagctgcctgcactaatgttccggcgttatttcttgatgtctctgaccagacacccatcaacagtattattttctcccatgaagatggtacgcgactgggcgtggagcatctggtcgcattgggtcaccagcaaatcgcgctgttagcgggcccattaagttctgtctcggcgcgtctgcgtctggctggctggcataaatatctcactcgcaatcaaattcagccgatagcggaacgggaaggcgactggagtgccatgtccggttttcaacaaaccatgcaaatgctgaatgagggcatcgttcccactgcgatgctggttgccaacgatcagatggcgctgggcgcaatgcgcgccattaccgagtccgggctgcgcgttggtgcggatatctcggtagtgggatacgacgataccgaagatagctcatgttatatcccgccgcttaccaccatcaaacaggattttcgcctgctggggcaaaccagcgtggaccgcttgctgcaactctctcagggccaggcggtgaagggcaatcagctgttgcccgtgtcactggtgaaaagaaaaaccaccctggcgcccaatacgcaaaccgcctctccccgcgcgttggccgattcattaatgcagctggcacgacaggtttcccgactggaaagcgggcagtgagcgcaacgcaattaatgtgagttaggatcgctaccttaagagacacgcgttatcgggggttagttcgtcatcattgatgagggttgattatcacagtttattactctgaattggctatccgcgtgtgtacctctacctggagtttttcccacggtggatatttcttcttgcgctgagcgtaagagctatctgacagaaacagttcttctttgcttcctcgccagttcgctcgctatgctcggttacacggctgcggcgagcgctagtggataataagtgactgaggtatgtgctcttcttatctccttttgtagtgttgctcttattttaaacaactttgcggttttttgatgactttgcgattttgttgttgctttgcagtaaattgcaagatttaataaaaaaacgcaaagcaatgattaaaggatgttcagaatgaaactcatggaaacacttaaccagtgcataaacgctggtcatgaaatgacgaaggctatcgccattgcacagtttaatgatgacagcccggaagcgaggaaaataacccggcgctggagaataggtgaagcagcggatttagttggggtttcttctcaggctatcagagatgccgagaaagcagggcgactaccgcacccggatatggaaattcgaggacgggttgagcaacgtgttggttatacaattgaacaaattaatcatatgcgtgatgtgtttggtacgcgattgcgacgtgctgaggacgtatttccaccggtgatcggggttgctgcccataaaggtggcgtttacaaaacctcagtttctgttcatcttgctcaggatctggctctgaaggggctacgtgttttgctcgtggaaggtaacgacccccagggaacagcctcaatgtatcacggatgggtaccagatcttcatattcatgcagaggacactctcctgcctttctatcttggggaaaaggacgatgtcacttatgcaataaagcccacttgctggccggggcttgacattattccttcctgtctggctctgcaccgtattgaaactgagttaatgggcaaatttgatgaaggtaaactgcccaccgatccacacctgatgctccgactggccattgaaactgttgctcatgactatgatgtcatagttattgacagcgcgcctaacctgggtatcggcacgattaatgtcgtatgtgctgctgatgtgctgattgttcccacgcctgctgagttgtttgactacacctccgcactgcagtttttcgatatgcttcgtgatctgctcaagaacgttgatcttaaagggttcgagcctgatgtacgtattttgcttaccaaatacagcaatagtaatggctctcagtccccgtggatggaggagcaaattcgggatgcctggggaagcatggttctaaaaaatgttgtacgtgaaacggatgaagttggtaaaggtcagatccggatgagaactgtttttgaacaggccattgatcaacgctcttcaactggtgcctggagaaatgctctttctatttgggaacctgtctgcaatgaaattttcgatcgtctgattaaaccacgctgggagattagataatgaagcgtgcgcctgttattccaaaacatacgctcaatactcaaccggttgaagatacttcgttatcgacaccagctgccccgatggtggattcgttaattgcgcgcgtaggagtaatggctcgcggtaatgccattactttgcctgtatgtggtcgggatgtgaagtttactcttgaagtgctccggggtgatagtgttgaaaagacctctcgggtatggtcaggtaatgaacgtgaccaggagctgcttactgaggacgcactggatgatctcatcccttcttttctactgactggtcaacagacaccggcgttcggtcgaagagtatctggtgtcatagaaattgccgatgggagtcgccgtcgtaaagctgctgcacttaccgaaagtgattatcgtgttctggttggcgagctggatgatgagcagatggctgcattatccagattgggtaacgattatcgcccaacaagtgcttatgaacgtggtcagcgttatgcaagccgattgcagaatgaatttgctggaaatatttctgcgctggctgatgcggaaaatatttcacgtaagattattacccgctgtatcaacaccgccaaattgcctaaatcagttgttgctcttttttctcaccccggtgaactatctgcccggtcaggtgatgcacttcaaaaagcctttacagataaagaggaattacttaagcagcaggcatctaaccttcatgagcagaaaaaagctggggtgatatttgaagctgaagaagttatcactcttttaacttctgtgcttaaaacgtcatctgcatcaagaactagcttaagctcacgacatcagtttgctcctggagcgacagtattgtataagggcgataaaatggtgcttaacctggacaggtcccgtgttccaactgagtgtatagagaaaattgaggccattcttaaggaacttgaaaagccagcaccctgatgcgaccacgttttagtctacgtttatctgtctttacttaatgtcctttgttacaggccagaaagcataactggcctgaatattctctctgggcccactgttccacttgtatcgtcggtctgataatcagactgggaccacggtcccactcgtatcgtcggtctgattattagtctgggaccacggtcccactcgtatcgtcggtctgattattagtctgggaccacggtcccactcgtatcgtcggtctgataatcagactgggaccacggtcccactcgtatcgtcggtctgattattagtctgggaccatggtcccactcgtatcgtcggtctgattattagtctgggaccacggtcccactcgtatcgtcggtctgattattagtctggaaccacggtcccactcgtatcgtcggtctgattattagtctgggaccacggtcccactcgtatcgtcggtctgattattagtctgggaccacgatcccactcgtgttgtcggtctgattatcggtctgggaccacggtcccacttgtattgtcgatcagactatcagcgtgagactacgattccatcaatgcctgtcaagggcaagtattgacatgtcgtcgtaacctgtagaacggagtaacctcggtgtgcggttgtatgcctgctgtggattgctgctgtgtcctgcttatccacaacattttgcgcacggttatgtggacaaaatacctggttacccaggccgtgccggcacgttaaccgggctgcatccgatgcaagtgtgtcgctgtcgacgagctcgcgagctcgattcgat

SEQ ID NO: 27 - DNA, 19758 bp, Artificial Sequence
  OGAB vector 2.2
ttcagaacgctcggttgccgccgggcgttttttatgagacgtctcggcctgtttggccattatgacggtcattacaacggttatacgacgccacgcgtagtgagacatacacgttcgttggatccgggttcactttggttcatgtgcagctccatcagcaaaaggggatgataagtttatcaccaccgactatttgcaacagtgccgttgatcgtgctatgatcgactgatgtcatcagcggtggagtgcaatgtcgtgcaatacgaatggcgaaaagccgagctcatcggtcagcttctcaaccttggggttacccccggcggtgtgctgctggtccacagctccttccgtagcgtccggcccctcgaagatgggccacttggactgatcgaggccctgcgtgctgcgctgggtccgggagggacgctcgtcatgccctcgtggtcaggtctggacgacgagccgttcgatcctgccacgtcgcccgttacaccggaccttggagttgtctctgacacattctggcgcctgccaaatgtaaagcgcagcgcccatccatttgcctttgcggcagcggggccacaggcagagcagatcatctctgatccattgcccctgccacctcactcgcctgcaagcccggtcgcccgtgtccatgaactcgatgggcaggtacttctcctcggcgtgggacacgatgccaacacgacgctgcatcttgccgagttgatggcaaaggttccctatggggtgccgagacactgcaccattcttcaggatggcaagttggtacgcgtcgattatctggagaatgaccactgctgtgagcgctttgccttggcggacaggtggctcaaggagaagagccttcagaaggaaggtccagtcggtcatgcctttgctcggttgatccgctcccgcgacattgtggcgacagccctgggtcaactgggccgagatccgttgatcttcctgcatccgccagaggcgggatgcgaagaatgcgatgccgctcgccagtcgattggctgagctcatgagcggagaacgagatgacgttggaggggcaaggtcgcgctgattgctggggcaacacgtggagcggatcggggattgtctttcttcagctcgctgatgatatgccttcctggttggcttggtttcatcagccatccgcttgccctcatctgttacgccggcggtagccggccagcctcgcagagcaggattcccgttgagcaccgccaggtgcgaataagggacagtgaagaaggaacacccgctcgcgggtgggcctacttcacctatcctgcccggctgacgccgttggatacaccaaggaaagtctacacgaaccctttggcaaaatcctgtatatcgtgcgaaaaaggatggatataccgaaaaaatcgctataatgaccccgaagcagggttatgcagcggaaaagatccgtcgacctgcaggcatgcaagctctagcgattccagacgtcccgaaggcgtggcgcggcttccccgtgccggagcaatcgccctgggtgggttacacgacgcccctctatggcccgtactgacggacacaccgaagccccggcggcaaccctcagcggatgccccggggcttcacgttttcccaggtcagaagcggttttgtttcgggtgctgggttgttgtctctggacagtgatccatgggaaactactcagcaccaccaatgttcccaaaagaaagcgcaggtcagcgcccatgagccaagatctaggcatgtcgcccttcatcgctcccgacgtccctgagcaccttctagacactgttcgcgtcttcctgtacgcgcgtcagtctaagggccggtccgacggctcagacgtgtcgaccgaagcacagctagcggccggtcgtgcgttggtcgcctctcgcaacgcccaggggggtgcgcgctgggtcgtggcaggcgagttcgtggacgtcgggcgctccggctgggacccgaacgtgacccgtgccgacttcgagcgcatgatgggcgaagtccgcgccggcgaaggtgacgttgtcgttgtgaatgagctttcccggctcactcgcaagggcgcccatgacgcgctcgaaatcgacaacgaattgaagaagcacggcgtgcgcttcatgtcggttcttgagccgttccttgacacgtctacccctatcggcgtcgccattttcgcgctgatcgctgcccttgcgaaacaggacagtgacctgaaggcggagcgcctgaagggtgcgaaagacgagattgccgcgctgggtggcgttcactcgtcttccgccccgttcggaatgcgcgccgtgcgcaagaaggtcgataatctcgtgatctccgttcttgagccggacgaagacaacccggatcacgtcgagctagttgagcgcatggcgaaaatgtcgttcgaaggcgtgtccgacaacgccattgcaacgaccttcgagaaggaaaagatcccgtcgcccggaatggctgagcggcgcgccacggaaaagcgtcttgcgtccatcaaggcacgtcgcctgaacggcgctgaaaagccgatcatgtggcgcgctcaaacggtccgatggattctcaaccatcccgcaatcggcggtttcgcattcgagcgtgtgaagcacggtaaggcgcacatcaacgtcatacggcgcgaccccggcggcaagccgctaacgccccacacgggcattctcagcggctcgaagtggcttgagcttcaagagaagcgttccgggaagaatctcagcgaccggaagcctggggccgaagtcgaaccgacgcttctgagcgggtggcgtttcctggggtgccgaatctgcggcggctcaatgggtcagtcccagggtggccgtaagcgcaacggcgaccttgccgaaggcaattacatgtgcgccaacccgaaggggcacggcggcttgtcggtcaagcgcagcgaactggacgaattcgttgcttcgaaggtgtgggcacggctccgcacagccgacatggaagatgaacacgatcaggcatggattgccgccgctgcggagcgcttcgcccttcagcacgacctagcgggggtggccgatgagcggcgcgaacaacaggcgcacctagacaacgtgcggcgctccatcaaggaccttcaggcggaccgtaaggccggtctgtacgtcgggcgtgaagagctggaaacgtggcgctcaacggtgctgcaataccggtcctacgaagcggagtgcacgacccgactcgctgagcttgacgagaagatgaacggcagcacccgcgttccgtctgagtggttcagcggcgaagacccgacggccgaagggggcatctgggcaagctgggacgtgtacgagcgtcgggagttcctgagcttcttccttgactccgtcatggtcgaccgggggcgccaccctgaaaccaagaaatacatccccctgaaggaccgtgtgacgctcaagtgggcggagctgctgaaggaggaagacgaagcgagcgaagccactgagcgggagcttgcggcgctgtagcgagacacccgggaagcctgatctacgtctgtcgagaagtttcgatgacactcgttcgttcacacgttgcagcatggatccctcgaggagttactggccctgatttctccgcttctaataccgcacatgcggccgcaagctgtctcgacggcgcgcctagaaacaaggcagttccgggctgaaagtagcgccgggactaggccattccgcctgacctttaacggcctgtttggccattatgagacgtttattaaagtgcaggtgtttgccctgatgacttgacgctcgagaaggttcacgattagcatgccggttacggacctttgaggagggctcaatgctttccaagggcgaggaggacaacatggccatcatcaaggagttcatgcgcttcaaggtccacatggagggctccgtcaacgggcacgagttcgagatcgagggcgagggggagggccggccgtacgagggcacccagaccgccaagctgaaggtgaccaagggcggccccctcccgttcgcctgggacatcctctccccccagttcatgtacggctcgaaggcctacgtcaagcacccggccgacatcccggactacctgaagctctcgttcccggaggggttcaagtgggagcgggtcatgaacttcgaggacggcggcgtcgtcaccgtcacccaggacagctccctgcaggacggcgagttcatctacaaggtcaagctgcggggcacgaacttcccgagcgacggccccgtgatgcagaagaaaacgatgggctgggaagcgtcctcggagcgcatgtacccggaggacggcgccctcaagggcgagatcaagcagcgcctgaagctgaaggacggcggccactacgacgccgaagtcaagacgacgtacaaggccaagaagccggtgcagctcccggacgcctacaacgtgaacatcaagctcgacatcacctcgcacaacgaggactacacgatcgtggagcagtacgagcgcgccgagggccggcactcgaccggcggcatggacgagctgtacaagtgatgatttcacctgcacttaaaatttcgtctctaaaatccccggataactgccttaaaggctaggtggaggctcaaaaaggccttcttggccaccccgggccgtcgaccaattctcatgtttgacagcttatcatcgaatttctgccattcatccgcttattatcacttattcaggcgtagcaaccaggcgtttaagggcaccaataactgccttaaaaaaattacgccccgccctgccactcatcgcagtactgttgtaattcattaagcattctgccgacatggaagccatcacaaacggcatgatgaacctgaatcgccagcggcatcagcaccttgtcgccttgcgtataatatttgcccatggtgaaaacgggggcgaagaagttgtccatattggccacgtttaaatcaaaactggtgaaactcacccagggattggctgagacgaaaaacatattctcaataaaccctttagggaaataggccaggttttcaccgtaacacgccacatcttgcgaatatatgtgtagaaactgccggaaatcgtcgtggtattcactccagagcgatgaaaacgtttcagtttgctcatggaaaacggtgtaacaagggtgaacactatcccatatcaccagctcaccgtctttcattgccatacggaattccggatgagcattcatcaggcgggcaagaatgtgaataaaggccggataaaacttgtgcttatttttctttacggtctttaaaaaggccgtaatatccagctgaacggtctggttataggtacattgagcaactgactgaaatgcctcaaaatgttctttacgatgccattgggatatatcaacggtggtatatccagtgatttttttctccattttagcttccttagctcctgaaaatctcgataactcaaaaaatacgcccggtagtgatcttatttcattatggtgaaagttggaacctcttacgtgccgatcaacgtctcattttcgccaaaagttggcccagggcttcccggtatcaacagggacaccaggatttatttattctgcgaagtgatcttccgtcacaggtatttattcgcgataagctcatggagcggcgtaaccgtcgcacaggaaggacagagaaagcgcggatctgggaagtgacggacagaacggtcaggacctggattggggaggcggttgccgccgctgctgctgacggtgtgacgttctctgttccggtcacaccacatacgttccgccattcctatgcgatgcacatgctgtatgccggtataccgctgaaagttctgcaaagcctgatgggacataagtccatcagttcaacggaagtctacacgaaggtttttgcgctggatgtggctgcccggcaccgggtgcagtttgcgatgccggagtctgatgcggttgcgatgctgaaacaattatcctgagaataaatgccttggcctttatatggaaatgtggaactgagtggatatgctgtttttgtctgttaaacagagaagctggctgttatccactgagaagcgaacgaaacagtcgggaaaatctcccattatcgtagagatccgcattattaatctcaggagcctgtgtagcgtttataggaagtagtgttctgtcatgatgcctgcaagcggtaacgaaaacgatttgaatatgccttcaggaacaatagaaatcttcgtgcggtgttacgttgaagtggagcggattatgtcagcaatggacagaacaacctaatgaacacagaaccatgatgtggtctgtccttttacagccagtagtgctcgccgcagtcgagcgacagggcgaagccctcgagtgagcgaggaagcaccagggaacagcacttatatattctgcttacacacgatgcctgaaaaaacttcccttggggttatccacttatccacggggatatttttataattattttttttatagtttttagatcttcttttttagagcgccttgtaggcctttatccatgctggttctagagaaggtgttgtgacaaattgccctttcagtgtgacaaatcaccctcaaatgacagtcctgtctgtgacaaattgcccttaaccctgtgacaaattgccctcagaagaagctgttttttcacaaagttatccctgcttattgactcttttttatttagtgtgacaatctaaaaacttgtcacacttcacatggatctgtcatggcggaaacagcggttatcaatcacaagaaacgtaaaaatagcccgcgaatcgtccagtcaaacgacctcactgaggcggcatatagtctctcccgggatcaaaaacgtatgctgtatctgttcgttgaccagatcagaaaatctgatggcaccctacaggaacatgacggtatctgcgagatccatgttgctaaatatgctgaaatattcggattgacctctgcggaagccagtaaggatatacggcaggcattgaagagtttcgcggggaaggaagtggttttttatcgccctgaagaggatgccggcgatgaaaaaggctatgaatcttttccttggtttatcaaacgtgcgcacagtccatccagagggctttacagtgtacatatcaacccatatctcattcccttctttatcgggttacagaaccggtttacgcagtttcggcttagtgaaacaaaagaaatcaccaatccgtatgccatgcgtttatacgaatccctgtgtcagtatcgtaagccggatggctcaggcatcgtctctctgaaaatcgactggatcatagagcgttaccagctgcctcaaagttaccagcgtatgcctgacttccgccgccgcttcctgcaggtctgtgttaatgagatcaacagcagaactccaatgcgcctctcatacattgagaaaaagaaaggccgccagacgactcatatcgtattttccttccgcgatatcacttccatgacgacaggatagtctgagggttatctgtcacagatttgagggtggttcgtcacatttgttctgacctactgagggtaatttgtcacagttttgctgtttccttcagcctgcatggattttctcatactttttgaactgtaatttttaaggaagccaaatttgagggcagtttgtcacagttgatttccttctctttcccttcgtcatgtgacctgatacgcgtgctaccttaagagagtcaattcgcccttcccggtcgatatgaacagcttatttacataattcacgttattggtagttataaatgaaattcctaatatcggttatgaagtgaaattgaatttctacttgatctttctctctatttttgtaaaataaaattaagaatatttaaatattcaatgattcatttttgcagaaatcggaggaagaagaatatatgaaaacatttaacatttctcaacaagatccccccatattgttgtataagtgatgaaatactgaatttaaaacttagtttatatgtggtaaaatgttttaatcaagtttaggaggaattaattatgaagtgtaatgaataatgaatgtaacagggttcaattaaaagagggaagcgtatcattaaccctataaactacgtctgccctcattattggagggtgaaatgtgaatacatcctattcacaatcgaatttacgacacaaccaaattttaatttggctttgcattttatctttttttagcgtattaaatgaaatggttttgaacgtctcattacctgatattgcaaatgattttaataaaccaccagcgagtacaaactgggtgaacacagcctttatgttaaccttttccattggaacagctgtatatggaaagctatctgatcaattaggcatcaaaaggttactcctatttggaattataataaattgtttcgggtcggtaattgggtttgttggccattctttcttttccttacttattatggctcgttttattcaaggggctggtgcagctgcatttccagcactcgtaatggttgtagttgcgcgctatattccaaaggaaaataggggtaaagcatttggtcttattggatcgatagtagccatgggagaaggagtcggtccagcgattggtggaatgatagcccattatattcattggtcctatcttctactcattcctatgataacaattatcactgttccgtttcttatgaaattattaaagaaagaagtaaggataaaaggtcattttgatatcaaaggaattatactaatgtctgtaggcattgtattttttatgttgtttacaacatcatatagcatttcttttcttatcgttagcgtgctgtcattcctgatatttgtaaaacatatcaggaaagtaacagatccttttgttgatcccggattagggaaaaatataccttttatgattggagttctttgtgggggaattatatttggaacagtagcagggtttgtctctatggttccttatatgatgaaagatgttcaccagctaagtactgccgaaatcggaagtgtaattattttccctggaacaatgagtgtcattattttcggctacattggtgggatacttgttgatagaagaggtcctttatacgtgttaaacatcggagttacatttctttctgttagctttttaactgcttcctttcttttagaaacaacatcatggttcatgacaattataatcgtatttgttttaggtgggctttcgttcaccaaaacagttatatcaacaattgtttcaagtagcttgaaacagcaggaagctggtgctggaatgagtttgcttaactttaccagctttttatcagagggaacaggtattgcaattgtaggtggtttattatccatacccttacttgatcaaaggttgttacctatggaagttgatcagtcaacttatctgtatagtaatttgttattacttttttcaggaatcattgtcattagttggctggttaccttgaatgtatataaacattctcaaagggatttctaaatcgttaagggatcaactttgggagagagttcaaaattgatcctttttttataacaggaattgggcatcaaataaaacgaaaggctcagtcgaaagactgggcctttcgttttatctgttgtttgtcggtgaacgctctcctgagtaggacaaatccgccgggagcggatttgaacgttgcgaagcaacggcccggagggtggcgggcaggacgcccgccataaactgccaggcatcaaattaagcagaaggccatcctgacggatggcctttttgcgtttctacaaactcttcctgtcgtcatatctacaattctacacagcccagtccagactattcggcactgaaattatgggtgaagtggtcaagacctcactaggcaccttaaaaatagcgcaccctgaagaagatttatttgaggtagcccttgcctacctagcttccaagaaagatatcctaacagcacaagagcggaaagatgttttgttctacatccagaacaacctctgctaaaattcctgaaaaattttgcaaaaagttgttgactttatctacaaggtgtggcataatgtgtggaattgtgagcggataacaattaagctaattctatggtaaaagcattcctgaacccaatatccttatttttagtggacaaggccttgttctcatatggttgcttgagccagtgccttacaaggctcttccgctttggcaggctgttcaaaattatttattagagcaactcaaggaactaggcggagatccaaaagcaaccgatgcagcacgtgtttttcggattgctgggagcgtcaatagtaagaatggagcggaagtaagagcggaatatcggcacgattacagatatgagttaaggcagattcaatttgattaccttccagaactcaatgaggttattaatcccgctccacaaaagaaaaaacgggggcgtaaaaagaaagtagttcagttattcaatacctacaaactccattacgctcgcctattggatatagtgaaattggtggaactacgaaattatgaggtaactggatacagggaaatcatttgctttttataccgttattggttgtgctgttacacgaacgaccctgtagaggctttaaatcaaacacagacacttaatttacagttcactgagcctttacccttaaaagaggttgaaagggctacacggagcgcagaaaaggcgtgggaagcacgaaataacgaagaggctaaccggattgcaatcgaaaaaggatatcccagtgctggatacaatattagcaataaaaagttgattgaatggctagatatcacaccagaagaacagaagcatttacagacgattatagacgctaatgagaaacggagaagaaagcgggaaagggataggatttatcaagaacaaaaacgtcgtgagcggggagatatgacccgacaggagtatattaagcaacaacaggataaaacagatgataaattatttaaattgcaggagttattagaacagaatcccaaaatctcaaaaattaaattagcaaaaatacttggtgtagataaatcgcacttatacagactgctgaaacaactataactggaaaaaattagtgtctcatggttcgtcgcccttatattatgggcgttagcctgcttgctaattggataggtgttattgtcatttcaacgtcggacgttttggtagatgaacgtcggacgttatttgcttcaatagattgttgatgtattaagggttgcagtgaatcgacaagcaaaaagttatgacgttgtgaaaaaattgaatagaaaattggaaattacgtcggacgttctaacttaaaaaccctgttatatcaatgatttaaaaggaaattaacgtcataaaagacctttctgcaacaaaagtttttctggaagagttgaggttattttataggtattatggacttttgtagactttttgtgtactttttgtggactccacactcgctggtatcgtgttattttttaattgagatatgaatatggaaattaaacgttttaggcgttggtttggtgatgacaaaaaaataagagtacccgctcacaacggatactctttcgagaaatgtacgaaacgctataaataaaaaataactagatacatttacattgtatcacgtttcgtacatttctccaataacaaattgattggaggaatgcaaagtgaataatgaaccagtaaaacgtggtaagaagaacagatgggaattaaacctacctataatgacttatgtagtagctgatgattggattgataaactaggacacgaaacgtttactttatggttgaggttccatacttgggtagatagagaagatgaactccgagattatgatcgcatacctagaagttttgagaacatatataaaaagacactaggaatctcaaaaagtaagttttatagattgataaaacctttatgggaatatggattaatagacatcatagaatacgaagaatctaaccgtaattctactaaacctaaaaatataattgtttatgagtatcctttacacgaaatagaaagaaagtataaaccactagaaaaattaagagattgggataaagactataattccgtttctaaagaattaggtaaaacaggtggtagaccaaggaaaaaagatagtgaagaagaacccgaaaagaaacccgaagaagtaactaaaaagaaacgtaaatataagttaaaaagagttatccacaacggtttcaaaaatgaaacggtggagggtttcaaaaatgaaacggtggagggtttcaaaaatgaaacggtgaccgtttcaaaaataaaacccaataattattcaaatatctttaataacttatcaaatatttctactaatgtttcaaataatttattaattgatgatgatgaggaaatcgaaaatgaaccaactggtcgtacaataaataggtcattacttttttcacaagaagatattaaacaggcctatcaatttattaatagattttcagttatacagttacgtgaaaactttagctttgataaacactttgaagaacggttggtatgttatttatggaaagcagggatttctactttttacacgcacgaaatcagtaaaatgataaaaaaaatagcagactatgaaaaatctaaaaaaggtagattaaacccaatacgtgaccgagccttatatatggtaaatggtcttgtaatgaatagagcttcttcccaaagtgaacatgctacttataaactaaaccaatataaaaaacagaaggaacaggaaaaacaacaacaggagcaacaaagatcaagagtaccgttctataattggttggaggaaagagaagaacaaaccgaaggtcaactacccaccacttaaagcctaacggcttttgaagtggggcttgtaaaaagccctagttgactaccccaagtctttcgaggactacgttggaaaggtcatgacacctacaaatgctcctctagttcgtagccactgtcgttgatggttaaaagtcctgatgggtagggacggtgctgtcaacatcacaagcccttccaacatgggggaagaggaagaacactccgagaaaggagggggctgtcgtacacgccttgttcgtgtacgtgatttttaacacttttatctctaatataatctctccttgagttagcagagactaagaataaaacacattaggattttttatctacataaggaggttcaatacatgcctactatttcgtttaagggaaagtcttttgtacaaaatcatcacttgactgtaaaatatcatgaattgatcccagaaccagaaaaaagtctgaccgataaagttagtcttcatgacaatcttatcattcatggggacaatttaaaggcgttgaaagctctactacctacatatgctggtaagatagattgcatctatattgacccaccatacaatactggaactgaaaaatggatttataatgataatgtcaactccccaatgattagggaatggcttggaaaagtggtagacaaagaagacttatcccgacatgataagtggctttgtatgatgatgccgaggttaaaactgttgaaagagttgttgtcagaagacggagtgatatttgtaagcattgactacaatgaaatacaccatcttacgtgccttatgaacgaaatattcggtgaggagaattttcgtgacgctattatcattcgtagaggagtaaaaaatgttcaagcgcaatttgacacaattgattctctttcaaatggttatgagtctattttggtttacactaaacagccatctcgacgatttaataaggtttatgaagatgtagaagaaaagcctggtagttggaataatcattggagaggtacagaccgtaaaactatgagatatgaattatttggggttactccgacagaaggtcaatggagatgggggaaagaacgtagtctccaggctattgaaaactatcaaatgatgttagatgaacttagacaaaaaggcattactaatccaactcaagaggatattgataaatggtatcttgaatatgtagaaaataatggggaagatattgacttgttacgacaaaatgataatggcacgattgagcactttgttccaccgactagcaaaaagttgttaagtaatgcctggtttgacttaaaacccaacggttctagtcaattaaagaagatatttggaaggaaggttttcgataaccctaaatcaattgatttggtaaaaagactaatacaatttgcgactgaaaacaaagaagcgattgtacttgactcatttgcagggagtggcactactgctcatgcagtattatcgcttaacaaacaagatggagggaatcgtcgtttcatccttattgagatggaagaatatgcacatgagattaccgcagaacgcggatctttatcgatttgcatgcaagctaattcggtggaaacgaggtcatcatttccttccgaaaaaacggttgcatttaaatcttacatatgtaatactttcaaagactacatttgtaagatttgatgtttgagtcggctgaaagatcgtacgtaccaattattgtttcgtgattgttcaagccataacactgtagggatagtggaaagagtgcttcatctggttacgatcaatcaaatattcaaacggagggagacgattttgatgaaaccagtaacgttatacgatgtcgcagagtatgccggtgtctcttatcagaccgtttcccgcgtggtgaaccaggccagccacgtttctgcgaaaacgcgggaaaaagtggaagcggcgatggcggagctgaattacattcccaaccgcgtggcacaacaactggcgggcaaacagtcgttgctgattggcgttgccacctccagtctggccctgcacgcgccgtcgcaaattgtcgcggcgattaaatctcgcgccgatcaactgggtgccagcgtggtggtgtcgatggtagaacgaagcggcgtcgaagcctgtaaaacggcggtgcacaatcttctcgcgcaacgcgtcagtgggctgatcattaactatccgctggatgaccaggatgccattgctgtggaagctgcctgcactaatgttccggcgttatttcttgatgtctctgaccagacacccatcaacagtattattttctcccatgaagacggtacgcgactgggcgtggagcatctggtcgcattgggtcaccagcaaatcgcgctgttagcgggcccattaagttctgtctcggcgcgtctgcgtctggctggctggcataaatatctcactcgcaatcaaattcagccgatagcggaacgggaaggcgactggagtgccatgtccggttttcaacaaaccatgcaaatgctgaatgagggcatcgttcccactgcgatgctggttgccaacgatcagatggcgctgggcgcaatgcgcgccattaccgagtccgggctgcgcgttggtgcggatatctcggtagtgggatacgacgataccgaagacagctcatgttatatcccgccgttaaccaccatcaaacaggattttcgcctgctggggcaaaccagcgtggaccgcttgctgcaactctctcagggccaggcggtgaagggcaatcagctgttgcccgtctcactggtgaaaagaaaaaccaccctggcgcccaatacgcaaaccgcctctccccgcgcgttggccgattcattaatgcagctggcacgacaggtttcccgactggaaagcgggcagtgagcgcaacgcaattaatgtgagttaggatcgctaccttaagagagacgcgttatcgggggttagttcgtcatcattgatgagggttgattatcacagtttattactctgaattggctatccgcgtgtgtacctctacctggagtttttcccacggtggatatttcttcttgcgctgagcgtaagagctatctgacagaacagttcttctttgcttcctcgccagttcgctcgctatgctcggttacacggctgcggcgagcgctagtgataataagtgactgaggtatgtgctcttcttatctccttttgtagtgttgctcttattttaaacaactttgcggttttttgatgactttgcgattttgttgttgctttgcagtaaattgcaagatttaataaaaaaacgcaaagcaatgattaaaggatgttcagaatgaaactcatggaaacacttaaccagtgcataaacgctggtcatgaaatgacgaaggctatcgccattgcacagtttaatgatgacagcccggaagcgaggaaaataacccggcgctggagaataggtgaagcagcggatttagttggggtttcttctcaggctatcagagatgccgagaaagcagggcgactaccgcacccggatatggaaattcgaggacgggttgagcaacgtgttggttatacaattgaacaaattaatcatatgcgtgatgtgtttggtacgcgattgcgacgtgctgaagacgtatttccaccggtgatcggggttgctgcccataaaggtggcgtttacaaaacctcagtttctgttcatcttgctcaggatctggctctgaaggggctacgtgttttgctcgtggaaggtaacgacccccagggaacagcctcaatgtatcacggatgggtaccagatcttcatattcatgcagaagacactctcctgcctttctatcttggggaaaaggacgatgtcacttatgcaataaagcccacttgctggccggggcttgacattattccttcctgtctggctctgcaccgtattgaaactgagttaatgggcaaatttgatgaaggtaaactgcccaccgatccacacctgatgctccgactggccattgaaactgttgctcatgactatgatgtcatagttattgacagcgcgcctaacctgggtatcggcacgattaatgtcgtatgtgctgctgatgtgctgattgttcccacgcctgctgagttgtttgactacacctccgcactgcagtttttcgatatgcttcgtgatctgctcaagaacgttgatcttaaagggttcgagcctgatgtacgtattttgcttaccaaatacagcaatagtaatggctctcagtccccgtggatggaggagcaaattcgggatgcctggggaagcatggttctaaaaaatgttgtacgtgaaacggatgaagttggtaaaggtcagatccggatgagaactgtttttgaacaggccattgatcaacgctcttcaactggtgcctggagaaatgctctttctatttgggaacctgtctgcaatgaaattttcgatcgtctgattaaaccacgctgggagattagataatgaagcgtgcgcctgttattccaaaacatacgctcaatactcaaccggttgaagatacttcgttatcgacaccagctgccccgatggtggattcgttaattgcgcgcgtaggagtaatggctcgcggtaatgccattactttgcctgtatgtggtcgggatgtgaagtttactcttgaagtgctccggggtgatagtgttgagaagacctctcgggtatggtcaggtaatgaacgtgaccaggagctgcttactgaggacgcactggatgatctcatcccttcttttctactgactggtcaacagacaccggcgttcggtcgaagagtatctggtgtcatagaaattgccgatgggagtcgccgtcgtaaagctgctgcacttaccgaaagtgattatcgtgttctggttggcgagctggatgatgagcagatggctgcattatccagattgggtaacgattatcgcccaacaagtgcttatgaacgtggtcagcgttatgcaagccgattgcagaatgaatttgctggaaatatttctgcgctggctgatgcggaaaatatttcacgtaagattattacccgctgtatcaacaccgccaaattgcctaaatcagttgttgctcttttttctcaccccggtgaactatctgcccggtcaggtgatgcacttcaaaaagcctttacagataaagaggaattacttaagcagcaggcatctaaccttcatgagcagaaaaaagctggggtgatatttgaagctgaagaagttatcactcttttaacttctgtgcttaaaacgtcatctgcatcaagaactagtttaagctcacgacatcagtttgctcctggagcgacagtattgtataagggcgataaaatggtgcttaacctggacaggtctcgtgttccaactgagtgtatagagaaaattgaggccattcttaaggaacttgaaaagccagcaccctgatgcgaccacgttttagtctacgtttatctgtctttacttaatgtcctttgttacaggccagaaagcataactggcctgaatattctctctgggcccactgttccacttgtatcgtcggtctgataatcagactgggaccacggtcccactcgtatcgtcggtctgattattagtctgggaccacggtcccactcgtatcgtcggtctgattattagtctgggaccacggtcccactcgtatcgtcggtctgataatcagactgggaccacggtcccactcgtatcgtcggtctgattattagtctgggaccatggtcccactcgtatcgtcggtctgattattagtctgggaccacggtcccactcgtatcgtcggtctgattattagtctggaaccacggtcccactcgtatcgtcggtctgattattagtctgggaccacggtcccactcgtatcgtcggtctgattattagtctgggaccacgatcccactcgtgttgtcggtctgattatcggtctgggaccacggtcccacttgtattgtcgatcagactatcagcgtgagactacgattccatcaatgcctgtcaagggcaagtattgacatgtcgtcgtaacctgtagaacggagtaacctcggtgtgcggttgtatgcctgctgtggattgctgctgtgtcctgcttatccacaacattttgcgcacggttatgtggacaaaatacctggttacccaggccgtgccggcacgttaaccgggctgcatccgatgcaagtgtgtcgctgtcgacgagctcgcgagctcggacatgaggttgccccgtattcagtgtcgctgatttgtattgtctgaagttgtttttacgttaagttgatgcagatcaattaatacgatacctgcgtcataattgattatttgacgtggtttgatggcctccacgcacgttgtgatatgtagatgataatcattatcactttacgggtcctttccggtgatccgacaggttacggggcggcgacctcgcgggttttcgctatttatgaaaattttccggtttaaggcgtttccgttcttcttcgtcataacttaatgtttttatttaaaataccctctgaaaagaaaggaaacgacaggtgctgaaagcgagctttttggcctctgtcgtttcctttctctgtttttgtccgtggaatgaacaatggaagtccgagctcatcgctaataacttcgtatagcatacattatacgaagttatattcgatgcggccgcaagcttgaagagctcttct

SEQ ID NO: 28 - DNA, 5624 bp, Artificial Sequence
  DNA fragment
attccgagaccatgtcgatactgaacgaatcgacgccacgcgtagtgagacatacacgttcgttgggttcacgactcaacacgctagggacgtgaagtcgattccttcgatgcattgtaatagccaccaaaagagtgatgatagtcatgggtgtctgtagcacgtgcatcgctcattacaacggttatacgcacactcccttccttgtgttcacattcgaacggtgtctgctttgacaacatgctgtgcggtgttgtaaagtcgtggccaggagaatacgacagcgtgcaggactgggggagttatgcagtccgcagaaaaggcaaagcctgctgatggcgccgcagcggcattgctggcaaccctcacccataaacggcgtctggacgcggccaccccgaaggaaagcgcactgtggttgctggaccgcctgctccctgaagcgggtgtaaacaatgttccactggccgtccgcgtcgatggtcgtctggacgccgcggctttgcaagcagcggtcgacggtctcgtgcgccgtcacgaggtgttgcgcaccgtatacctggatcggcaggccggtctggtgcgtgaagtgctgggagaggacaccccaggaccgcgcgtggaggtccatgacacggtggccggcgtcccggagaaagccttgcgtgaattcgccgctacaccgatccggtgtgacggccggctgatgctgcgcgcagcggtgttccgcggtccggatgctgacaccctcgcggtcgttgtgcatcacctggtgttcgacgccgcttcggtacctgtactgatcgccgaacttgccgctgcctacgacgcaagagccaccggtcgtgacttgcctgatgaactgcgcaccccggtcgcggcattgcgggatcccgcaccccgtgaggaatccctggcatattggcgcaccgccctggatggtttcgacccagcgggactggacctcgattgcgcacggcccgccccagcgcgtgcgaccctcgtgggtgacaccgttcttcacgtccttgacgatgaaacccgtgacctggtccggggcctgcagcgaacgcaaagagcaccagaagctgttatcctgttcacggcattctgtctgctcttggcagctcacggtgcgggtccagatttggtcgtgggctccccggtgaacatatgagacgaggctaggtggaggctcagtgatgataagtctgcgatggtggatgcatgtgtcatggtcatagctgtttcctgtgtgaaattgttatccgctcagagggcacaatcctattccgcgctatccgacaatctccaagacattaggtggagttcagttcggcgtatggcatatgtcgctggaaagaacatgtgagcaaaaggccagcaaaaggccaggaaccgtaaaaaggccgcgttgctggcgtttttccataggctccgcccccctgacgagcatcacaaaaatcgacgctcaagtcagaggtggcgaaacccgacaggactataaagataccaggcgtttccccctggaagctccctcgtgcgctctcctgttccgaccctgccgcttaccggatacctgtccgcctttctcccttcgggaagcgtggcgctttctcatagctcacgctgtaggtatctcagttcggtgtaggtcgttcgctccaagctgggctgtgtgcacgaaccccccgttcagcccgaccgctgcgccttatccggtaactatcgtcttgagtccaacccggtaagacacgacttatcgccactggcagcagccactggtaacaggattagcagagcgaggtatgtaggcggtgctacagagttcttgaagtggtggcctaactacggctacactagaagaacagtatttggtatctgcgctctgctgaagccagttaccttcggaaaaagagttggtagctcttgatccggcaaacaaaccaccgctggtagcggtggtttttttgtttgcaagcagcagattacgcgcagaaaaaaaggatctcaagaagatcctttgatcttttctacggggtctgacgctctattcaacaaagccgccgtcccgtcaagtcagcgtaaatgggtagggggcttcaaatcgtcctcgtgataccaattcggagcctgcttttttgtacaaacttgttgataatggcaattcaaggatcttcacctagatccttttaaattaaaaatgaagttttaaatcaatctaaagtatatatgagtaaacttggtctgacagttaccaatgcttaatcagtgaggcacctatctcagcgatctgtctatttcgttcatccatagttgcctgactccccgtcgtgtagataactacgatacgggagggcttaccatctggccccagtgctgcaatgataccgcgagagccacgctcaccggctccagatttatcagcaataaaccagccagccggaagggccgagcgcagaagtggtcctgcaactttatccgcctccatccagtctattaattgttgccgggaagctagagtaagtagttcgccagttaatagtttgcgcaacgttgttgccattgctacaggcatcgtggtgtcacgctcgtcgtttggtatggcttcattcagctccggttcccaacgatcaaggcgagttacatgatcccccatgttgtgcaaaaaagcggttagctccttcggtcctccgatcgttgtcagaagtaagttggccgcagtgttatcactcatggttatggcagcactgcataattctcttactgtcatgccatccgtaagatgcttttctgtgactggtgagtactcaaccaagtcattctgagaatagtgtatgcggcgaccgagttgctcttgcccggcgtcaatacgggataataccgcgccacatagcagaactttaaaagtgctcatcattggaaaacgttcttcggggcgaaaactctcaaggatcttaccgctgttgagatccagttcgatgtaacccactcgtgcacccaactgatcttcagcatcttttactttcaccagcgtttctgggtgagcaaaaacaggaaggcaaaatgccgcaaaaaagggaataagggcgacacggaaatgttgaatactcatactcttcctttttcaatattattgaagcatttatcagggttattgtctcatgagcggatacatatttgaatgtatttagaaaaataaacaaataggggttccgcgcacatttccccgaaaagtgccagatacctgaaacaaaacccatcgtacggccaaggaagtctccaataactgtgatccaccacaagcgccagggttttcccagtcacgacgttgtaaaacgacggccagtcatgcataatccgcacgcatctggaataaggaagtgccattccgcctgacctcgtctcagagattggccctgatgctatacttaccggcctggtagaacaaaaccagaccctcgacacgcaggccgtacccgtactgcgccgtgaccgggacgaggtgcgcgctgcagtcgaggctgtcggtcgcctgcacctggcgggcatccccgtggattggccggcggtccttcctggtgcccgccgtgtcgaactgccgacctacgcgttccaacacgagcgctactggctggacccagaggaactggcggctgcagccgaggacaccgttgcaccttcaggtacggaagtccccgaccccgatacccgcttctggggcgccgtcgcagacgaggatttgggcagcttggcagcgctgcttggtatagacggagaaaagggaggtgctcaggaccgcgcggctgtggaagcggctctgcctgtgctggcttcgtggttgggccgccggcaggctgcggcacgcgtgtcccactatcgggtgggttggacgccagtcgctagacggcctgacggcacgacagcgcggttgcggggtatctggctgttgaccattcccgcacgcataggcgccgacgatgcgttggtgactcgtctggcaagtgcattgggcggtgccggagccgacgttcgtgtggttacggttggtgatccgggagcagattcgtatgacgatctggctgccgaagtttcgtcgttgaccgccgacggcggtgaactcgccggcgtcctgagtctgctgggattggcgtctgctgatggtcccggggatgcgcgtgaggccgcagtaggtacactcgccctgctgcgtgcgctctcgggttcggttgcatcagtccctgtttggtcactgacatctggtgccgtatcgaccggcggatcagagcgtgtaagcgcccctgcccaggctgtgctctggggactgggtcgcctgctggccgaagacagtgatgtgcgttgggcgggcgttgtggatgtgccggcgccgtgtggtgatcgtgtgttgcgccgcctcgccgaagtgctcgcaaatccagccgaggagactgaagtggccgtacgtgacgctggcgtgtttgcgcgtcgtcttctgcgtgcaaccggggcagcggacgggcccgcccgtcctactgctcttgctccccgcggcaccctgttggtatcaggcggttcagatacatggcgtgatcgtgttgctcgccgtctgcttgcatcgggcgcggcacatgtgttggtcgcgacagcgccagatgagccagaacctgcttctaccccggggtcggcggttaccggggtttcccgtgtcgtgtgtgacgtttctgacggtccggctctggcgcatttggccgccagcctgccggcgggccccgacggccgtccgctgacgggtgtagtgcacgcgcccccggcaacagccagcgatggacccttggataaggcactggatgaggtattgggtgctggactgccggcgctggcaggcgtatcatcgaccgctggcccgatcgccctcttcctggccgtggatgttgatgacctggttggcgccccgggagcaggcgccgtcgcggctctggccggttggtgggaagccgccgcacgcgtacgtacggccgaccgcgcacctgtacgcctgattgcggcagatcccgatgcactggatctggccgtgttggatcgtgcaatggaacgtgccgatggtctgctcgtcgtgacgggtcgtgattgggcacaatacgcgggaacccacgcggatacccgcggtcgccgcttgctggaaggagtgcctgaggcacgtgcagttcttgcagcagcagcccctgcgggtgacgcgggcaagagcgggctgttggctggtgtagacgggccggaatcgttgcgtcgcgtgttggcggcgcgcgaagcagaccacaagctcgcgaccctggtggagctggtgcgcggtcaagtcgcggtcgtcctcggacacgcgagtgccgatgcggtcagtgcggatggagactttatggatctgggatttgcttcgctgacagccgttgagtttggccaccgtttaagcgccatcacaggcctcaaattgcctacgactctggtctacgaccacctgaacccagtggaactggccgagcacctggctgacgagctggcgagggaactgaccgccgcgtgatagcataaccccttggggcctctaaacgggtcttgaggggttttttgcaaac

SEQ ID NO: 29 - DNA, 5588 bp, Artificial Sequence
  DNA fragment
tagatgagaccgcgcagatgtacgacaatatcgcttagtcacccacgccacgcgtagtgagacatacacgttcgttgggttcacgactcaacacgctagggacgtgaagtcgattccttcgatgcattgtaatagccaccaaaagagtgatgatagtcatgggtgtctgtagcacgtgcatcgctcattacaacggttatttgggcctgttcacattcgaacggtgtctgctttgacaacatgctgtgcggtgttgtaaagtcgtggccaggagaatacgacagcgtgcaggactgggggagttatggcgaccccaaacgagaaagttgtggaggctctgcgcgcctccctcaaggaaaccgaactccttcgtcaacagaacaatgcgctccgcgcggccagctcggaaccagtagcaatcgttggcatgggctgccgcttccctggaggtgtggtatcccctgaaggtctctgggaagtcgtgttgtccggtgccgacgtcatctcggagttcccaaccgaccggggttgggatgtcgaaggtctgtatgatcctgacccggaccggcccggtaagacgtacggtcgccgtggtggattcgtcgacgcggtagcggacttcgatgccgggtttttcggcatctcacctcgggaagccctggcgatggatccacagcaacgtctgctcttggaaactagctgggaggcgttcgagcgcgccggtatcgaccccgcaaccctgcgcggatcgcggacgggtgtgttcgccggtgtcatgtatcatgattacgcgagcaggctgcgtgaggtacctggacaccttgaaggccttatgggcacgggcaacgccaccagcgtcatcgcgggtcgcttgtcttataccttcggactggagggcccgagtgtttcggtggacaccgcctgttcctcgagtctcgttgccctgcacctggctgtgcaagccctccgggcaggggaatgcgagatggccctcgcgggcggagtaaccgtgatggcgaccccagaggcgttcatcaacttcagtcgccagagaggtctggctgcagacggccggtgcaaggcgttcggtgcaggagcagacggcacgggttgggccgaaggagctggaatgagacgaggctaggtggaggctcagtgatgataagtctgcgatggtggatgcatgtgtcatggtcatagctgtttcctgtgtgaaattgttatccgctcagagggcacaatcctattccgcgctatccgacaatctccaagacattaggtggagttcagttcggcgtatggcatatgtcgctggaaagaacatgtgagcaaaaggccagcaaaaggccaggaaccgtaaaaaggccgcgttgctggcgtttttccataggctccgcccccctgacgagcatcacaaaaatcgacgctcaagtcagaggtggcgaaacccgacaggactataaagataccaggcgtttccccctggaagctccctcgtgcgctctcctgttccgaccctgccgcttaccggatacctgtccgcctttctcccttcgggaagcgtggcgctttctcatagctcacgctgtaggtatctcagttcggtgtaggtcgttcgctccaagctgggctgtgtgcacgaaccccccgttcagcccgaccgctgcgccttatccggtaactatcgtcttgagtccaacccggtaagacacgacttatcgccactggcagcagccactggtaacaggattagcagagcgaggtatgtaggcggtgctacagagttcttgaagtggtggcctaactacggctacactagaagaacagtatttggtatctgcgctctgctgaagccagttaccttcggaaaaagagttggtagctcttgatccggcaaacaaaccaccgctggtagcggtggtttttttgtttgcaagcagcagattacgcgcagaaaaaaaggatctcaagaagatcctttgatcttttctacggggtctgacgctctattcaacaaagccgccgtcccgtcaagtcagcgtaaatgggtagggggcttcaaatcgtcctcgtgataccaattcggagcctgcttttttgtacaaacttgttgataatggcaattcaaggatcttcacctagatccttttaaattaaaaatgaagttttaaatcaatctaaagtatatatgagtaaacttggtctgacagttaccaatgcttaatcagtgaggcacctatctcagcgatctgtctatttcgttcatccatagttgcctgactccccgtcgtgtagataactacgatacgggagggcttaccatctggccccagtgctgcaatgataccgcgagagccacgctcaccggctccagatttatcagcaataaaccagccagccggaagggccgagcgcagaagtggtcctgcaactttatccgcctccatccagtctattaattgttgccgggaagctagagtaagtagttcgccagttaatagtttgcgcaacgttgttgccattgctacaggcatcgtggtgtcacgctcgtcgtttggtatggcttcattcagctccggttcccaacgatcaaggcgagttacatgatcccccatgttgtgcaaaaaagcggttagctccttcggtcctccgatcgttgtcagaagtaagttggccgcagtgttatcactcatggttatggcagcactgcataattctcttactgtcatgccatccgtaagatgcttttctgtgactggtgagtactcaaccaagtcattctgagaatagtgtatgcggcgaccgagttgctcttgcccggcgtcaatacgggataataccgcgccacatagcagaactttaaaagtgctcatcattggaaaacgttcttcggggcgaaaactctcaaggatcttaccgctgttgagatccagttcgatgtaacccactcgtgcacccaactgatcttcagcatcttttactttcaccagcgtttctgggtgagcaaaaacaggaaggcaaaatgccgcaaaaaagggaataagggcgacacggaaatgttgaatactcatactcttcctttttcaatattattgaagcatttatcagggttattgtctcatgagcggatacatatttgaatgtatttagaaaaataaacaaataggggttccgcgcacatttccccgaaaagtgccagatacctgaaacaaaacccatcgtacggccaaggaagtctccaataactgtgatccaccacaagcgccagggttttcccagtcacgacgttgtaaaacgacggccagtcatgcataatccgcacgcatctggaataaggaagtgccattccgcctgacctcgtctcactttgccagaggaagcggctaacgcggctgacgcattcggtctgcaccccgcgcttctggatgcagccctgcacgccatcggcttgctgcaattggctgactcggagggaatgcgtctgccattcgcttggagtggagtttcgctccaagctgtcggcgctaccacgcttcgcgtgagaatcgcccccgacggtcgcggtggagctaccgttgacctgttcgacgaagcgggcctgcccgtcgccagggtcgagagtctgacccttcgcgaagtctcgcgcgagcagatggcggccgcggcctccgcggccggcgacgagtccttgttccaggtcgaatgggtaccggtggttggcgatcccgatgaagctgtgtcctgggccgtgctcggcgactcgccgctggcagagggcggattggtcttcgctgatgtagaagccttgctggccagctcccaggacctgccaggtacagtcgtgttggaatgccctgcagttgaaggtgctccagtgcctgatgcagttcgcgaccggctcaccggcgtgttgggcgtcctgcagcgctgggtggctgatgaacgactggcctcgtcccggttggtcgtggtcacgcgtggtgccgtcgccgcgagcgccaacgaaccagcggacgtccgcgtcgcgcctgtatggggcctcgtccgggcggctcaggccgaacatccggaccggttcgtactggcagatttgcctgcaggcgccggtgcccgcgagttggccgctggtctggcttgtgacgaaccgcagtgggcgatccgcgatggtgcgatccatgtaccacgtctggttcgcgctcaagactctaccgacggagcctccggtttcggcgatggccccgtcttgatcaccggagccagcggcgcgttgggtggagtggtagcgcgccacctcgtaagcgtgcacggtgtgcgtgaactcgtcttgctttcacgtaggggcctggcggcagagggaatggatacgctgcgggatgagctgacccaccaaggcgcatcggtcgaagtgctggcatgtgatgcggctgaccgcaacgctctggcacaggcgctgtcaggccgccggctgacggcagtgatccacgccgctggagtcttggacgatggtgtcctggaagccctggacgcctcacgcttggataccgttcttcggccgaagatggacgctgcctggaacctccatgaactcactcgacaccttgacctcaccgccttcgtattgttctcgagcgctaccggtgtactcggcaatgcgggccaggccaactacgcagcggcaaacgtattcctcgatgccttggcacagacgcggcgcacagaaaacctgcccggccacagccttgcttgggggctctgggctgaggcttcagccatgaccgccggactggcggagactgatcgtcataggatcgcgcgcctgggcgctcaacctctgaacgaggctgaagctctggcccttctggacaaggccgtgaccggtgatggcgaaggtctgctcgtacccgtgcgtttgaacctcccggcactccgcgcacttgcggattccggtcgcctccctgccctgctttccggcttggtccgcacccggccccgccgtgctgcagaaaccaaggccggctcgggtgtgggtctgcgcgatcgcctggccggtatgaacgaagctgaggctgagagacatctggtccgcctggtgcgctcggaagtggctaccgtactgggtcacgcgtccccggacgcggtgggctccaagcgatccttcaccgaactgggtttcgactcgttgacggcggtcgaattgcgcaaccgtctgacagcagccaccggtctgcggctgccggctaccctcatatttgaccacccgaatagcaccctcctggccgaacgtatacggctggagatactcccggagggtgcagcgacggaattggacgatcctgaagagaacgcgttccgcgaagcagtttcagctatacctatgtcacggttccgagaagcaggcctgttggatgtggtcttgcagctcgcgggacctaagcggcagcaagaaacggcggtcgagggcgaagaaaccgagtcgatcgacgagatggatgtagataaccttattcggatggcactggacgggaaagactcctgatgacataaccccttggggcctctaaacgggtcttgaggggttttttgaggac

SEQ ID NO: 30 - DNA, 5627 bp, Artificial Sequence
  DNA fragment
gtaatgagaccttgaggtaaaccaacgccacgcgtagtgagacatacacgttcgttgggttcacgactcaacacgctagggacgtgaagtcgattccttcgatgcattgtaatagccaccaaaagagtgatgatagtcatgggtgtctgtagcacgtgcatcgctcattacaacggttataataagcacgtagtggctgttcacattcgaacggtgtctgctttgacaacatgctgtgcggtgttgtaaagtcgtggccaggagaatacgacagcgtgcaggactgggggagttatgtcgaacgaacaaaagctccgtgattatttgaagcgcgtcaccacagatcttgcagaaacccggcgtcgtctgggtcaagccgaggcggcacggcacgaaccaatagcgattgtcggcatggcctgccgctatccagggggtgtagagtctccagaagacctgtgggaactggttgcggagggccgcgacgccatcgatgtcatgccaggcgaccggggttgggatgtcgacgcgctgtatgatcctgacccgagctcgaccggtaagacgtactctcgcgagggtggattcctgcgaaacgcagcggaattcgatcccgcgtttttcggcatctcacctcgggaagccctggcgatggatccacagcaacgtttgctcttggaaactagctgggaggcgttcgagcgcgccggtatcgaccccgcaaccctgcgcggatcgcggacgggtgtgttcgccggtgtcatgtatcatgattacgggtctcggctgggtaccggaacggtacccgaggacgtcgagggctatgtcggcaacggaagcgccggttcgatcgccacgggtcgtatcgcctacacccttggcctggaaggtccggcggtcaccgtcgataccgcgtgcagctctagtctggtcgccatgcatttggccatccaagcgatacggcaaggagagtgcagcatggcgctggccggaggtgtgaccgtcatggcaaccccggacacctttgtggaattctcgagacagcgcggtctggcccccgacggccgctgtaaggctttcggagcaggagccgatggtaccggctgggcagagggagctggtatgctgctcgtggaacgtctgtcggatgctgaacgtttgggccatcccatccttgctgtcgtacggggtagcgcggtcaaccaggacggagccagtaacggcttgaccgcgccaaacggaccctcgcagcaacgcgtgatacgccaggccctggccacagcaggtttgggtcccaccgatatcgacgcggtcgagggtcacggaaccggcacgtccctgggtgaccccattgaagtgcaagcgctgcaagcgacctacggccaggagcggccggcagagcggccgttgtggttgggtagcctcaagtctaacattgggcacgcccaggcggccgctggtgtgggcggtgtgatcaagatggtcatggcccttcgggaaggcgtgctgccgcggacccttcacgctgacgaaccttcaccgcatatcgattggacagccggtgcggtccgcctcctgaccgaacaatccgcctggccggacaccgatcgtccacggcgtgccgcggtgtcgtccttcggagtctcgggcaccaacgcgcacgttatcattgagcagccatccgaacctgtagaacctgcggacacggacccggagtcacacagcgacagcgaggcagattcggatggaaccccagtggtacaccctgcactgctcccctggcctgtctccgcccggggtgcagatgccgtcagagctcaagctgcccgtttgcatgcgcatctgttggccaggccggatctcacggcggctgatgtagctttcagccttggcaccacacggaccgcgctgcctcatcggtttattgcactgggtaccgaccgcgccgaattgatcaacaccctcgcccggttcgccgaaggctcggaatcagcggctgatggcctcaccggcactgcgaccccaggcgcaaccgcattcctcttcagcggccaaggctcacaatgggcgggcatgggtagagaactccaagctcggttcccccgctttaggcaggccttggatgagacgaggctaggtggaggctcagtgatgataagtctgcgatggtggatgcatgtgtcatggtcatagctgtttcctgtgtgaaattgttatccgctcagagggcacaatcctattccgcgctatccgacaatctccaagacattaggtggagttcagttcggcgtatggcatatgtcgctggaaagaacatgtgagcaaaaggccagcaaaaggccaggaaccgtaaaaaggccgcgttgctggcgtttttccataggctccgcccccctgacgagcatcacaaaaatcgacgctcaagtcagaggtggcgaaacccgacaggactataaagataccaggcgtttccccctggaagctccctcgtgcgctctcctgttccgaccctgccgcttaccggatacctgtccgcctttctcccttcgggaagcgtggcgctttctcatagctcacgctgtaggtatctcagttcggtgtaggtcgttcgctccaagctgggctgtgtgcacgaaccccccgttcagcccgaccgctgcgccttatccggtaactatcgtcttgagtccaacccggtaagacacgacttatcgccactggcagcagccactggtaacaggattagcagagcgaggtatgtaggcggtgctacagagttcttgaagtggtggcctaactacggctacactagaagaacagtatttggtatctgcgctctgctgaagccagttaccttcggaaaaagagttggtagctcttgatccggcaaacaaaccaccgctggtagcggtggtttttttgtttgcaagcagcagattacgcgcagaaaaaaaggatctcaagaagatcctttgatcttttctacggggtctgacgctctattcaacaaagccgccgtcccgtcaagtcagcgtaaatgggtagggggcttcaaatcgtcctcgtgataccaattcggagcctgcttttttgtacaaacttgttgataatggcaattcaaggatcttcacctagatccttttaaattaaaaatgaagttttaaatcaatctaaagtatatatgagtaaacttggtctgacagttaccaatgcttaatcagtgaggcacctatctcagcgatctgtctatttcgttcatccatagttgcctgactccccgtcgtgtagataactacgatacgggagggcttaccatctggccccagtgctgcaatgataccgcgagagccacgctcaccggctccagatttatcagcaataaaccagccagccggaagggccgagcgcagaagtggtcctgcaactttatccgcctccatccagtctattaattgttgccgggaagctagagtaagtagttcgccagttaatagtttgcgcaacgttgttgccattgctacaggcatcgtggtgtcacgctcgtcgtttggtatggcttcattcagctccggttcccaacgatcaaggcgagttacatgatcccccatgttgtgcaaaaaagcggttagctccttcggtcctccgatcgttgtcagaagtaagttggccgcagtgttatcactcatggttatggcagcactgcataattctcttactgtcatgccatccgtaagatgcttttctgtgactggtgagtactcaaccaagtcattctgagaatagtgtatgcggcgaccgagttgctcttgcccggcgtcaatacgggataataccgcgccacatagcagaactttaaaagtgctcatcattggaaaacgttcttcggggcgaaaactctcaaggatcttaccgctgttgagatccagttcgatgtaacccactcgtgcacccaactgatcttcagcatcttttactttcaccagcgtttctgggtgagcaaaaacaggaaggcaaaatgccgcaaaaaagggaataagggcgacacggaaatgttgaatactcatactcttcctttttcaatattattgaagcatttatcagggttattgtctcatgagcggatacatatttgaatgtatttagaaaaataaacaaataggggttccgcgcacatttccccgaaaagtgccagatacctgaaacaaaacccatcgtacggccaaggaagtctccaataactgtgatccaccacaagcgccagggttttcccagtcacgacgttgtaaaacgacggccagtcatgcataatccgcacgcatctggaataaggaagtgccattccgcctgacctcgtctcatactgctttcgcggcgcggtccatccgccgatggcatggccgaagtccaacgcgagttggctgaagctggagcgtccgtagaagtactggcgtgcgatgctgcggaccgcgacgctttggcccaggtactggacggtcgagagctcacggctgtcatccatgcggccggcgtcctggacgatggagtgctggaagcgctggacgcgtcgcggttggacaccgtcttgcaaccaaagatggatgcggcatggaacctgcacgagcttacacggcacctggacttgacagcgtttgtcttgttctccagcgccaccggcgtcctgggcaacgctggccaggcgaactatgcggccgctaacgtattccttgacgcattggcacaaacccgcaggaccgaaaacctccctggtcatagcttggcatggggtctgtgggcagaagcttccgccatgacggccggcctgagcgaaaccgaccgccatagaattgcccgtctgggcgctcagccgctcaacgaaaccgaagcactggcacttttggacagggctttgggtgaagacgcacccgcactgttggtccctgtgcgtctgaaccttgcggcactgcagggtcgctctcaagcggttcctgccgttctgcgcgcgcttgtaccagtccgggcgcggcgccaggccgcggtcggcgcagccgctggttctggtggaggcctcgtagaaaggcttgcggctatgtccgagtcacgacgtgccgcgcatctgcttgatctggtccggaccgaagtcgctggtgtactgggccaccgctccgcggctaccattgaacccgagcgcgccttcaaggacctgggtttcgattcgctcaccgccgtcgagctgcggaaccggctccatgctgccaccggtctgaagccggcggccaccgtggtcttcgaccacccaacctccgccgacctggcgcgccaccttcgtacgcagatcccagatctgccagctgccggaccagaatgtcttctgggcgaactggatcggatagaacagatgctgacagatgttgaccccacagacgaaaagtcgggagacatccagcgccgcctgacggcgctgcttgctcgctttgacgaggccgcggggccagtcgaagcagctcaagtggcagataagatcgatgcagccaccgacgatgaaatttttgctttcattgacaacgagctcggttgatagcataaccccttggggcctctaaacgggtcttgaggggttttttgactac

SEQ ID NO: 31 - DNA, 5629 bp, Artificial Sequence
  DNA fragment
aactagagaccgtcagcgtcgacgccacgcgtagtgagacatacacgttcgttgggttcacgactcaacacgctagggacgtgaagtcgattccttcgatgcattgtaatagccaccaaaagagtgatgatagtcatgggtgtctgtagcacgtgcatcgctcattacaacggttatagcacgcggctgttcacattcgaacggtgtctgctttgacaacatgctgtgcggtgttgtaaagtcgtggccaggagaatacgacagcgtgcaggactgggggagttatggcggaccacgacaagctcgttgattatttgaagcgcgtcaccgcagatcttcaacagacccgccagcgtctgcgggagtacgaaacccagagccatgaaccaatagcaatcgttggcatgggctgccgctaccctggatccgtggcatcccctgaagagctgtggcgcctggtccacggtggcgtggacgccgtcggcggtctcccgaccgaccgggggtgggatgtggaagccttgtacgatcctaaggcacagaacccgggcacgacctatgcccgtgaaggtggctacctgaccggagcgacagagttcgacccggaattctttggtatctccccccgtgaggccctggccatggatcctcaacagcgcttggtgctcgaggtcgcttgggaaaccctggagcatgccggcatcgactccgccacactgcgcggcagctcgaccggtgttttcgtgggatgtaactatcaggagtaccgggcaaggctgtcggaggtacaggaaggccttgaaggccatctggtgaccggctccgtaagctccgtggtgtcgggccgtgtttcttacgtcctcggccttgagggccccgctcttacggtcgacaccgcttgttccagtagcttggtcaccctgcacttggcttgcgaagcacttaggcggaacgaatgtaccatggcacttgccggcggagtggctgtcatgtcaacaccgcataccatcacgggtttctcccggcaacggggcgtggcagcggacggccggtgcaaggcatttagcgcaagcgcagacggtatgggtttcggcgaaggtgtaggtcttctgctcgtggaacgtctgtcggatgctcgacgtttgggccatcgcgtgcttgctgtcgtacggggtagcgcggtcaaccaggacggagccagtaacggcttgtccgcgccatcaggacccgctcagcaacgcgtgatacgccaggccctggtcaacgccggtgtgcaggccagccaggtcgacgtggtcgaggctcacggaaccggcacgcgcctgggtgaccccattgaagctcaagcgctgcaagcgacctacggccagggtcggccggcagagcggccgttgtggttgggtagcctcaagtctaacattgggcacgcccaggcggccgctggtgtgggcggtgtgatcaagatggtcatggcccttcgggaaggcgtgctgccgcccacccttcacgctgacgaaccttcaccgcatatcgattggacagccggtaacgtccgcctcctgaccgaatcacgggaatggccggaagcgggtcagccacggcgtgccgcggtgtcgtccttcggaatctcgggcaccaacgcgcacgttatcttggaggcggcagaagcagttgacgcatcgggggaggctgacggcggtgccggcgacgaaggcacgccagtgctttctggaaccgacgtggtagcctggcctgtcagtgcagcctcgccagacgccctgcgggcacaggccgaaagattgagggctcatgtggctgagcgtcctgggttggccagcgcggatgtagctttctcgcttgcaactagcaggtcggcccttgcacggcgcgcgctggttgtgggtggggatcgcgacgagctggtcgcaggcctggagagtctggccgcagaccggcccggcaacggccttgtcaagggtttggctgacctcgcaaccaagccggtgttcgtcttccccggccagggatcccaatgggccggaatggccgtcgaactgctcgatagctccccagtctttgcggatagtatgcaagcttgctcggaagctctgaacgagttcgtagattggaacctcctggaggtcctgcggtccgatgacgaagagttgagcaaccgcgtagatgtggtccagcctgtgctgtgggccgtaatggtgtccctcgcggcactctggcaggcgtgcggcgtccgcccggcagccgtggtaggccattctcagggcgagatagcagctgccgtggtcgctggtgccctgtcactccgtgatggggcccgcgtggtagccttgcggtcggcggtaatagcgcggctgttggccggtaagggtgcgatggcctccgttgcgctcgcatccgataccgtgcgtgaacgcctgaccccctgggagggtcgtctgtccttggcggctgtaaacggcccttcgtcatcggtggtctgcggccacttggacgcgttggatgagttcgtgtctgcattggaacatgacggcgtgagggtgcgcaggatagccgtggactacgcgtcccactctgtcttcgtagaacaagcggaggaagagttgcgcaacgtcctgaccgaagtctcgccgttgccgggcgaggtaccgttctattccaccgttaccggcgcggtgctcgacaccacgacccttgatgctggatattggtaccggaacttgcgccagacggtacgtttcgaagagactgtgcgcgaactgaccaggcgcggtcacgatgcattcattgaagtttctgcccatccggtcctgacggtcggcattcaggacaccttggaggctaccggaacacgccacgccgtctgtgggacactgcgtcgcggcgaaggaggcgcgcaacggctcctgacgtcccttggagaagcatgggtggcgggcatcgcggtcgattggtcgcgattgacgcccaccgctaccgccgtagaactgccaacgtacgcctttcaacattgagacgaggctaggtggaggctcagtgatgataagtctgcgatggtggatgcatgtgtcatggtcatagctgtttcctgtgtgaaattgttatccgctcagagggcacaatcctattccgcgctatccgacaatctccaagacattaggtggagttcagttcggcgtatggcatatgtcgctggaaagaacatgtgagcaaaaggccagcaaaaggccaggaaccgtaaaaaggccgcgttgctggcgtttttccataggctccgcccccctgacgagcatcacaaaaatcgacgctcaagtcagaggtggcgaaacccgacaggactataaagataccaggcgtttccccctggaagctccctcgtgcgctctcctgttccgaccctgccgcttaccggatacctgtccgcctttctcccttcgggaagcgtggcgctttctcatagctcacgctgtaggtatctcagttcggtgtaggtcgttcgctccaagctgggctgtgtgcacgaaccccccgttcagcccgaccgctgcgccttatccggtaactatcgtcttgagtccaacccggtaagacacgacttatcgccactggcagcagccactggtaacaggattagcagagcgaggtatgtaggcggtgctacagagttcttgaagtggtggcctaactacggctacactagaagaacagtatttggtatctgcgctctgctgaagccagttaccttcggaaaaagagttggtagctcttgatccggcaaacaaaccaccgctggtagcggtggtttttttgtttgcaagcagcagattacgcgcagaaaaaaaggatctcaagaagatcctttgatcttttctacggggtctgacgctctattcaacaaagccgccgtcccgtcaagtcagcgtaaatgggtagggggcttcaaatcgtcctcgtgataccaattcggagcctgcttttttgtacaaacttgttgataatggcaattcaaggatcttcacctagatccttttaaattaaaaatgaagttttaaatcaatctaaagtatatatgagtaaacttggtctgacagttaccaatgcttaatcagtgaggcacctatctcagcgatctgtctatttcgttcatccatagttgcctgactccccgtcgtgtagataactacgatacgggagggcttaccatctggccccagtgctgcaatgataccgcgagagccacgctcaccggctccagatttatcagcaataaaccagccagccggaagggccgagcgcagaagtggtcctgcaactttatccgcctccatccagtctattaattgttgccgggaagctagagtaagtagttcgccagttaatagtttgcgcaacgttgttgccattgctacaggcatcgtggtgtcacgctcgtcgtttggtatggcttcattcagctccggttcccaacgatcaaggcgagttacatgatcccccatgttgtgcaaaaaagcggttagctccttcggtcctccgatcgttgtcagaagtaagttggccgcagtgttatcactcatggttatggcagcactgcataattctcttactgtcatgccatccgtaagatgcttttctgtgactggtgagtactcaaccaagtcattctgagaatagtgtatgcggcgaccgagttgctcttgcccggcgtcaatacgggataataccgcgccacatagcagaactttaaaagtgctcatcattggaaaacgttcttcggggcgaaaactctcaaggatcttaccgctgttgagatccagttcgatgtaacccactcgtgcacccaactgatcttcagcatcttttactttcaccagcgtttctgggtgagcaaaaacaggaaggcaaaatgccgcaaaaaagggaataagggcgacacggaaatgttgaatactcatactcttcctttttcaatattattgaagcatttatcagggttattgtctcatgagcggatacatatttgaatgtatttagaaaaataaacaaataggggttccgcgcacatttccccgaaaagtgccagatacctgaaacaaaacccatcgtacggccaaggaagtctccaataactgtgatccaccacaagcgccagggttttcccagtcacgacgttgtaaaacgacggccagtcatgcataatccgcacgcatctggaataaggaagtgccattccgcctgacctcgtctcaactggtcttcgaccaccctaccccgctggctatcgccgcatacttgaaggccgagctgtacggacctgatccgggtgacgattccagcgtcctgaccgagctcgatggcctgtcccaacggttggcggcaatcgatcccgacaccaacacccgccttgagatcaccctgcgtctgcgctcgttgctgacgcagtggtccgaaccggacggtggacgcaccactgcagagacagcaacggcaacgagtaccacggcattggaatcggcatccgcggacgaggtcctggctttcattgacaccgagttggggatttgatgacataaccccttggggcctctaaacgggtcttgaggggttttttgccgtg

SEQ ID NO: 32 - DNA, 5608 bp, Artificial Sequence
  DNA fragment
acaatgagaccttgaggtaaaccaaataagacgccacgcgtagtgagacatacacgttcgttgggttcacgactcaacacgctagggacgtgaagtcgattccttcgatgcattgtaatagccaccaaaagagtgatgatagtcatgggtgtctgtagcacgtgcatcgctcattacaacggttatcacgtagtggctgttcacattcgaacggtgtctgctttgacaacatgctgtgcggtgttgtaaagtcgtggccaggagaatacgacagcgtgcaggactgggggagttatggcgggcccaccgcctttccctcgtcggcgtggcccctcaggccgacgtcggtgcggcggacgggctacaccgggtagcgtccgggaccgcaccggcagacgcccagcggctgtccccagccgcgccgtgtgcgcggccgacctttgtgaagagaacgacgatggctccaagaacgtgtcggaacaccgcggatcagcgggtggtagcgttctgtttcctcgtacgggcacagtcctgccatgggtgcttacgggaccgggcgcagcggcggtgcgtgcacgctccgaagcgctgcgcacccacctccgcgcctctacggaatggagccctgcaggcgtaggtcaggcgctgctggcaggaacaggggcgggcgcggacacccaccgtgccgttgttctcgccggtgatcgtgcccaaactctgaatgccctggccgcgctgtctgcaggagcggaccacccagccgtctttaccagcacccgtgccgacgccagcccagctggtccagtgtttgtgtttccaggccaggggtctcaatggactggtatggctcgcgaattgttggattctgcccccgtatttgcccgtaaattgcatgattgcgccgacgcatttgccccgtatttgggtcacagcctcctggattccgttactggggcggccggcgggccagagcctgttggcgcggatgttgtgcaaccagccttgttcgcagtgatggttgccttgacggatctctggaatgcggccggtgtggcaccaggcgccttgctcggtcattcactgggggagctcgccgccgcccacgtcgctggcgttctcagcctggacgattcggcgcgcgtggtcgcgcgctggagccaagcccaagcaactctcgcaggccgtggggacatggtttccgtgctgctgcctgcggacgaactggcggatctgttggaccgccgttggccggggcgtctggtagttgcggtggagaatggcccgggtagtgccgtagccagcggtgatctggatgccgcggcagaacttgtagcccatcttactgcggaaggcattcatgcgcgtcgtgtcgatgtcggcttggccgcgcactctccccacatcgacgctattctcccccgcatccgcgcggatattgctccgatccgcgcacatacccccagtatccctgtttacagcgcgctgcacggcggcgcactcgacggtacccctatggatgcggcgtattggtgccgtaatttgcgttcaactgtgcgttttgcggatgctacgcgcgcagctttggaagcaggccatacaacatttgtggaagtttcacctcatccggtcttgacgacggccatggaagtgagtgccacccgtgcggcccatgcggcgaccgtattgggaactcttcgtcgtggtgagggtggtccaagccgttttctggcatcactggcggaactccatgtttcaggtggtgatgccgatttgcgtacggttctgcccgcgagccaggcggctggcttgccggaaaccgtcctgacggcgggtccgcgtggcgagagcgctgacggcgatagccgtcatgaagtgctgtgtgcacgtctggcaccgctcgacccagccgaacgccgcgcccaacttctgacagttgtgcgtgaatctgcggcggcggccttggatggcgatgaccagggaagcatcgatggtcgtcgcacctttcgtgatttgggtattacttcacttgcggcggttggcattcgtgatcgcctgcactccgcgacaggtcttcgcctgtcacctaccgtggtctttgaccatcctactccagatgcattggccgcccaccttgatacagaactgtttgggaccggggcagatgccgaaccggctccggcagccggcggccgtgcagttccacatgatgaaccgatggcaattgtgggtatggcctgtcgttacccgggtggagttggcgcaccggcggatctctggcgtactgtcctggcaggggtggatgcggtcggcccattgccagccgatcgtggctggaatatcgctgatggctacgacccggaacttgccgggccgggccgttttagccaacgcgagggcgggtttctgcacgatgcggcagagtttgacgccgaattcttcggcatctcaccccgtgaagctctggccatggatccgcaacagcgcctcgcccttgaaagtgcatgggaagcgattgaagacgcgggcttggatgcgcattcgctccgtggcagtcgtaccggagttttcctcggcctgattacccaggattatggcccgcgcgcgggcgagccgactacccgtgcgggtgccgttgaaggtcatctgtttctggggtcaacggggagtgtagcgtcggggcgcctgagttacaccctcggcctggagggcccttccctgaccattgatactgcctgcagttccagcctggtagcgttgcatgaggcgtgccaagcattgcgtacgggtgactgcgatatggcactgacaggcggcgtgacggtaatgccttctacaggcatgctggtcgagttttcgcgtcagcgtggtctgtcacctgatggccgttgtaaagcctttagtgcgtcagctgatggctttgggctggcagaaggggttggtatgcttgttgtggaacgcttgagcgacgcacgtcgcctcgggcatcgtgtgcttgccgtggttcgcggttcagcggttaatcaagatggggccagtaatggtctgtcggcaccatccggcccggcacaacagcgtgttattcgtcaagcgcttgtgaatgcgggtgtccaggcctctcaagtggacgtggttgaagctcatggtaccggcactaagcttggtgatccaattgaagcgcaggcgcttcaggccacttatggtcaaggccgcccggcagaacgtcctttgtggctcggatctctgaaaagcaatattgggcatgcacaagcagcggcgggtgttggtggcgttatcaaaatggttatggcactgcgcgagggcgtacttccccctacgcttcatgctgattgagacgaggctaggtggaggctcagtgatgataagtctgcgatggtggatgcatgtgtcatggtcatagctgtttcctgtgtgaaattgttatccgctcagagggcacaatcctattccgcgctatccgacaatctccaagacattaggtggagttcagttcggcgtatggcatatgtcgctggaaagaacatgtgagcaaaaggccagcaaaaggccaggaaccgtaaaaaggccgcgttgctggcgtttttccataggctccgcccccctgacgagcatcacaaaaatcgacgctcaagtcagaggtggcgaaacccgacaggactataaagataccaggcgtttccccctggaagctccctcgtgcgctctcctgttccgaccctgccgcttaccggatacctgtccgcctttctcccttcgggaagcgtggcgctttctcatagctcacgctgtaggtatctcagttcggtgtaggtcgttcgctccaagctgggctgtgtgcacgaaccccccgttcagcccgaccgctgcgccttatccggtaactatcgtcttgagtccaacccggtaagacacgacttatcgccactggcagcagccactggtaacaggattagcagagcgaggtatgtaggcggtgctacagagttcttgaagtggtggcctaactacggctacactagaagaacagtatttggtatctgcgctctgctgaagccagttaccttcggaaaaagagttggtagctcttgatccggcaaacaaaccaccgctggtagcggtggtttttttgtttgcaagcagcagattacgcgcagaaaaaaaggatctcaagaagatcctttgatcttttctacggggtctgacgctctattcaacaaagccgccgtcccgtcaagtcagcgtaaatgggtagggggcttcaaatcgtcctcgtgataccaattcggagcctgcttttttgtacaaacttgttgataatggcaattcaaggatcttcacctagatccttttaaattaaaaatgaagttttaaatcaatctaaagtatatatgagtaaacttggtctgacagttaccaatgcttaatcagtgaggcacctatctcagcgatctgtctatttcgttcatccatagttgcctgactccccgtcgtgtagataactacgatacgggagggcttaccatctggccccagtgctgcaatgataccgcgagagccacgctcaccggctccagatttatcagcaataaaccagccagccggaagggccgagcgcagaagtggtcctgcaactttatccgcctccatccagtctattaattgttgccgggaagctagagtaagtagttcgccagttaatagtttgcgcaacgttgttgccattgctacaggcatcgtggtgtcacgctcgtcgtttggtatggcttcattcagctccggttcccaacgatcaaggcgagttacatgatcccccatgttgtgcaaaaaagcggttagctccttcggtcctccgatcgttgtcagaagtaagttggccgcagtgttatcactcatggttatggcagcactgcataattctcttactgtcatgccatccgtaagatgcttttctgtgactggtgagtactcaaccaagtcattctgagaatagtgtatgcggcgaccgagttgctcttgcccggcgtcaatacgggataataccgcgccacatagcagaactttaaaagtgctcatcattggaaaacgttcttcggggcgaaaactctcaaggatcttaccgctgttgagatccagttcgatgtaacccactcgtgcacccaactgatcttcagcatcttttactttcaccagcgtttctgggtgagcaaaaacaggaaggcaaaatgccgcaaaaaagggaataagggcgacacggaaatgttgaatactcatactcttcctttttcaatattattgaagcatttatcagggttattgtctcatgagcggatacatatttgaatgtatttagaaaaataaacaaataggggttccgcgcacatttccccgaaaagtgccagatacctgaaacaaaacccatcgtacggccaaggaagtctccaataactgtgatccaccacaagcgccagggttttcccagtcacgacgttgtaaaacgacggccagtcatgcataatccgcacgcatctggaataaggaagtgccattccgcctgacctcgtctcaattagcacctgcttggattaactac

SEQ ID NO: 33 - DNA, 5647 bp, Artificial Sequence
  DNA fragment
attccgagaccatgtcgatactgaacacgccacgcgtagtgagacatacacgttcgttgggttcacgactcaacacgctagggacgtgaagtcgattccttcgatgcattgtaatagccaccaaaagagtgatgatagtcatgggtgtctgtagcacgtgcatcgctcattacaacggttatgaatcgacgcacactcccttccttggtgcacgcggtcgatcttgacggctggcgagaggtgcggggaggatctgaccgacgcggtccacacgtggcaccgcgatgctgttgtgggcacaatcgtgccggttggtaggatccagcgatgcagtccgcagaaaaggcaaagcctgctgatggcgccgcagcggcattgctggcaaccctcacccataaacggcgtctggacgcggccaccccgaaggaaagcgcactgtggttgctggaccgcctgctccctgaagcgggtgtaaacaatgttccactggccgtccgcgtcgatggtcgtctggacgccgcggctttgcaagcagcggtcgacggtctcgtgcgccgtcacgaggtgttgcgcaccgtatacctggatcggcaggccggtctggtgcgtgaagtgctgggagaggacaccccaggaccgcgcgtggaggtccatgacacggtggccggcgtcccggagaaagccttgcgtgaattcgccgctacaccgatccggtgtgacggccggctgatgctgcgcgcagcggtgttccgcggtccggatgctgacaccctcgcggtcgttgtgcatcacctggtgttcgacgccgcttcggtacctgtactgatcgccgaacttgccgctgcctacgacgcaagagccaccggtcgtgacttgcctgatgaactgcgcaccccggtcgcggcattgcgggatcccgcaccccgtgaggaatccctggcatattggcgcaccgccctggatggtttcgacccagcgggactggacctcgattgcgcacggcccgccccagcgcgtgcgaccctcgtgggtgacaccgttcttcacgtccttgacgatgaaacccgtgacctggtccggggcctgcagcgaacgcaaagagcaccagaagctgttatcctgttcacggcattctgtctgctcttggcagctcacggtgcgggtccagatttggtcgtgggctccccggtgaacatatgagacgaggctaggtggaggctcagtgatgataagtctgcgatggtggatgcatgtgtcatggtcatagctgtttcctgtgtgaaattgttatccgctcagagggcacaatcctattccgcgctatccgacaatctccaagacattaggtggagttcagttcggcgtatggcatatgtcgctggaaagaacatgtgagcaaaaggccagcaaaaggccaggaaccgtaaaaaggccgcgttgctggcgtttttccataggctccgcccccctgacgagcatcacaaaaatcgacgctcaagtcagaggtggcgaaacccgacaggactataaagataccaggcgtttccccctggaagctccctcgtgcgctctcctgttccgaccctgccgcttaccggatacctgtccgcctttctcccttcgggaagcgtggcgctttctcatagctcacgctgtaggtatctcagttcggtgtaggtcgttcgctccaagctgggctgtgtgcacgaaccccccgttcagcccgaccgctgcgccttatccggtaactatcgtcttgagtccaacccggtaagacacgacttatcgccactggcagcagccactggtaacaggattagcagagcgaggtatgtaggcggtgctacagagttcttgaagtggtggcctaactacggctacactagaagaacagtatttggtatctgcgctctgctgaagccagttaccttcggaaaaagagttggtagctcttgatccggcaaacaaaccaccgctggtagcggtggtttttttgtttgcaagcagcagattacgcgcagaaaaaaaggatctcaagaagatcctttgatcttttctacggggtctgacgctctattcaacaaagccgccgtcccgtcaagtcagcgtaaatgggtagggggcttcaaatcgtcctcgtgataccaattcggagcctgcttttttgtacaaacttgttgataatggcaattcaaggatcttcacctagatccttttaaattaaaaatgaagttttaaatcaatctaaagtatatatgagtaaacttggtctgacagttaccaatgcttaatcagtgaggcacctatctcagcgatctgtctatttcgttcatccatagttgcctgactccccgtcgtgtagataactacgatacgggagggcttaccatctggccccagtgctgcaatgataccgcgagagccacgctcaccggctccagatttatcagcaataaaccagccagccggaagggccgagcgcagaagtggtcctgcaactttatccgcctccatccagtctattaattgttgccgggaagctagagtaagtagttcgccagttaatagtttgcgcaacgttgttgccattgctacaggcatcgtggtgtcacgctcgtcgtttggtatggcttcattcagctccggttcccaacgatcaaggcgagttacatgatcccccatgttgtgcaaaaaagcggttagctccttcggtcctccgatcgttgtcagaagtaagttggccgcagtgttatcactcatggttatggcagcactgcataattctcttactgtcatgccatccgtaagatgcttttctgtgactggtgagtactcaaccaagtcattctgagaatagtgtatgcggcgaccgagttgctcttgcccggcgtcaatacgggataataccgcgccacatagcagaactttaaaagtgctcatcattggaaaacgttcttcggggcgaaaactctcaaggatcttaccgctgttgagatccagttcgatgtaacccactcgtgcacccaactgatcttcagcatcttttactttcaccagcgtttctgggtgagcaaaaacaggaaggcaaaatgccgcaaaaaagggaataagggcgacacggaaatgttgaatactcatactcttcctttttcaatattattgaagcatttatcagggttattgtctcatgagcggatacatatttgaatgtatttagaaaaataaacaaataggggttccgcgcacatttccccgaaaagtgccagatacctgaaacaaaacccatcgtacggccaaggaagtctccaataactgtgatccaccacaagcgccagggttttcccagtcacgacgttgtaaaacgacggccagtcatgcataatccgcacgcatctggaataaggaagtgccattccgcctgacctcgtctcagagattggccctgatgctatacttaccggcctggtagaacaaaaccagaccctcgacacgcaggccgtacccgtactgcgccgtgaccgggacgaggtgcgcgctgcagtcgaggctgtcggtcgcctgcacctggcgggcatccccgtggattggccggcggtccttcctggtgcccgccgtgtcgaactgccgacctacgcgttccaacacgagcgctactggctggacccagaggaactggcggctgcagccgaggacaccgttgcaccttcaggtacggaagtccccgaccccgatacccgcttctggggcgccgtcgcagacgaggatttgggcagcttggcagcgctgcttggtatagacggagaaaagggaggtgctcaggaccgcgcggctgtggaagcggctctgcctgtgctggcttcgtggttgggccgccggcaggctgcggcacgcgtgtcccactatcgggtgggttggacgccagtcgctagacggcctgacggcacgacagcgcggttgcggggtatctggctgttgaccattcccgcacgcataggcgccgacgatgcgttggtgactcgtctggcaagtgcattgggcggtgccggagccgacgttcgtgtggttacggttggtgatccgggagcagattcgtatgacgatctggctgccgaagtttcgtcgttgaccgccgacggcggtgaactcgccggcgtcctgagtctgctgggattggcgtctgctgatggtcccggggatgcgcgtgaggccgcagtaggtacactcgccctgctgcgtgcgctctcgggttcggttgcatcagtccctgtttggtcactgacatctggtgccgtatcgaccggcggatcagagcgtgtaagcgcccctgcccaggctgtgctctggggactgggtcgcctgctggccgaagacagtgatgtgcgttgggcgggcgttgtggatgtgccggcgccgtgtggtgatcgtgtgttgcgccgcctcgccgaagtgctcgcaaatccagccgaggagactgaagtggccgtacgtgacgctggcgtgtttgcgcgtcgtcttctgcgtgcaaccggggcagcggacgggcccgcccgtcctactgctcttgctccccgcggcaccctgttggtatcaggcggttcagatacatggcgtgatcgtgttgctcgccgtctgcttgcatcgggcgcggcacatgtgttggtcgcgacagcgccagatgagccagaacctgcttctaccccggggtcggcggttaccggggtttcccgtgtcgtgtgtgacgtttctgacggtccggctctggcgcatttggccgccagcctgccggcgggccccgacggccgtccgctgacgggtgtagtgcacgcgcccccggcaacagccagcgatggacccttggataaggcactggatgaggtattgggtgctggactgccggcgctggcaggcgtatcatcgaccgctggcccgatcgccctcttcctggccgtggatgttgatgacctggttggcgccccgggagcaggcgccgtcgcggctctggccggttggtgggaagccgccgcacgcgtacgtacggccgaccgcgcacctgtacgcctgattgcggcagatcccgatgcactggatctggccgtgttggatcgtgcaatggaacgtgccgatggtctgctcgtcgtgacgggtcgtgattgggcacaatacgcgggaacccacgcggatacccgcggtcgccgcttgctggaaggagtgcctgaggcacgtgcagttcttgcagcagcagcccctgcgggtgacgcgggcaagagcgggctgttggctggtgtagacgggccggaatcgttgcgtcgcgtgttggcggcgcgcgaagcagaccacaagctcgcgaccctggtggagctggtgcgcggtcaagtcgcggtcgtcctcggacacgcgagtgccgatgcggtcagtgcggatggagactttatggatctgggatttgcttcgctgacagccgttgagtttggccaccgtttaagcgccatcacaggcctcaaattgcctacgactctggtctacgaccacctgaacccagtggaactggccgagcacctggctgacgagctggcgagggaactgaccgccgcgtgatagcataaccccttggggcctctaaacgggtcttgaggggttttttgcaaac

SEQ ID NO: 34 - DNA, 5611 bp, Artificial Sequence
  DNA fragment
tagatgagaccgcgcagatgtacgacaatatcgcacgccacgcgtagtgagacatacacgttcgttgggttcacgactcaacacgctagggacgtgaagtcgattccttcgatgcattgtaatagccaccaaaagagtgatgatagtcatgggtgtctgtagcacgtgcatcgctcattacaacggttatttagtcacccttgggccgtgcacgcggtcgatcttgacggctggcgagaggtgcggggaggatctgaccgacgcggtccacacgtggcaccgcgatgctgttgtgggcacaatcgtgccggttggtaggatccagcgatggcgaccccaaacgagaaagttgtggaggctctgcgcgcctccctcaaggaaaccgaactccttcgtcaacagaacaatgcgctccgcgcggccagctcggaaccagtagcaatcgttggcatgggctgccgcttccctggaggtgtggtatcccctgaaggtctctgggaagtcgtgttgtccggtgccgacgtcatctcggagttcccaaccgaccggggttgggatgtcgaaggtctgtatgatcctgacccggaccggcccggtaagacgtacggtcgccgtggtggattcgtcgacgcggtagcggacttcgatgccgggtttttcggcatctcacctcgggaagccctggcgatggatccacagcaacgtctgctcttggaaactagctgggaggcgttcgagcgcgccggtatcgaccccgcaaccctgcgcggatcgcggacgggtgtgttcgccggtgtcatgtatcatgattacgcgagcaggctgcgtgaggtacctggacaccttgaaggccttatgggcacgggcaacgccaccagcgtcatcgcgggtcgcttgtcttataccttcggactggagggcccgagtgtttcggtggacaccgcctgttcctcgagtctcgttgccctgcacctggctgtgcaagccctccgggcaggggaatgcgagatggccctcgcgggcggagtaaccgtgatggcgaccccagaggcgttcatcaacttcagtcgccagagaggtctggctgcagacggccggtgcaaggcgttcggtgcaggagcagacggcacgggttgggccgaaggagctggaatgagacgaggctaggtggaggctcagtgatgataagtctgcgatggtggatgcatgtgtcatggtcatagctgtttcctgtgtgaaattgttatccgctcagagggcacaatcctattccgcgctatccgacaatctccaagacattaggtggagttcagttcggcgtatggcatatgtcgctggaaagaacatgtgagcaaaaggccagcaaaaggccaggaaccgtaaaaaggccgcgttgctggcgtttttccataggctccgcccccctgacgagcatcacaaaaatcgacgctcaagtcagaggtggcgaaacccgacaggactataaagataccaggcgtttccccctggaagctccctcgtgcgctctcctgttccgaccctgccgcttaccggatacctgtccgcctttctcccttcgggaagcgtggcgctttctcatagctcacgctgtaggtatctcagttcggtgtaggtcgttcgctccaagctgggctgtgtgcacgaaccccccgttcagcccgaccgctgcgccttatccggtaactatcgtcttgagtccaacccggtaagacacgacttatcgccactggcagcagccactggtaacaggattagcagagcgaggtatgtaggcggtgctacagagttcttgaagtggtggcctaactacggctacactagaagaacagtatttggtatctgcgctctgctgaagccagttaccttcggaaaaagagttggtagctcttgatccggcaaacaaaccaccgctggtagcggtggtttttttgtttgcaagcagcagattacgcgcagaaaaaaaggatctcaagaagatcctttgatcttttctacggggtctgacgctctattcaacaaagccgccgtcccgtcaagtcagcgtaaatgggtagggggcttcaaatcgtcctcgtgataccaattcggagcctgcttttttgtacaaacttgttgataatggcaattcaaggatcttcacctagatccttttaaattaaaaatgaagttttaaatcaatctaaagtatatatgagtaaacttggtctgacagttaccaatgcttaatcagtgaggcacctatctcagcgatctgtctatttcgttcatccatagttgcctgactccccgtcgtgtagataactacgatacgggagggcttaccatctggccccagtgctgcaatgataccgcgagagccacgctcaccggctccagatttatcagcaataaaccagccagccggaagggccgagcgcagaagtggtcctgcaactttatccgcctccatccagtctattaattgttgccgggaagctagagtaagtagttcgccagttaatagtttgcgcaacgttgttgccattgctacaggcatcgtggtgtcacgctcgtcgtttggtatggcttcattcagctccggttcccaacgatcaaggcgagttacatgatcccccatgttgtgcaaaaaagcggttagctccttcggtcctccgatcgttgtcagaagtaagttggccgcagtgttatcactcatggttatggcagcactgcataattctcttactgtcatgccatccgtaagatgcttttctgtgactggtgagtactcaaccaagtcattctgagaatagtgtatgcggcgaccgagttgctcttgcccggcgtcaatacgggataataccgcgccacatagcagaactttaaaagtgctcatcattggaaaacgttcttcggggcgaaaactctcaaggatcttaccgctgttgagatccagttcgatgtaacccactcgtgcacccaactgatcttcagcatcttttactttcaccagcgtttctgggtgagcaaaaacaggaaggcaaaatgccgcaaaaaagggaataagggcgacacggaaatgttgaatactcatactcttcctttttcaatattattgaagcatttatcagggttattgtctcatgagcggatacatatttgaatgtatttagaaaaataaacaaataggggttccgcgcacatttccccgaaaagtgccagatacctgaaacaaaacccatcgtacggccaaggaagtctccaataactgtgatccaccacaagcgccagggttttcccagtcacgacgttgtaaaacgacggccagtcatgcataatccgcacgcatctggaataaggaagtgccattccgcctgacctcgtctcactttgccagaggaagcggctaacgcggctgacgcattcggtctgcaccccgcgcttctggatgcagccctgcacgccatcggcttgctgcaattggctgactcggagggaatgcgtctgccattcgcttggagtggagtttcgctccaagctgtcggcgctaccacgcttcgcgtgagaatcgcccccgacggtcgcggtggagctaccgttgacctgttcgacgaagcgggcctgcccgtcgccagggtcgagagtctgacccttcgcgaagtctcgcgcgagcagatggcggccgcggcctccgcggccggcgacgagtccttgttccaggtcgaatgggtaccggtggttggcgatcccgatgaagctgtgtcctgggccgtgctcggcgactcgccgctggcagagggcggattggtcttcgctgatgtagaagccttgctggccagctcccaggacctgccaggtacagtcgtgttggaatgccctgcagttgaaggtgctccagtgcctgatgcagttcgcgaccggctcaccggcgtgttgggcgtcctgcagcgctgggtggctgatgaacgactggcctcgtcccggttggtcgtggtcacgcgtggtgccgtcgccgcgagcgccaacgaaccagcggacgtccgcgtcgcgcctgtatggggcctcgtccgggcggctcaggccgaacatccggaccggttcgtactggcagatttgcctgcaggcgccggtgcccgcgagttggccgctggtctggcttgtgacgaaccgcagtgggcgatccgcgatggtgcgatccatgtaccacgtctggttcgcgctcaagactctaccgacggagcctccggtttcggcgatggccccgtcttgatcaccggagccagcggcgcgttgggtggagtggtagcgcgccacctcgtaagcgtgcacggtgtgcgtgaactcgtcttgctttcacgtaggggcctggcggcagagggaatggatacgctgcgggatgagctgacccaccaaggcgcatcggtcgaagtgctggcatgtgatgcggctgaccgcaacgctctggcacaggcgctgtcaggccgccggctgacggcagtgatccacgccgctggagtcttggacgatggtgtcctggaagccctggacgcctcacgcttggataccgttcttcggccgaagatggacgctgcctggaacctccatgaactcactcgacaccttgacctcaccgccttcgtattgttctcgagcgctaccggtgtactcggcaatgcgggccaggccaactacgcagcggcaaacgtattcctcgatgccttggcacagacgcggcgcacagaaaacctgcccggccacagccttgcttgggggctctgggctgaggcttcagccatgaccgccggactggcggagactgatcgtcataggatcgcgcgcctgggcgctcaacctctgaacgaggctgaagctctggcccttctggacaaggccgtgaccggtgatggcgaaggtctgctcgtacccgtgcgtttgaacctcccggcactccgcgcacttgcggattccggtcgcctccctgccctgctttccggcttggtccgcacccggccccgccgtgctgcagaaaccaaggccggctcgggtgtgggtctgcgcgatcgcctggccggtatgaacgaagctgaggctgagagacatctggtccgcctggtgcgctcggaagtggctaccgtactgggtcacgcgtccccggacgcggtgggctccaagcgatccttcaccgaactgggtttcgactcgttgacggcggtcgaattgcgcaaccgtctgacagcagccaccggtctgcggctgccggctaccctcatatttgaccacccgaatagcaccctcctggccgaacgtatacggctggagatactcccggagggtgcagcgacggaattggacgatcctgaagagaacgcgttccgcgaagcagtttcagctatacctatgtcacggttccgagaagcaggcctgttggatgtggtcttgcagctcgcgggacctaagcggcagcaagaaacggcggtcgagggcgaagaaaccgagtcgatcgacgagatggatgtagataaccttattcggatggcactggacgggaaagactcctgatgacataaccccttggggcctctaaacgggtcttgaggggttttttgaggac

SEQ ID NO: 35 - DNA, 5650 bp, Artificial Sequence
  DNA fragment
gtaatgagaccttgaggtaaaccaaataagacgccacgcgtagtgagacatacacgttcgttgggttcacgactcaacacgctagggacgtgaagtcgattccttcgatgcattgtaatagccaccaaaagagtgatgatagtcatgggtgtctgtagcacgtgcatcgctcattacaacggttatcacgtagtggcgtgcacgcggtcgatcttgacggctggcgagaggtgcggggaggatctgaccgacgcggtccacacgtggcaccgcgatgctgttgtgggcacaatcgtgccggttggtaggatccagcgatgtcgaacgaacaaaagctccgtgattatttgaagcgcgtcaccacagatcttgcagaaacccggcgtcgtctgggtcaagccgaggcggcacggcacgaaccaatagcgattgtcggcatggcctgccgctatccagggggtgtagagtctccagaagacctgtgggaactggttgcggagggccgcgacgccatcgatgtcatgccaggcgaccggggttgggatgtcgacgcgctgtatgatcctgacccgagctcgaccggtaagacgtactctcgcgagggtggattcctgcgaaacgcagcggaattcgatcccgcgtttttcggcatctcacctcgggaagccctggcgatggatccacagcaacgtttgctcttggaaactagctgggaggcgttcgagcgcgccggtatcgaccccgcaaccctgcgcggatcgcggacgggtgtgttcgccggtgtcatgtatcatgattacgggtctcggctgggtaccggaacggtacccgaggacgtcgagggctatgtcggcaacggaagcgccggttcgatcgccacgggtcgtatcgcctacacccttggcctggaaggtccggcggtcaccgtcgataccgcgtgcagctctagtctggtcgccatgcatttggccatccaagcgatacggcaaggagagtgcagcatggcgctggccggaggtgtgaccgtcatggcaaccccggacacctttgtggaattctcgagacagcgcggtctggcccccgacggccgctgtaaggctttcggagcaggagccgatggtaccggctgggcagagggagctggtatgctgctcgtggaacgtctgtcggatgctgaacgtttgggccatcccatccttgctgtcgtacggggtagcgcggtcaaccaggacggagccagtaacggcttgaccgcgccaaacggaccctcgcagcaacgcgtgatacgccaggccctggccacagcaggtttgggtcccaccgatatcgacgcggtcgagggtcacggaaccggcacgtccctgggtgaccccattgaagtgcaagcgctgcaagcgacctacggccaggagcggccggcagagcggccgttgtggttgggtagcctcaagtctaacattgggcacgcccaggcggccgctggtgtgggcggtgtgatcaagatggtcatggcccttcgggaaggcgtgctgccgcggacccttcacgctgacgaaccttcaccgcatatcgattggacagccggtgcggtccgcctcctgaccgaacaatccgcctggccggacaccgatcgtccacggcgtgccgcggtgtcgtccttcggagtctcgggcaccaacgcgcacgttatcattgagcagccatccgaacctgtagaacctgcggacacggacccggagtcacacagcgacagcgaggcagattcggatggaaccccagtggtacaccctgcactgctcccctggcctgtctccgcccggggtgcagatgccgtcagagctcaagctgcccgtttgcatgcgcatctgttggccaggccggatctcacggcggctgatgtagctttcagccttggcaccacacggaccgcgctgcctcatcggtttattgcactgggtaccgaccgcgccgaattgatcaacaccctcgcccggttcgccgaaggctcggaatcagcggctgatggcctcaccggcactgcgaccccaggcgcaaccgcattcctcttcagcggccaaggctcacaatgggcgggcatgggtagagaactccaagctcggttcccccgctttaggcaggccttggatgagacgaggctaggtggaggctcagtgatgataagtctgcgatggtggatgcatgtgtcatggtcatagctgtttcctgtgtgaaattgttatccgctcagagggcacaatcctattccgcgctatccgacaatctccaagacattaggtggagttcagttcggcgtatggcatatgtcgctggaaagaacatgtgagcaaaaggccagcaaaaggccaggaaccgtaaaaaggccgcgttgctggcgtttttccataggctccgcccccctgacgagcatcacaaaaatcgacgctcaagtcagaggtggcgaaacccgacaggactataaagataccaggcgtttccccctggaagctccctcgtgcgctctcctgttccgaccctgccgcttaccggatacctgtccgcctttctcccttcgggaagcgtggcgctttctcatagctcacgctgtaggtatctcagttcggtgtaggtcgttcgctccaagctgggctgtgtgcacgaaccccccgttcagcccgaccgctgcgccttatccggtaactatcgtcttgagtccaacccggtaagacacgacttatcgccactggcagcagccactggtaacaggattagcagagcgaggtatgtaggcggtgctacagagttcttgaagtggtggcctaactacggctacactagaagaacagtatttggtatctgcgctctgctgaagccagttaccttcggaaaaagagttggtagctcttgatccggcaaacaaaccaccgctggtagcggtggtttttttgtttgcaagcagcagattacgcgcagaaaaaaaggatctcaagaagatcctttgatcttttctacggggtctgacgctctattcaacaaagccgccgtcccgtcaagtcagcgtaaatgggtagggggcttcaaatcgtcctcgtgataccaattcggagcctgcttttttgtacaaacttgttgataatggcaattcaaggatcttcacctagatccttttaaattaaaaatgaagttttaaatcaatctaaagtatatatgagtaaacttggtctgacagttaccaatgcttaatcagtgaggcacctatctcagcgatctgtctatttcgttcatccatagttgcctgactccccgtcgtgtagataactacgatacgggagggcttaccatctggccccagtgctgcaatgataccgcgagagccacgctcaccggctccagatttatcagcaataaaccagccagccggaagggccgagcgcagaagtggtcctgcaactttatccgcctccatccagtctattaattgttgccgggaagctagagtaagtagttcgccagttaatagtttgcgcaacgttgttgccattgctacaggcatcgtggtgtcacgctcgtcgtttggtatggcttcattcagctccggttcccaacgatcaaggcgagttacatgatcccccatgttgtgcaaaaaagcggttagctccttcggtcctccgatcgttgtcagaagtaagttggccgcagtgttatcactcatggttatggcagcactgcataattctcttactgtcatgccatccgtaagatgcttttctgtgactggtgagtactcaaccaagtcattctgagaatagtgtatgcggcgaccgagttgctcttgcccggcgtcaatacgggataataccgcgccacatagcagaactttaaaagtgctcatcattggaaaacgttcttcggggcgaaaactctcaaggatcttaccgctgttgagatccagttcgatgtaacccactcgtgcacccaactgatcttcagcatcttttactttcaccagcgtttctgggtgagcaaaaacaggaaggcaaaatgccgcaaaaaagggaataagggcgacacggaaatgttgaatactcatactcttcctttttcaatattattgaagcatttatcagggttattgtctcatgagcggatacatatttgaatgtatttagaaaaataaacaaataggggttccgcgcacatttccccgaaaagtgccagatacctgaaacaaaacccatcgtacggccaaggaagtctccaataactgtgatccaccacaagcgccagggttttcccagtcacgacgttgtaaaacgacggccagtcatgcataatccgcacgcatctggaataaggaagtgccattccgcctgacctcgtctcatactgctttcgcggcgcggtccatccgccgatggcatggccgaagtccaacgcgagttggctgaagctggagcgtccgtagaagtactggcgtgcgatgctgcggaccgcgacgctttggcccaggtactggacggtcgagagctcacggctgtcatccatgcggccggcgtcctggacgatggagtgctggaagcgctggacgcgtcgcggttggacaccgtcttgcaaccaaagatggatgcggcatggaacctgcacgagcttacacggcacctggacttgacagcgtttgtcttgttctccagcgccaccggcgtcctgggcaacgctggccaggcgaactatgcggccgctaacgtattccttgacgcattggcacaaacccgcaggaccgaaaacctccctggtcatagcttggcatggggtctgtgggcagaagcttccgccatgacggccggcctgagcgaaaccgaccgccatagaattgcccgtctgggcgctcagccgctcaacgaaaccgaagcactggcacttttggacagggctttgggtgaagacgcacccgcactgttggtccctgtgcgtctgaaccttgcggcactgcagggtcgctctcaagcggttcctgccgttctgcgcgcgcttgtaccagtccgggcgcggcgccaggccgcggtcggcgcagccgctggttctggtggaggcctcgtagaaaggcttgcggctatgtccgagtcacgacgtgccgcgcatctgcttgatctggtccggaccgaagtcgctggtgtactgggccaccgctccgcggctaccattgaacccgagcgcgccttcaaggacctgggtttcgattcgctcaccgccgtcgagctgcggaaccggctccatgctgccaccggtctgaagccggcggccaccgtggtcttcgaccacccaacctccgccgacctggcgcgccaccttcgtacgcagatcccagatctgccagctgccggaccagaatgtcttctgggcgaactggatcggatagaacagatgctgacagatgttgaccccacagacgaaaagtcgggagacatccagcgccgcctgacggcgctgcttgctcgctttgacgaggccgcggggccagtcgaagcagctcaagtggcagataagatcgatgcagccaccgacgatgaaatttttgctttcattgacaacgagctcggttgatagcataaccccttggggcctctaaacgggtcttgaggggttttttgactac

SEQ ID NO: 36 - DNA, 5652 bp, Artificial Sequence
  DNA fragment
aactagagaccgtcagcgtcacgccacgcgtagtgagacatacacgttcgttgggttcacgactcaacacgctagggacgtgaagtcgattccttcgatgcattgtaatagccaccaaaagagtgatgatagtcatgggtgtctgtagcacgtgcatcgctcattacaacggttatgagcacgcggcgtgcacgcggtcgatcttgacggctggcgagaggtgcggggaggatctgaccgacgcggtccacacgtggcaccgcgatgctgttgtgggcacaatcgtgccggttggtaggatccagcgatggcggaccacgacaagctcgttgattatttgaagcgcgtcaccgcagatcttcaacagacccgccagcgtctgcgggagtacgaaacccagagccatgaaccaatagcaatcgttggcatgggctgccgctaccctggatccgtggcatcccctgaagagctgtggcgcctggtccacggtggcgtggacgccgtcggcggtctcccgaccgaccgggggtgggatgtggaagccttgtacgatcctaaggcacagaacccgggcacgacctatgcccgtgaaggtggctacctgaccggagcgacagagttcgacccggaattctttggtatctccccccgtgaggccctggccatggatcctcaacagcgcttggtgctcgaggtcgcttgggaaaccctggagcatgccggcatcgactccgccacactgcgcggcagctcgaccggtgttttcgtgggatgtaactatcaggagtaccgggcaaggctgtcggaggtacaggaaggccttgaaggccatctggtgaccggctccgtaagctccgtggtgtcgggccgtgtttcttacgtcctcggccttgagggccccgctcttacggtcgacaccgcttgttccagtagcttggtcaccctgcacttggcttgcgaagcacttaggcggaacgaatgtaccatggcacttgccggcggagtggctgtcatgtcaacaccgcataccatcacgggtttctcccggcaacggggcgtggcagcggacggccggtgcaaggcatttagcgcaagcgcagacggtatgggtttcggcgaaggtgtaggtcttctgctcgtggaacgtctgtcggatgctcgacgtttgggccatcgcgtgcttgctgtcgtacggggtagcgcggtcaaccaggacggagccagtaacggcttgtccgcgccatcaggacccgctcagcaacgcgtgatacgccaggccctggtcaacgccggtgtgcaggccagccaggtcgacgtggtcgaggctcacggaaccggcacgcgcctgggtgaccccattgaagctcaagcgctgcaagcgacctacggccagggtcggccggcagagcggccgttgtggttgggtagcctcaagtctaacattgggcacgcccaggcggccgctggtgtgggcggtgtgatcaagatggtcatggcccttcgggaaggcgtgctgccgcccacccttcacgctgacgaaccttcaccgcatatcgattggacagccggtaacgtccgcctcctgaccgaatcacgggaatggccggaagcgggtcagccacggcgtgccgcggtgtcgtccttcggaatctcgggcaccaacgcgcacgttatcttggaggcggcagaagcagttgacgcatcgggggaggctgacggcggtgccggcgacgaaggcacgccagtgctttctggaaccgacgtggtagcctggcctgtcagtgcagcctcgccagacgccctgcgggcacaggccgaaagattgagggctcatgtggctgagcgtcctgggttggccagcgcggatgtagctttctcgcttgcaactagcaggtcggcccttgcacggcgcgcgctggttgtgggtggggatcgcgacgagctggtcgcaggcctggagagtctggccgcagaccggcccggcaacggccttgtcaagggtttggctgacctcgcaaccaagccggtgttcgtcttccccggccagggatcccaatgggccggaatggccgtcgaactgctcgatagctccccagtctttgcggatagtatgcaagcttgctcggaagctctgaacgagttcgtagattggaacctcctggaggtcctgcggtccgatgacgaagagttgagcaaccgcgtagatgtggtccagcctgtgctgtgggccgtaatggtgtccctcgcggcactctggcaggcgtgcggcgtccgcccggcagccgtggtaggccattctcagggcgagatagcagctgccgtggtcgctggtgccctgtcactccgtgatggggcccgcgtggtagccttgcggtcggcggtaatagcgcggctgttggccggtaagggtgcgatggcctccgttgcgctcgcatccgataccgtgcgtgaacgcctgaccccctgggagggtcgtctgtccttggcggctgtaaacggcccttcgtcatcggtggtctgcggccacttggacgcgttggatgagttcgtgtctgcattggaacatgacggcgtgagggtgcgcaggatagccgtggactacgcgtcccactctgtcttcgtagaacaagcggaggaagagttgcgcaacgtcctgaccgaagtctcgccgttgccgggcgaggtaccgttctattccaccgttaccggcgcggtgctcgacaccacgacccttgatgctggatattggtaccggaacttgcgccagacggtacgtttcgaagagactgtgcgcgaactgaccaggcgcggtcacgatgcattcattgaagtttctgcccatccggtcctgacggtcggcattcaggacaccttggaggctaccggaacacgccacgccgtctgtgggacactgcgtcgcggcgaaggaggcgcgcaacggctcctgacgtcccttggagaagcatgggtggcgggcatcgcggtcgattggtcgcgattgacgcccaccgctaccgccgtagaactgccaacgtacgcctttcaacattgagacgaggctaggtggaggctcagtgatgataagtctgcgatggtggatgcatgtgtcatggtcatagctgtttcctgtgtgaaattgttatccgctcagagggcacaatcctattccgcgctatccgacaatctccaagacattaggtggagttcagttcggcgtatggcatatgtcgctggaaagaacatgtgagcaaaaggccagcaaaaggccaggaaccgtaaaaaggccgcgttgctggcgtttttccataggctccgcccccctgacgagcatcacaaaaatcgacgctcaagtcagaggtggcgaaacccgacaggactataaagataccaggcgtttccccctggaagctccctcgtgcgctctcctgttccgaccctgccgcttaccggatacctgtccgcctttctcccttcgggaagcgtggcgctttctcatagctcacgctgtaggtatctcagttcggtgtaggtcgttcgctccaagctgggctgtgtgcacgaaccccccgttcagcccgaccgctgcgccttatccggtaactatcgtcttgagtccaacccggtaagacacgacttatcgccactggcagcagccactggtaacaggattagcagagcgaggtatgtaggcggtgctacagagttcttgaagtggtggcctaactacggctacactagaagaacagtatttggtatctgcgctctgctgaagccagttaccttcggaaaaagagttggtagctcttgatccggcaaacaaaccaccgctggtagcggtggtttttttgtttgcaagcagcagattacgcgcagaaaaaaaggatctcaagaagatcctttgatcttttctacggggtctgacgctctattcaacaaagccgccgtcccgtcaagtcagcgtaaatgggtagggggcttcaaatcgtcctcgtgataccaattcggagcctgcttttttgtacaaacttgttgataatggcaattcaaggatcttcacctagatccttttaaattaaaaatgaagttttaaatcaatctaaagtatatatgagtaaacttggtctgacagttaccaatgcttaatcagtgaggcacctatctcagcgatctgtctatttcgttcatccatagttgcctgactccccgtcgtgtagataactacgatacgggagggcttaccatctggccccagtgctgcaatgataccgcgagagccacgctcaccggctccagatttatcagcaataaaccagccagccggaagggccgagcgcagaagtggtcctgcaactttatccgcctccatccagtctattaattgttgccgggaagctagagtaagtagttcgccagttaatagtttgcgcaacgttgttgccattgctacaggcatcgtggtgtcacgctcgtcgtttggtatggcttcattcagctccggttcccaacgatcaaggcgagttacatgatcccccatgttgtgcaaaaaagcggttagctccttcggtcctccgatcgttgtcagaagtaagttggccgcagtgttatcactcatggttatggcagcactgcataattctcttactgtcatgccatccgtaagatgcttttctgtgactggtgagtactcaaccaagtcattctgagaatagtgtatgcggcgaccgagttgctcttgcccggcgtcaatacgggataataccgcgccacatagcagaactttaaaagtgctcatcattggaaaacgttcttcggggcgaaaactctcaaggatcttaccgctgttgagatccagttcgatgtaacccactcgtgcacccaactgatcttcagcatcttttactttcaccagcgtttctgggtgagcaaaaacaggaaggcaaaatgccgcaaaaaagggaataagggcgacacggaaatgttgaatactcatactcttcctttttcaatattattgaagcatttatcagggttattgtctcatgagcggatacatatttgaatgtatttagaaaaataaacaaataggggttccgcgcacatttccccgaaaagtgccagatacctgaaacaaaacccatcgtacggccaaggaagtctccaataactgtgatccaccacaagcgccagggttttcccagtcacgacgttgtaaaacgacggccagtcatgcataatccgcacgcatctggaataaggaagtgccattccgcctgacctcgtctcaactggtcttcgaccaccctaccccgctggctatcgccgcatacttgaaggccgagctgtacggacctgatccgggtgacgattccagcgtcctgaccgagctcgatggcctgtcccaacggttggcggcaatcgatcccgacaccaacacccgccttgagatcaccctgcgtctgcgctcgttgctgacgcagtggtccgaaccggacggtggacgcaccactgcagagacagcaacggcaacgagtaccacggcattggaatcggcatccgcggacgaggtcctggctttcattgacaccgagttggggatttgatgacataaccccttggggcctctaaacgggtcttgaggggttttttgccgtg

SEQ ID NO: 37 - DNA, 5631 bp, Artificial Sequence
  DNA fragment
acaatgagaccttgaggtaaaccaaaacgccacgcgtagtgagacatacacgttcgttgggttcacgactcaacacgctagggacgtgaagtcgattccttcgatgcattgtaatagccaccaaaagagtgatgatagtcatgggtgtctgtagcacgtgcatcgctcattacaacggttattaagcacgtagtggcgtgcacgcggtcgatcttgacggctggcgagaggtgcggggaggatctgaccgacgcggtccacacgtggcaccgcgatgctgttgtgggcacaatcgtgccggttggtaggatccagcgatggcgggcccaccgcctttccctcgtcggcgtggcccctcaggccgacgtcggtgcggcggacgggctacaccgggtagcgtccgggaccgcaccggcagacgcccagcggctgtccccagccgcgccgtgtgcgcggccgacctttgtgaagagaacgacgatggctccaagaacgtgtcggaacaccgcggatcagcgggtggtagcgttctgtttcctcgtacgggcacagtcctgccatgggtgcttacgggaccgggcgcagcggcggtgcgtgcacgctccgaagcgctgcgcacccacctccgcgcctctacggaatggagccctgcaggcgtaggtcaggcgctgctggcaggaacaggggcgggcgcggacacccaccgtgccgttgttctcgccggtgatcgtgcccaaactctgaatgccctggccgcgctgtctgcaggagcggaccacccagccgtctttaccagcacccgtgccgacgccagcccagctggtccagtgtttgtgtttccaggccaggggtctcaatggactggtatggctcgcgaattgttggattctgcccccgtatttgcccgtaaattgcatgattgcgccgacgcatttgccccgtatttgggtcacagcctcctggattccgttactggggcggccggcgggccagagcctgttggcgcggatgttgtgcaaccagccttgttcgcagtgatggttgccttgacggatctctggaatgcggccggtgtggcaccaggcgccttgctcggtcattcactgggggagctcgccgccgcccacgtcgctggcgttctcagcctggacgattcggcgcgcgtggtcgcgcgctggagccaagcccaagcaactctcgcaggccgtggggacatggtttccgtgctgctgcctgcggacgaactggcggatctgttggaccgccgttggccggggcgtctggtagttgcggtggagaatggcccgggtagtgccgtagccagcggtgatctggatgccgcggcagaacttgtagcccatcttactgcggaaggcattcatgcgcgtcgtgtcgatgtcggcttggccgcgcactctccccacatcgacgctattctcccccgcatccgcgcggatattgctccgatccgcgcacatacccccagtatccctgtttacagcgcgctgcacggcggcgcactcgacggtacccctatggatgcggcgtattggtgccgtaatttgcgttcaactgtgcgttttgcggatgctacgcgcgcagctttggaagcaggccatacaacatttgtggaagtttcacctcatccggtcttgacgacggccatggaagtgagtgccacccgtgcggcccatgcggcgaccgtattgggaactcttcgtcgtggtgagggtggtccaagccgttttctggcatcactggcggaactccatgtttcaggtggtgatgccgatttgcgtacggttctgcccgcgagccaggcggctggcttgccggaaaccgtcctgacggcgggtccgcgtggcgagagcgctgacggcgatagccgtcatgaagtgctgtgtgcacgtctggcaccgctcgacccagccgaacgccgcgcccaacttctgacagttgtgcgtgaatctgcggcggcggccttggatggcgatgaccagggaagcatcgatggtcgtcgcacctttcgtgatttgggtattacttcacttgcggcggttggcattcgtgatcgcctgcactccgcgacaggtcttcgcctgtcacctaccgtggtctttgaccatcctactccagatgcattggccgcccaccttgatacagaactgtttgggaccggggcagatgccgaaccggctccggcagccggcggccgtgcagttccacatgatgaaccgatggcaattgtgggtatggcctgtcgttacccgggtggagttggcgcaccggcggatctctggcgtactgtcctggcaggggtggatgcggtcggcccattgccagccgatcgtggctggaatatcgctgatggctacgacccggaacttgccgggccgggccgttttagccaacgcgagggcgggtttctgcacgatgcggcagagtttgacgccgaattcttcggcatctcaccccgtgaagctctggccatggatccgcaacagcgcctcgcccttgaaagtgcatgggaagcgattgaagacgcgggcttggatgcgcattcgctccgtggcagtcgtaccggagttttcctcggcctgattacccaggattatggcccgcgcgcgggcgagccgactacccgtgcgggtgccgttgaaggtcatctgtttctggggtcaacggggagtgtagcgtcggggcgcctgagttacaccctcggcctggagggcccttccctgaccattgatactgcctgcagttccagcctggtagcgttgcatgaggcgtgccaagcattgcgtacgggtgactgcgatatggcactgacaggcggcgtgacggtaatgccttctacaggcatgctggtcgagttttcgcgtcagcgtggtctgtcacctgatggccgttgtaaagcctttagtgcgtcagctgatggctttgggctggcagaaggggttggtatgcttgttgtggaacgcttgagcgacgcacgtcgcctcgggcatcgtgtgcttgccgtggttcgcggttcagcggttaatcaagatggggccagtaatggtctgtcggcaccatccggcccggcacaacagcgtgttattcgtcaagcgcttgtgaatgcgggtgtccaggcctctcaagtggacgtggttgaagctcatggtaccggcactaagcttggtgatccaattgaagcgcaggcgcttcaggccacttatggtcaaggccgcccggcagaacgtcctttgtggctcggatctctgaaaagcaatattgggcatgcacaagcagcggcgggtgttggtggcgttatcaaaatggttatggcactgcgcgagggcgtacttccccctacgcttcatgctgattgagacgaggctaggtggaggctcagtgatgataagtctgcgatggtggatgcatgtgtcatggtcatagctgtttcctgtgtgaaattgttatccgctcagagggcacaatcctattccgcgctatccgacaatctccaagacattaggtggagttcagttcggcgtatggcatatgtcgctggaaagaacatgtgagcaaaaggccagcaaaaggccaggaaccgtaaaaaggccgcgttgctggcgtttttccataggctccgcccccctgacgagcatcacaaaaatcgacgctcaagtcagaggtggcgaaacccgacaggactataaagataccaggcgtttccccctggaagctccctcgtgcgctctcctgttccgaccctgccgcttaccggatacctgtccgcctttctcccttcgggaagcgtggcgctttctcatagctcacgctgtaggtatctcagttcggtgtaggtcgttcgctccaagctgggctgtgtgcacgaaccccccgttcagcccgaccgctgcgccttatccggtaactatcgtcttgagtccaacccggtaagacacgacttatcgccactggcagcagccactggtaacaggattagcagagcgaggtatgtaggcggtgctacagagttcttgaagtggtggcctaactacggctacactagaagaacagtatttggtatctgcgctctgctgaagccagttaccttcggaaaaagagttggtagctcttgatccggcaaacaaaccaccgctggtagcggtggtttttttgtttgcaagcagcagattacgcgcagaaaaaaaggatctcaagaagatcctttgatcttttctacggggtctgacgctctattcaacaaagccgccgtcccgtcaagtcagcgtaaatgggtagggggcttcaaatcgtcctcgtgataccaattcggagcctgcttttttgtacaaacttgttgataatggcaattcaaggatcttcacctagatccttttaaattaaaaatgaagttttaaatcaatctaaagtatatatgagtaaacttggtctgacagttaccaatgcttaatcagtgaggcacctatctcagcgatctgtctatttcgttcatccatagttgcctgactccccgtcgtgtagataactacgatacgggagggcttaccatctggccccagtgctgcaatgataccgcgagagccacgctcaccggctccagatttatcagcaataaaccagccagccggaagggccgagcgcagaagtggtcctgcaactttatccgcctccatccagtctattaattgttgccgggaagctagagtaagtagttcgccagttaatagtttgcgcaacgttgttgccattgctacaggcatcgtggtgtcacgctcgtcgtttggtatggcttcattcagctccggttcccaacgatcaaggcgagttacatgatcccccatgttgtgcaaaaaagcggttagctccttcggtcctccgatcgttgtcagaagtaagttggccgcagtgttatcactcatggttatggcagcactgcataattctcttactgtcatgccatccgtaagatgcttttctgtgactggtgagtactcaaccaagtcattctgagaatagtgtatgcggcgaccgagttgctcttgcccggcgtcaatacgggataataccgcgccacatagcagaactttaaaagtgctcatcattggaaaacgttcttcggggcgaaaactctcaaggatcttaccgctgttgagatccagttcgatgtaacccactcgtgcacccaactgatcttcagcatcttttactttcaccagcgtttctgggtgagcaaaaacaggaaggcaaaatgccgcaaaaaagggaataagggcgacacggaaatgttgaatactcatactcttcctttttcaatattattgaagcatttatcagggttattgtctcatgagcggatacatatttgaatgtatttagaaaaataaacaaataggggttccgcgcacatttccccgaaaagtgccagatacctgaaacaaaacccatcgtacggccaaggaagtctccaataactgtgatccaccacaagcgccagggttttcccagtcacgacgttgtaaaacgacggccagtcatgcataatccgcacgcatctggaataaggaagtgccattccgcctgacctcgtctcaattagcacctgcttggattaactac

SEQ ID NO: 38 - DNA, 5426 bp, Artificial Sequence
  pSYN0002 vector
cgagacacccgggaagcctgatctacgtctgtcgagaagtttcgatgacactcgttcgttcacacgttgcagcagattacgagaccactagtgctgctccttcggtcggacgtgcgtctacgggcaccttaccgcagccgtcggctgtgcgacacggacggatcgggcgaactggccgatgctgggagaagcgcgctgctgtacggcgcgcaccgggtgcggagcccctcggcgagcggtgtgaaacttctgtgaatggcctgttcggttgctttttttatacggctgccagataaggcttgcagcatctgggcggctaccgctatgatcggggcgttcctgcaattcttagtgcgagtatctgaaaggggatacgccatatgctttccaagggcgaggaggacaacatggccatcatcaaggagttcatgcgcttcaaggtccacatggagggctccgtcaacgggcacgagttcgagatcgagggcgagggggagggccggccgtacgagggcacccagaccgccaagctgaaggtgaccaagggcggccccctcccgttcgcctgggacatcctctccccccagttcatgtacggctcgaaggcctacgtcaagcacccggccgacatcccggactacctgaagctctcgttcccggaggggttcaagtgggagcgggtcatgaacttcgaggacggcggcgtcgtcaccgtcacccaggacagctccctgcaggacggcgagttcatctacaaggtcaagctgcggggcacgaacttcccgagcgacggccccgtgatgcagaagaaaacgatgggctgggaagcgtcctcggagcgcatgtacccggaggacggcgccctcaagggcgagatcaagcagcgcctgaagctgaaggacggcggccactacgacgccgaagtcaagacgacgtacaaggccaagaagccggtgcagctcccggacgcctacaacgtgaacatcaagctcgacatcacctcgcacaacgaggactacacgatcgtggagcagtacgagcgcgccgagggccggcactcgaccggcggcatggacgagctgtacaagtgagccgttcgcgccgccccggctcgcatcgtccccgacccgtcaacctcatccgcaaggagtctctagaggatccgcggccgcgcgcgatatcgaattcctggtctccaaaagagtaacttaagccgaacaggaagcacagctcctactgaacatgtgagcaaaaggccagcaaaaggccaggaaccgtaaaaaggccgcgttgctggcgtttttccataggctccgcccccctgacgagcatcacaaaaatcgacgctcaagtcagaggtggcgaaacccgacaggactataaagataccaggcgtttccccctggaagctccctcgtgcgctctcctgttccgaccctgccgcttaccggatacctgtccgcctttctcccttcgggaagcgtggcgctttctcatagctcacgctgtaggtatctcagttcggtgtaggtcgttcgctccaagctgggctgtgtgcacgaaccccccgttcagcccgaccgctgcgccttatccggtaactatcgtcttgagtccaacccggtaagacacgacttatcgccactggcagcagccactggtaacaggattagcagagcgaggtatgtaggcggtgctacagagttcttgaagtggtggcctaactacggctacactagaagaacagtatttggtatctgcgctctgctgaagccagttaccttcggaaaaagagttggtagctcttgatccggcaaacaaaccaccgctggtagcggtggtttttttgtttgcaagcagcagattacgcgcagaaaaaaaggatctcaagaagatcctttgatcttttctacggggtctgacgctcagtggaacgaaaactcacgttaagggattttggtcatgagattatcaaaaaggatcttcacctagatccttttggttcatgtgcagctccatcagcaaaaggggatgataagtttatcaccaccgactatttgcaacagtgccgttgatcgtgctatgatcgactgatgtcatcagcggtggagtgcaatgtcgtgcaatacgaatggcgaaaagccgagctcatcggtcagcttctcaaccttggggttacccccggcggtgtgctgctggtccacagctccttccgtagcgtccggcccctcgaagatgggccacttggactgatcgaggccctgcgtgctgcgctgggtccgggagggacgctcgtcatgccctcgtggtcaggtctggacgacgagccgttcgatcctgccacgtcgcccgttacaccggaccttggagttgtctctgacacattctggcgcctgccaaatgtaaagcgcagcgcccatccatttgcctttgcggcagcggggccacaggcagagcagatcatctctgatccattgcccctgccacctcactcgcctgcaagcccggtcgcccgtgtccatgaactcgatgggcaggtacttctcctcggcgtgggacacgatgccaacacgacgctgcatcttgccgagttgatggcaaaggttccctatggggtgccgagacactgcaccattcttcaggatggcaagttggtacgcgtcgattatctcgagaatgaccactgctgtgagcgctttgccttggcggacaggtggctcaaggagaagagccttcagaaggaaggtccagtcggtcatgcctttgctcggttgatccgctcccgcgacattgtggcgacagccctgggtcaactgggccgagatccgttgatcttcctgcatccgccagaggcgggatgcgaagaatgcgatgccgctcgccagtcgattggctgagctcatgagcggagaacgagatgacgttggaggggcaaggtcgcgctgattgctggggcaacacgtggagcggatcggggattgtctttcttcagctcgctgatgatatgccttcctggttggcttggtttcatcagccatccgcttgccctcatctgttacgccggcggtagccggccagcctcgcagagcaggattcccgttgagcaccgccaggtgcgaataagggacagtgaagaaggaacacccgctcgcgggtgggcctacttcacctatcctgcccggctgacgccgttggatacaccaaggaaagtctacacgaaccctttggcaaaatcctgtatatcgtgcgaaaaaggatggatataccgaaaaaatcgctataatgaccccgaagcagggttatgcagcggaaaagatccgtcgacctgcaggcatgcaagctctagcgattccagacgtcccgaaggcgtggcgcggcttccccgtgccggagcaatcgccctgggtgggttacacgacgcccctctatggcccgtactgacggacacaccgaagccccggcggcaaccctcagcggatgccccggggcttcacgttttcccaggtcagaagcggttttcgggagtagtgccccaactggggtaacctttgagttctctcagttgggggcgtagggtcgccgacatgacacaaggggttgtgaccggggtggacacgtacgcgggtgcttacgaccgtcagtcgcgcgagcgcgaaaattcgagcgcagcaagcccagcgacacagcgtagcgccaacgaggacaaggcggccgaccttcagcgcgaagtcgagcgcgacgggggccggttcaggttcgtcgggcatttcagcgaagcgccgggcacgtcggcgttcgggacggcggagcgcccggagttcgaacgcatcctgaacgaatgccgcgccgggcggctcaacatgatcattgtctatgacgtgtcgcgcttctcgcgcctgaaggtcatggacgcgattccgattgtctcggaattgctcgccctgggcgtgacgattgtttccactcaggaaggcgtgttccggcagggaaacgtcatggacctgattcacctgattatgcggctcgacgcgtcgcacaaagaatcttcgctgaagtcggcgaagattctcgacacgaagaaccttcagcgcgaattgggcgggtacgtcggcgggaaggcgccttacggcttcgagcttgtttcggagacgaaggagatcacgcgcaacggccgaatggtcaatgtcgtcatcaacaagcttgcgcactcgaccactccccttaccggacccttcgagttcgagcccgacgtaatccggtggtggtggcgtgagatcaagacgcacaagcaccttcccttcaagccgggcagtcaagccgccattcacccgggcagcatcacggggctttgtaagcgcatggacgctgacgccgtgccgacccggggcgagacgattgggaagaaaaccgcttcaagcgcctgggacccggcaaccgttatgcgaatccttcgggacccgcgtattgcgggcttcgccgctgaggtgatctacaagaagaagccggacggcacgccgaccacgaagattgagggttaccgcattcagcgcgacccgatcacgctccggccggtcgagcttgattgcggaccgatcatcgagcccgctgagtggtatgagcttcaggcgtggttggacggcagggggcgcggcaaggggctttcccgggggcaagccattctgtccgccatggacaagctgtactgcgagtgtggcgccgtcatgacttcgaagcgcggggaagaatcgatcaaggactcttaccgctgccgtcgccggaaggtggtcgacccgtccgcacctgggcagcacgaaggcacgtgcaacgtcagcatggcggcactcgacaagttcgttgcggaacgcatcttcaacaagatcaggcacgccgaaggcgacgaagagacgttggcgcttctgtgggaagccgcccgacgcttcggcaagctcactgaggcgcctgagaagagcggcgaacgggcgaaccttgttgcggagcgcgccgacgccctgaacgcccttgaagagctgtacgaggaccgcgcggcaggcgcgtacgacggacccgttggcaggaagcacttccggaagcaacaggcagcgctgacgctccggcagcaaggggcggaagagcggcttgccgaacttgaagccgccgaagccccgaagcttccccttgaccaatggttccccgaggacgccgacgctgacccgaccggccctaagtcgtggtgggggcgcgcgtcagtagacgacaagcgcgtgttcgtcgggctcttcgtagacaagatcgttgtcacgaagtcgactacgggcagggggcagggaacgcccatcgagaagcgcgcttcgatcacgtgggcgaagccgccgaccgacgacgacgaggacgacgcccaggacggcacggaggacgtagcggcgtag